European Patent Application EP 4 578 878 A1, published July 2, 2025. Title: 一种融合前构象的呼吸道合胞病毒重组融合蛋白、其制备方法及用途. Applicant: 北京百邑无忧科技发展有限公司. The sequence listing filed with the application follows.

SEQUENCE LISTING (180 sequences)

SEQ ID NO: 1 - protein, 574 aa, synthetic construct
MELLILKANAITTILTAVTFCFASGQNITEEFYQSTCSAVSKGYLSALRTGWYTSVITIELSNIKENKCNGTDAKVKLIKQELDKYKNAVTELQLLMQSTPATNNRARRELPRFMNYTLNNAKKTNVTLSKKRKRRFLGFLLGVGSAIASGVAVSKVLHLEGEVNKIKSALLSTNKAVVSLSNGVSVLTSKVLDLKNYIDKQLLPIVNKQSCSISNIETVIEFQQKNNRLLEITREFSVNAGVTTPVSTYMLTNSELLSLINDMPITNDQKKLMSNNVQIVRQQSYSIMSIIKEEVLAYVVQLPLYGVIDTPCWKLHTSPLCTTNTKEGSNICLTRTDRGWYCDNAGSVSFFPQAETCKVQSNRVFCDTMNSLTLPSEVNLCNVDIFNPKYDCKIMTSKTDVSSSVITSLGAIVSCYGKTKCTASNKNRGIIKTFSNGCDYVSNKGVDTVSVGNTLYYVNKQEGKSLYVKGEPIINFYDPLVFPSDEFDASISQVNEKINQSLAFIRKSDELLHNVNAGKSTTNIMITTIIIVIIVILLSLIAVGLLLYCKARSTPVTLSKDQLSGINNIAFSN

SEQ ID NO: 2 - protein, 15 aa, synthetic construct
GGGGSGGGGSGGGGS

SEQ ID NO: 3 - protein, 15 aa, synthetic construct
GGPGSGGGGSGGGGS

SEQ ID NO: 4 - protein, 15 aa, synthetic construct
GGGGSPGGGSGGGGS

SEQ ID NO: 5 - protein, 15 aa, synthetic construct
GGGGPGGGGSGGGGS

SEQ ID NO: 6 - protein, 15 aa, synthetic construct
GGGGSGGGPSGGGGS

SEQ ID NO: 7 - protein, 7 aa, synthetic construct
GSGSGRS

SEQ ID NO: 8 - skipped

SEQ ID NO: 9 - protein, 36 aa, synthetic construct
TPATNNRARRELPRFMNYTLNNAKKTNVTLSKKRKR

SEQ ID NO: 10 - protein, 36 aa, synthetic construct
TPATNNGSASELPRFMNYTLNNAKKTNVTLSKKGKG

SEQ ID NO: 11 - protein, 25 aa, synthetic construct
MELLILKANAITTILTAVTFCFASG

SEQ ID NO: 12 - protein, 25 aa, synthetic construct
MELPILKTNAITAILAAVTLCFASS

SEQ ID NO: 13 - protein, 25 aa, synthetic construct
MELLIHRSSAIFLTLAVNALYLTSS

SEQ ID NO: 14 - protein, 16 aa, synthetic construct
MKCLLYLAFLFIGVNC

SEQ ID NO: 15 - protein, 19 aa, synthetic construct
MGWSCIILFLVATATGVHS

SEQ ID NO: 16 - protein, 17 aa, synthetic construct
MRAWIFFLLCLAGRALA

SEQ ID NO: 17 - protein, 18 aa, synthetic construct
MAFLWLLSCWALLGTTFG

SEQ ID NO: 18 - protein, 20 aa, synthetic construct
MYRMQLLSCIALSLALVTNS

SEQ ID NO: 19 - protein, 16 aa, synthetic construct
MKPIFLVLLVVTSAYA

SEQ ID NO: 20 - protein, 21 aa, synthetic construct
MAPGRIFLVLFLISNTKPIHP

SEQ ID NO: 21 - protein, 25 aa, synthetic construct
MATTAMRMIISIIFISTYVTHITLC

SEQ ID NO: 22 - protein, 21 aa, synthetic construct
MIPGRIFLVLLLIFNTKPIHP

SEQ ID NO: 23 - protein, 15 aa, synthetic construct
MNLLLILTFVAAAVA

SEQ ID NO: 24 - protein, 29 aa, synthetic construct
GSGYIPEAPRDGQAYVRKDGEWVLLSTFL

SEQ ID NO: 25 - protein, 35 aa, synthetic construct
GSRMKQIERKIEEILSKIYHIENEIARIKKLIGER

SEQ ID NO: 26 - protein, 31 aa, synthetic construct
SAIGGYIPEAPRDGQAYVRKDGEWVLLSTFL

SEQ ID NO: 27 - protein, 37 aa, synthetic construct
SAIGRMKQIERKIEEILSKIYHIENEIARIKKLIGER

SEQ ID NO: 28 - protein, 8 aa, synthetic construct
HHHHHHHH

SEQ ID NO: 29 - protein, 467 aa, synthetic construct
QNITEEFYQSTCSAVSKGYLSALRTGWYTSVITIELSNIKEPKCNGTDAKVKLIKQELDKYKNAVTELQLLMQSGGPGSGGGGSGGGGSRFLGFLLGVGSAIASGVAVSKVLHLEGEVNKIKSALLSTNKAVVSLSNGVSVLTSKVLDLKNYIDKQLLPIVNKQSCSISNIETVIEFQQKNNRLLEITREFSVNAGVTTPVSTYMLTNSELLSLINDMPITNDQKKLMSNNVQIVRQQSYSIMSIIKEEVLAYVVQLPLYGVIDTPCWKLHTSPLCTTNTKEGSNICLTRTDRGWYCDNAGSVSFFPQAETCKVQSNRVFCDTMNSLTLPSEVNLCNVDIFNPKYDCKIMTSKTDVSSSVITSLGAIVSCYGKTKCTASNKNRGIIKTFSNGCDYVSNKGVDTVSVGNTLYYVNKQEGKSLYVKGEPIINFYDPLVFPSDEFDASISQVNEKINQSLAFIRKSDELL

SEQ ID NO: 30 - protein, 467 aa, synthetic construct
QNITEEFYQSTCSAVSKGYLSALRTGWYTSVITIELSNIKENKCNGTDAKVKLIKQELDKYKNAVTELQLLMQSGGPGSGGGGSGGGGSRFLGFPLGVGSAIASGVAVSKVLHLEGEVNKIKSALLSTNKAVVSLSNGVSVLTSKVLDLKNYIDKQLLPIVNKQSCSISNIETVIEFQQKNNRLLEITREFSVNAGVTTPVSTYMLTNSELLSLINDMPITNDQKKLMSNNVQIVRQQSYSIMSIIKEEVLAYVVQLPLYGVIDTPCWKLHTSPLCTTNTKEGSNICLTRTDRGWYCDNAGSVSFFPQAETCKVQSNRVFCDTMNSLTLPSEVNLCNVDIFNPKYDCKIMTSKTDVSSSVITSLGAIVSCYGKTKCTASNKNRGIIKTFSNGCDYVSNKGVDTVSVGNTLYYVNKQEGKSLYVKGEPIINFYDPLVFPSDEFDASISQVNEKINQSLAFIRKSDELL

SEQ ID NO: 31 - protein, 467 aa, synthetic construct
QNITEEFYQSTCSAVSKGYLSALRTGWYTSVITIELSNIKENKCNGTDAKVKLIKQELDKYKNAVTELQLLMQSGGPGSGGGGSGGGGSRFLGFLLGVGSAIASGVAVSKVLHLEGEVNKIKSALLSTNKAVVSLSNGVSVLTSKVLDLKNYIDKQLLPIVNKQSCSISNIETVIEFQQKNNRLLEITREFSVNAGVTTPVSTYMLTNSELLSLINDMPITNDQKKLMSNNVPIVRQQSYSIMSIIKEEVLAYVVQLPLYGVIDTPCWKLHTSPLCTTNTKEGSNICLTRTDRGWYCDNAGSVSFFPQAETCKVQSNRVFCDTMNSLTLPSEVNLCNVDIFNPKYDCKIMTSKTDVSSSVITSLGAIVSCYGKTKCTASNKNRGIIKTFSNGCDYVSNKGVDTVSVGNTLYYVNKQEGKSLYVKGEPIINFYDPLVFPSDEFDASISQVNEKINQSLAFIRKSDELL

SEQ ID NO: 32 - protein, 467 aa, synthetic construct
QNITEEFYQSTCSAVSKGYLSALRTGWYTSVITIELSNIKENKCNGTDAKVKLIKQELDKYKNAVTELQLLMQSGGPGSGGGGSGGGGSRFLGFLLGVGSAIASGVAVSKVLHLEGEVNKIKSALLSTNKAVVSLSNGVSVLTSKVLDLKNYIDKQLLPIVNKQSCSISNIETVIEFQQKNNRLLEITREFSVNAGVTTPVSTYMLTNSELLSLINDMPITNDQKKLMSNNVQIVRQQSYSIMSIIKEEVLAYVVQLPLYGVIDTPCWKLHTSPLCTTNTKEGSNICLTRTDRGWYCDNAGSVSFFPQAETCKVQSNRVFCDTMNSLTLPPEVNLCNVDIFNPKYDCKIMTSKTDVSSSVITSLGAIVSCYGKTKCTASNKNRGIIKTFSNGCDYVSNKGVDTVSVGNTLYYVNKQEGKSLYVKGEPIINFYDPLVFPSDEFDASISQVNEKINQSLAFIRKSDELL

SEQ ID NO: 33 - protein, 467 aa, synthetic construct
QNITEEFYQSTCSAVSKGYLSALRTGWYTSVITIELSNIKEPKCNGTDAKVKLIKQELDKYKNAVTELQLLMQSGGPGSGGGGSGGGGSRFLGFPLGVGSAIASGVAVSKVLHLEGEVNKIKSALLSTNKAVVSLSNGVSVLTSKVLDLKNYIDKQLLPIVNKQSCSISNIETVIEFQQKNNRLLEITREFSVNAGVTTPVSTYMLTNSELLSLINDMPITNDQKKLMSNNVQIVRQQSYSIMSIIKEEVLAYVVQLPLYGVIDTPCWKLHTSPLCTTNTKEGSNICLTRTDRGWYCDNAGSVSFFPQAETCKVQSNRVFCDTMNSLTLPSEVNLCNVDIFNPKYDCKIMTSKTDVSSSVITSLGAIVSCYGKTKCTASNKNRGIIKTFSNGCDYVSNKGVDTVSVGNTLYYVNKQEGKSLYVKGEPIINFYDPLVFPSDEFDASISQVNEKINQSLAFIRKSDELL

SEQ ID NO: 34 - protein, 467 aa, synthetic construct
QNITEEFYQSTCSAVSKGYLSALRTGWYTSVITIELSNIKEPKCNGTDAKVKLIKQELDKYKNAVTELQLLMQSGGPGSGGGGSGGGGSRFLGFLLGVGSAIASGVAVSKVLHLEGEVNKIKSALLSTNKAVVSLSNGVSVLTSKVLDLKNYIDKQLLPIVNKQSCSISNIETVIEFQQKNNRLLEITREFSVNAGVTTPVSTYMLTNSELLSLINDMPITNDQKKLMSNNVPIVRQQSYSIMSIIKEEVLAYVVQLPLYGVIDTPCWKLHTSPLCTTNTKEGSNICLTRTDRGWYCDNAGSVSFFPQAETCKVQSNRVFCDTMNSLTLPSEVNLCNVDIFNPKYDCKIMTSKTDVSSSVITSLGAIVSCYGKTKCTASNKNRGIIKTFSNGCDYVSNKGVDTVSVGNTLYYVNKQEGKSLYVKGEPIINFYDPLVFPSDEFDASISQVNEKINQSLAFIRKSDELL

SEQ ID NO: 35 - protein, 467 aa, synthetic construct
QNITEEFYQSTCSAVSKGYLSALRTGWYTSVITIELSNIKEPKCNGTDAKVKLIKQELDKYKNAVTELQLLMQSGGPGSGGGGSGGGGSRFLGFLLGVGSAIASGVAVSKVLHLEGEVNKIKSALLSTNKAVVSLSNGVSVLTSKVLDLKNYIDKQLLPIVNKQSCSISNIETVIEFQQKNNRLLEITREFSVNAGVTTPVSTYMLTNSELLSLINDMPITNDQKKLMSNNVQIVRQQSYSIMSIIKEEVLAYVVQLPLYGVIDTPCWKLHTSPLCTTNTKEGSNICLTRTDRGWYCDNAGSVSFFPQAETCKVQSNRVFCDTMNSLTLPPEVNLCNVDIFNPKYDCKIMTSKTDVSSSVITSLGAIVSCYGKTKCTASNKNRGIIKTFSNGCDYVSNKGVDTVSVGNTLYYVNKQEGKSLYVKGEPIINFYDPLVFPSDEFDASISQVNEKINQSLAFIRKSDELL

SEQ ID NO: 36 - protein, 467 aa, synthetic construct
QNITEEFYQSTCSAVSKGYLSALRTGWYTSVITIELSNIKENKCNGTDAKVKLIKQELDKYKNAVTELQLLMQSGGPGSGGGGSGGGGSRFLGFPLGVGSAIASGVAVSKVLHLEGEVNKIKSALLSTNKAVVSLSNGVSVLTSKVLDLKNYIDKQLLPIVNKQSCSISNIETVIEFQQKNNRLLEITREFSVNAGVTTPVSTYMLTNSELLSLINDMPITNDQKKLMSNNVPIVRQQSYSIMSIIKEEVLAYVVQLPLYGVIDTPCWKLHTSPLCTTNTKEGSNICLTRTDRGWYCDNAGSVSFFPQAETCKVQSNRVFCDTMNSLTLPSEVNLCNVDIFNPKYDCKIMTSKTDVSSSVITSLGAIVSCYGKTKCTASNKNRGIIKTFSNGCDYVSNKGVDTVSVGNTLYYVNKQEGKSLYVKGEPIINFYDPLVFPSDEFDASISQVNEKINQSLAFIRKSDELL

SEQ ID NO: 37 - protein, 467 aa, synthetic construct
QNITEEFYQSTCSAVSKGYLSALRTGWYTSVITIELSNIKENKCNGTDAKVKLIKQELDKYKNAVTELQLLMQSGGPGSGGGGSGGGGSRFLGFPLGVGSAIASGVAVSKVLHLEGEVNKIKSALLSTNKAVVSLSNGVSVLTSKVLDLKNYIDKQLLPIVNKQSCSISNIETVIEFQQKNNRLLEITREFSVNAGVTTPVSTYMLTNSELLSLINDMPITNDQKKLMSNNVQIVRQQSYSIMSIIKEEVLAYVVQLPLYGVIDTPCWKLHTSPLCTTNTKEGSNICLTRTDRGWYCDNAGSVSFFPQAETCKVQSNRVFCDTMNSLTLPPEVNLCNVDIFNPKYDCKIMTSKTDVSSSVITSLGAIVSCYGKTKCTASNKNRGIIKTFSNGCDYVSNKGVDTVSVGNTLYYVNKQEGKSLYVKGEPIINFYDPLVFPSDEFDASISQVNEKINQSLAFIRKSDELL

SEQ ID NO: 38 - protein, 467 aa, synthetic construct
QNITEEFYQSTCSAVSKGYLSALRTGWYTSVITIELSNIKENKCNGTDAKVKLIKQELDKYKNAVTELQLLMQSGGPGSGGGGSGGGGSRFLGFLLGVGSAIASGVAVSKVLHLEGEVNKIKSALLSTNKAVVSLSNGVSVLTSKVLDLKNYIDKQLLPIVNKQSCSISNIETVIEFQQKNNRLLEITREFSVNAGVTTPVSTYMLTNSELLSLINDMPITNDQKKLMSNNVPIVRQQSYSIMSIIKEEVLAYVVQLPLYGVIDTPCWKLHTSPLCTTNTKEGSNICLTRTDRGWYCDNAGSVSFFPQAETCKVQSNRVFCDTMNSLTLPPEVNLCNVDIFNPKYDCKIMTSKTDVSSSVITSLGAIVSCYGKTKCTASNKNRGIIKTFSNGCDYVSNKGVDTVSVGNTLYYVNKQEGKSLYVKGEPIINFYDPLVFPSDEFDASISQVNEKINQSLAFIRKSDELL

SEQ ID NO: 39 - protein, 467 aa, synthetic construct
QNITEEFYQSTCSAVSKGYLSALRTGWYTSVITIELSNIKEPKCNGTDAKVKLIKQELDKYKNAVTELQLLMQSGGPGSGGGGSGGGGSRFLGFPLGVGSAIASGVAVSKVLHLEGEVNKIKSALLSTNKAVVSLSNGVSVLTSKVLDLKNYIDKQLLPIVNKQSCSISNIETVIEFQQKNNRLLEITREFSVNAGVTTPVSTYMLTNSELLSLINDMPITNDQKKLMSNNVPIVRQQSYSIMSIIKEEVLAYVVQLPLYGVIDTPCWKLHTSPLCTTNTKEGSNICLTRTDRGWYCDNAGSVSFFPQAETCKVQSNRVFCDTMNSLTLPSEVNLCNVDIFNPKYDCKIMTSKTDVSSSVITSLGAIVSCYGKTKCTASNKNRGIIKTFSNGCDYVSNKGVDTVSVGNTLYYVNKQEGKSLYVKGEPIINFYDPLVFPSDEFDASISQVNEKINQSLAFIRKSDELL

SEQ ID NO: 40 - protein, 467 aa, synthetic construct
QNITEEFYQSTCSAVSKGYLSALRTGWYTSVITIELSNIKEPKCNGTDAKVKLIKQELDKYKNAVTELQLLMQSGGPGSGGGGSGGGGSRFLGFPLGVGSAIASGVAVSKVLHLEGEVNKIKSALLSTNKAVVSLSNGVSVLTSKVLDLKNYIDKQLLPIVNKQSCSISNIETVIEFQQKNNRLLEITREFSVNAGVTTPVSTYMLTNSELLSLINDMPITNDQKKLMSNNVQIVRQQSYSIMSIIKEEVLAYVVQLPLYGVIDTPCWKLHTSPLCTTNTKEGSNICLTRTDRGWYCDNAGSVSFFPQAETCKVQSNRVFCDTMNSLTLPPEVNLCNVDIFNPKYDCKIMTSKTDVSSSVITSLGAIVSCYGKTKCTASNKNRGIIKTFSNGCDYVSNKGVDTVSVGNTLYYVNKQEGKSLYVKGEPIINFYDPLVFPSDEFDASISQVNEKINQSLAFIRKSDELL

SEQ ID NO: 41 - protein, 467 aa, synthetic construct
QNITEEFYQSTCSAVSKGYLSALRTGWYTSVITIELSNIKEPKCNGTDAKVKLIKQELDKYKNAVTELQLLMQSGGPGSGGGGSGGGGSRFLGFLLGVGSAIASGVAVSKVLHLEGEVNKIKSALLSTNKAVVSLSNGVSVLTSKVLDLKNYIDKQLLPIVNKQSCSISNIETVIEFQQKNNRLLEITREFSVNAGVTTPVSTYMLTNSELLSLINDMPITNDQKKLMSNNVPIVRQQSYSIMSIIKEEVLAYVVQLPLYGVIDTPCWKLHTSPLCTTNTKEGSNICLTRTDRGWYCDNAGSVSFFPQAETCKVQSNRVFCDTMNSLTLPPEVNLCNVDIFNPKYDCKIMTSKTDVSSSVITSLGAIVSCYGKTKCTASNKNRGIIKTFSNGCDYVSNKGVDTVSVGNTLYYVNKQEGKSLYVKGEPIINFYDPLVFPSDEFDASISQVNEKINQSLAFIRKSDELL

SEQ ID NO: 42 - protein, 467 aa, synthetic construct
QNITEEFYQSTCSAVSKGYLSALRTGWYTSVITIELSNIKENKCNGTDAKVKLIKQELDKYKNAVTELQLLMQSGGPGSGGGGSGGGGSRFLGFPLGVGSAIASGVAVSKVLHLEGEVNKIKSALLSTNKAVVSLSNGVSVLTSKVLDLKNYIDKQLLPIVNKQSCSISNIETVIEFQQKNNRLLEITREFSVNAGVTTPVSTYMLTNSELLSLINDMPITNDQKKLMSNNVPIVRQQSYSIMSIIKEEVLAYVVQLPLYGVIDTPCWKLHTSPLCTTNTKEGSNICLTRTDRGWYCDNAGSVSFFPQAETCKVQSNRVFCDTMNSLTLPPEVNLCNVDIFNPKYDCKIMTSKTDVSSSVITSLGAIVSCYGKTKCTASNKNRGIIKTFSNGCDYVSNKGVDTVSVGNTLYYVNKQEGKSLYVKGEPIINFYDPLVFPSDEFDASISQVNEKINQSLAFIRKSDELL

SEQ ID NO: 43 - protein, 467 aa, synthetic construct
QNITEEFYQSTCSAVSKGYLSALRTGWYTSVITIELSNIKEPKCNGTDAKVKLIKQELDKYKNAVTELQLLMQSGGPGSGGGGSGGGGSRFPPFLLGVGSAIASGVAVSKVLHLEGEVNKIKSALLSTNKAVVSLSNGVSVLTSKVLDLKNYIDKQLLPIVNKQSCSISNIETVIEFQQKNNRLLEITREFSVNAGVTTPVSTYMLTNSELLSLINDMPITNDQKKLMSNNVQIVRQQSYSIMSIIKEEVLAYVVQLPLYGVIDTPCWKLHTSPLCTTNTKEGSNICLTRTDRGWYCDNAGSVSFFPQAETCKVQSNRVFCDTMNSLTLPSEVNLCNVDIFNPKYDCKIMTSKTDVSSSVITSLGAIVSCYGKTKCTASNKNRGIIKTFSNGCDYVSNKGVDTVSVGNTLYYVNKQEGKSLYVKGEPIINFYDPLVFPSDEFDASISQVNEKINQSLAFIRKSDELL

SEQ ID NO: 44 - protein, 467 aa, synthetic construct
QNITEEFYQSTCSAVSKGYLSALRTGWYTSVITIELSNIKENKCNGTDAKVKLIKQELDKYKNAVTELQLLMQSGGPGSGGGGSGGGGSRFPPFLLGVGSAIASGVAVSKVLHLEGEVNKIKSALLSTNKAVVSLSNGVSVLTSKVLDLKNYIDKQLLPIVNKQSCSISNIETVIEFQQKNNRLLEITREFSVNAGVTTPVSTYMLTNSELLSLINDMPITNDQKKLMSNNVPIVRQQSYSIMSIIKEEVLAYVVQLPLYGVIDTPCWKLHTSPLCTTNTKEGSNICLTRTDRGWYCDNAGSVSFFPQAETCKVQSNRVFCDTMNSLTLPSEVNLCNVDIFNPKYDCKIMTSKTDVSSSVITSLGAIVSCYGKTKCTASNKNRGIIKTFSNGCDYVSNKGVDTVSVGNTLYYVNKQEGKSLYVKGEPIINFYDPLVFPSDEFDASISQVNEKINQSLAFIRKSDELL

SEQ ID NO: 45 - protein, 467 aa, synthetic construct
QNITEEFYQSTCSAVSKGYLSALRTGWYTSVITIELSNIKENKCNGTDAKVKLIKQELDKYKNAVTELQLLMQSGGPGSGGGGSGGGGSRFPPFLLGVGSAIASGVAVSKVLHLEGEVNKIKSALLSTNKAVVSLSNGVSVLTSKVLDLKNYIDKQLLPIVNKQSCSISNIETVIEFQQKNNRLLEITREFSVNAGVTTPVSTYMLTNSELLSLINDMPITNDQKKLMSNNVQIVRQQSYSIMSIIKEEVLAYVVQLPLYGVIDTPCWKLHTSPLCTTNTKEGSNICLTRTDRGWYCDNAGSVSFFPQAETCKVQSNRVFCDTMNSLTLPPEVNLCNVDIFNPKYDCKIMTSKTDVSSSVITSLGAIVSCYGKTKCTASNKNRGIIKTFSNGCDYVSNKGVDTVSVGNTLYYVNKQEGKSLYVKGEPIINFYDPLVFPSDEFDASISQVNEKINQSLAFIRKSDELL

SEQ ID NO: 46 - protein, 467 aa, synthetic construct
QNITEEFYQSTCSAVSKGYLSALRTGWYTSVITIELSNIKEPKCNGTDAKVKLIKQELDKYKNAVTELQLLMQSGGPGSGGGGSGGGGSRFPPFLLGVGSAIASGVAVSKVLHLEGEVNKIKSALLSTNKAVVSLSNGVSVLTSKVLDLKNYIDKQLLPIVNKQSCSISNIETVIEFQQKNNRLLEITREFSVNAGVTTPVSTYMLTNSELLSLINDMPITNDQKKLMSNNVPIVRQQSYSIMSIIKEEVLAYVVQLPLYGVIDTPCWKLHTSPLCTTNTKEGSNICLTRTDRGWYCDNAGSVSFFPQAETCKVQSNRVFCDTMNSLTLPSEVNLCNVDIFNPKYDCKIMTSKTDVSSSVITSLGAIVSCYGKTKCTASNKNRGIIKTFSNGCDYVSNKGVDTVSVGNTLYYVNKQEGKSLYVKGEPIINFYDPLVFPSDEFDASISQVNEKINQSLAFIRKSDELL

SEQ ID NO: 47 - protein, 467 aa, synthetic construct
QNITEEFYQSTCSAVSKGYLSALRTGWYTSVITIELSNIKEPKCNGTDAKVKLIKQELDKYKNAVTELQLLMQSGGPGSGGGGSGGGGSRFPPFLLGVGSAIASGVAVSKVLHLEGEVNKIKSALLSTNKAVVSLSNGVSVLTSKVLDLKNYIDKQLLPIVNKQSCSISNIETVIEFQQKNNRLLEITREFSVNAGVTTPVSTYMLTNSELLSLINDMPITNDQKKLMSNNVQIVRQQSYSIMSIIKEEVLAYVVQLPLYGVIDTPCWKLHTSPLCTTNTKEGSNICLTRTDRGWYCDNAGSVSFFPQAETCKVQSNRVFCDTMNSLTLPPEVNLCNVDIFNPKYDCKIMTSKTDVSSSVITSLGAIVSCYGKTKCTASNKNRGIIKTFSNGCDYVSNKGVDTVSVGNTLYYVNKQEGKSLYVKGEPIINFYDPLVFPSDEFDASISQVNEKINQSLAFIRKSDELL

SEQ ID NO: 48 - protein, 467 aa, synthetic construct
QNITEEFYQSTCSAVSKGYLSALRTGWYTSVITIELSNIKEPKCNGTDAKVKLIKQELDKYKNAVTELQLLMQSGGPGSGGGGSGGGGSRFLGFPLGVGSAIASGVAVSKVLHLEGEVNKIKSALLSTNKAVVSLSNGVSVLTSKVLDLKNYIDKQLLPIVNKQSCSISNIETVIEFQQKNNRLLEITREFSVNAGVTTPVSTYMLTNSELLSLINDMPITNDQKKLMSNNVPIVRQQSYSIMSIIKEEVLAYVVQLPLYGVIDTPCWKLHTSPLCTTNTKEGSNICLTRTDRGWYCDNAGSVSFFPQAETCKVQSNRVFCDTMNSLTLPPEVNLCNVDIFNPKYDCKIMTSKTDVSSSVITSLGAIVSCYGKTKCTASNKNRGIIKTFSNGCDYVSNKGVDTVSVGNTLYYVNKQEGKSLYVKGEPIINFYDPLVFPSDEFDASISQVNEKINQSLAFIRKSDELL

SEQ ID NO: 49 - protein, 467 aa, synthetic construct
QNITEEFYQSTCSAVSKGYLSALRTGWYTSVITIELSNIKENKCNGTDAKVKLIKQELDKYKNAVTELQLLMQSGGPGSGGGGSGGGGSRFPPFLLGVGSAIASGVAVSKVLHLEGEVNKIKSALLSTNKAVVSLSNGVSVLTSKVLDLKNYIDKQLLPIVNKQSCSISNIETVIEFQQKNNRLLEITREFSVNAGVTTPVSTYMLTNSELLSLINDMPITNDQKKLMSNNVPIVRQQSYSIMSIIKEEVLAYVVQLPLYGVIDTPCWKLHTSPLCTTNTKEGSNICLTRTDRGWYCDNAGSVSFFPQAETCKVQSNRVFCDTMNSLTLPPEVNLCNVDIFNPKYDCKIMTSKTDVSSSVITSLGAIVSCYGKTKCTASNKNRGIIKTFSNGCDYVSNKGVDTVSVGNTLYYVNKQEGKSLYVKGEPIINFYDPLVFPSDEFDASISQVNEKINQSLAFIRKSDELL

SEQ ID NO: 50 - protein, 467 aa, synthetic construct
QNITEEFYQSTCSAVSKGYLSALRTGWYTSVITIELSNIKEPKCNGTDAKVKLIKQELDKYKNAVTELQLLMQSGGPGSGGGGSGGGGSRFPPFLLGVGSAIASGVAVSKVLHLEGEVNKIKSALLSTNKAVVSLSNGVSVLTSKVLDLKNYIDKQLLPIVNKQSCSISNIETVIEFQQKNNRLLEITREFSVNAGVTTPVSTYMLTNSELLSLINDMPITNDQKKLMSNNVPIVRQQSYSIMSIIKEEVLAYVVQLPLYGVIDTPCWKLHTSPLCTTNTKEGSNICLTRTDRGWYCDNAGSVSFFPQAETCKVQSNRVFCDTMNSLTLPPEVNLCNVDIFNPKYDCKIMTSKTDVSSSVITSLGAIVSCYGKTKCTASNKNRGIIKTFSNGCDYVSNKGVDTVSVGNTLYYVNKQEGKSLYVKGEPIINFYDPLVFPSDEFDASISQVNEKINQSLAFIRKSDELL

SEQ ID NO: 51 - protein, 467 aa, synthetic construct
QNITEEFYQSTCSAVSKGYLSALRTGWYTSVITIELSNIKEPKCNGTDAKVKLIKQELDKYKNAVTELQLLMQSGGPGSGGGGSGGGGSRFPPFPLGVGSAIASGVAVSKVLHLEGEVNKIKSALLSTNKAVVSLSNGVSVLTSKVLDLKNYIDKQLLPIVNKQSCSISNIETVIEFQQKNNRLLEITREFSVNAGVTTPVSTYMLTNSELLSLINDMPITNDQKKLMSNNVPIVRQQSYSIMSIIKEEVLAYVVQLPLYGVIDTPCWKLHTSPLCTTNTKEGSNICLTRTDRGWYCDNAGSVSFFPQAETCKVQSNRVFCDTMNSLTLPPEVNLCNVDIFNPKYDCKIMTSKTDVSSSVITSLGAIVSCYGKTKCTASNKNRGIIKTFSNGCDYVSNKGVDTVSVGNTLYYVNKQEGKSLYVKGEPIINFYDPLVFPSDEFDASISQVNEKINQSLAFIRKSDELL

SEQ ID NO: 52 - protein, 467 aa, synthetic construct
QNITEEFYQSTCSAVSKGYLSALRTGWYTSVITIELSNIPENKCNGTDAKVKLIKQELDKYKNAVTELQLLMQSGGPGSGGGGSGGGGSRFLGFPLGVGSAIASGVAVSKVLHLEGEVNKIKSALLSTNKAVVSLSNGVSVLTSKVLDLKNYIDKQLLPIVNKQSCSISNIETVIEFQQKNNRLLEITREFSVNAGVTTPVSTYMLTNSELLSLINDMPITNDQKKLMSNNVPIVRQQSYSIMSIIKEEVLAYVVQLPLYGVIDTPCWKLHTSPLCTTNTKEGSNICLTRTDRGWYCDNAGSVSFFPQAETCKVQSNRVFCDTMNSLTLPPEVNLCNVDIFNPKYDCKIMTSKTDVSSSVITSLGAIVSCYGKTKCTASNKNRGIIKTFSNGCDYVSNKGVDTVSVGNTLYYVNKQEGKSLYVKGEPIINFYDPLVFPSDEFDASISQVNEKINQSLAFIRKSDELL

SEQ ID NO: 53 - protein, 467 aa, synthetic construct
QNITEEFYQSTCSAVSKGYLSALRTGWYTSVITIELSNIKENKCNGTPAKVKLIKQELDKYKNAVTELQLLMQSGGPGSGGGGSGGGGSRFLGFPLGVGSAIASGVAVSKVLHLEGEVNKIKSALLSTNKAVVSLSNGVSVLTSKVLDLKNYIDKQLLPIVNKQSCSISNIETVIEFQQKNNRLLEITREFSVNAGVTTPVSTYMLTNSELLSLINDMPITNDQKKLMSNNVPIVRQQSYSIMSIIKEEVLAYVVQLPLYGVIDTPCWKLHTSPLCTTNTKEGSNICLTRTDRGWYCDNAGSVSFFPQAETCKVQSNRVFCDTMNSLTLPPEVNLCNVDIFNPKYDCKIMTSKTDVSSSVITSLGAIVSCYGKTKCTASNKNRGIIKTFSNGCDYVSNKGVDTVSVGNTLYYVNKQEGKSLYVKGEPIINFYDPLVFPSDEFDASISQVNEKINQSLAFIRKSDELL

SEQ ID NO: 54 - protein, 467 aa, synthetic construct
QNITEEFYQSTCSAVSKGYLSALRTGWYTSVITIELSNIKENKCNGTDAKVKLIKQELDKYKNAVTELQLLMQSGGPGSGGGGSGGGGSRFLGFPLGVGSAIASGVAVSKVLHLEGEVNKIKSALLSTNKAVVSLSNGVSVLTSKVLDLKNYIDKQLLPIVNKQSCSIPNIETVIEFQQKNNRLLEITREFSVNAGVTTPVSTYMLTNSELLSLINDMPITNDQKKLMSNNVQIVRQQSYSIMSIIKEEVLAYVVQLPLYGVIDTPCWKLHTSPLCTTNTKEGSNICLTRTDRGWYCDNAGSVSFFPQAETCKVQSNRVFCDTMNSLTLPSEVNLCNVDIFNPKYDCKIMTSKTDVSSSVITSLGAIVSCYGKTKCTASNKNRGIIKTFSNGCDYVSNKGVDTVSVGNTLYYVNKQEGKSLYVKGEPIINFYDPLVFPSDEFDASISQVNEKINQSLAFIRKSDELL

SEQ ID NO: 55 - protein, 467 aa, synthetic construct
QNITEEFYQSTCSAVSKGYLSALRTGWYTSVITIELSNIKEPKCNGTDAKVKLIKQELDKYKNAVTELQLLMQSGGPGSGGGGSGGGGSRFLGFPLGVGSAIASGVAVSKVLHLEGEVNKIKSALLSTNKAVVSLSNGVSVLTSKVLDLKNYIDKQLLPIVNKQSCSIPNIETVIEFQQKNNRLLEITREFSVNAGVTTPVSTYMLTNSELLSLINDMPITNDQKKLMSNNVQIVRQQSYSIMSIIKEEVLAYVVQLPLYGVIDTPCWKLHTSPLCTTNTKEGSNICLTRTDRGWYCDNAGSVSFFPQAETCKVQSNRVFCDTMNSLTLPSEVNLCNVDIFNPKYDCKIMTSKTDVSSSVITSLGAIVSCYGKTKCTASNKNRGIIKTFSNGCDYVSNKGVDTVSVGNTLYYVNKQEGKSLYVKGEPIINFYDPLVFPSDEFDASISQVNEKINQSLAFIRKSDELL

SEQ ID NO: 56 - protein, 467 aa, synthetic construct
QNITEEFYQSTCSAVSKGYLSALRTGWYTSVITIELSNIKEPKCNGTDAKVKLIKQELDKYKNAVTELQLLMQSGGPGSGGGGSGGGGSRFLGFPLGVGSAIASGVAVSKVLHLEGEVNKIKSALLSTNKAVVSLSNGVSVLTSKVLDLKNYIDKQLLPIVNKQSCSIPNIETVIEFQQKNNRLLEITREFSVNAGVTTPVSTYMLTNSELLSLINDMPITNDQKKLMSNNVQIVRQQSYSIMSIIKEEVLAYVVQLPLYGVIDTPCWKLHTSPLCTTNTKEGSNICLTRTDRGWYCDNAGSVSFFPQAETCKVQSNRVFCDTMNSLTLPPEVNLCNVDIFNPKYDCKIMTSKTDVSSSVITSLGAIVSCYGKTKCTASNKNRGIIKTFSNGCDYVSNKGVDTVSVGNTLYYVNKQEGKSLYVKGEPIINFYDPLVFPSDEFDASISQVNEKINQSLAFIRKSDELL

SEQ ID NO: 57 - protein, 467 aa, synthetic construct
QNITEEFYQSTCSAVSKGYLSALRTGWYTSVITIELSNIKEPKCNGTDAKVKLIKQELDKYKNAVTELQLLMQSGGPGSGGGGSGGGGSRFLGFPLGVGSAIASGVAVSKVLHLEGEVNKIKSALLSTNKAVVSLSNGVSVLTSKVLDLKNYIDKQLLPIVNKQSCSIPNIETVIEFQQKNNRLLEITREFSVNAGVTTPVSTYMLTNSELLSLINDMPITNDQKKLMSNNVPIVRQQSYSIMSIIKEEVLAYVVQLPLYGVIDTPCWKLHTSPLCTTNTKEGSNICLTRTDRGWYCDNAGSVSFFPQAETCKVQSNRVFCDTMNSLTLPSEVNLCNVDIFNPKYDCKIMTSKTDVSSSVITSLGAIVSCYGKTKCTASNKNRGIIKTFSNGCDYVSNKGVDTVSVGNTLYYVNKQEGKSLYVKGEPIINFYDPLVFPSDEFDASISQVNEKINQSLAFIRKSDELL

SEQ ID NO: 58 - protein, 467 aa, synthetic construct
QNITEEFYQSTCSAVSKGYLSALRTGWYTSVITIELSNIKEPKCNGTDAKVKLIKQELDKYKNAVTELQLLMQSGGPGSGGGGSGGGGSRFPPFLLGVGSAIASGVAVSKVLHLEGEVNKIKSALLSTNKAVVSLSNGVSVLTSKVLDLKNYIDKQLLPIVNKQSCSIPNIETVIEFQQKNNRLLEITREFSVNAGVTTPVSTYMLTNSELLSLINDMPITNDQKKLMSNNVQIVRQQSYSIMSIIKEEVLAYVVQLPLYGVIDTPCWKLHTSPLCTTNTKEGSNICLTRTDRGWYCDNAGSVSFFPQAETCKVQSNRVFCDTMNSLTLPPEVNLCNVDIFNPKYDCKIMTSKTDVSSSVITSLGAIVSCYGKTKCTASNKNRGIIKTFSNGCDYVSNKGVDTVSVGNTLYYVNKQEGKSLYVKGEPIINFYDPLVFPSDEFDASISQVNEKINQSLAFIRKSDELL

SEQ ID NO: 59 - protein, 467 aa, synthetic construct
QNITEEFYQSTCSAVSKGYLSALRTGWYTSVITIELSNIKEPKCNGTDAKVKLIKQELDKYKNAVTELQLLMQSGGPGSGGGGSGGGGSRFPPFPLGVGSAIASGVAVSKVLHLEGEVNKIKSALLSTNKAVVSLSNGVSVLTSKVLDLKNYIDKQLLPIVNKQSCSIPNIETVIEFQQKNNRLLEITREFSVNAGVTTPVSTYMLTNSELLSLINDMPITNDQKKLMSNNVQIVRQQSYSIMSIIKEEVLAYVVQLPLYGVIDTPCWKLHTSPLCTTNTKEGSNICLTRTDRGWYCDNAGSVSFFPQAETCKVQSNRVFCDTMNSLTLPPEVNLCNVDIFNPKYDCKIMTSKTDVSSSVITSLGAIVSCYGKTKCTASNKNRGIIKTFSNGCDYVSNKGVDTVSVGNTLYYVNKQEGKSLYVKGEPIINFYDPLVFPSDEFDASISQVNEKINQSLAFIRKSDELL

SEQ ID NO: 60 - protein, 467 aa, synthetic construct
QNITEEFYQSTCSAVSKGYLSALRTGWYTSVITIELSNIKEPKCNGTDAKVKLIKQELDKYKNAVTELQLLMQSGGPGSGGGGSGGGGSRFLGFPLGVGSAIASGVAVSKVLHLEGEVNKIKSALLSTNKAVVSLSNGVSVLTSKVLDLKNYIDKQLLPIVNKQSCSIPNIETVIEFQQKNNRLLEITREFSVNAGVTTPVSTYMLTNSELLSLINDMPITNDQKKLMSNNVPIVRQQSYSIMSIIKEEVLAYVVQLPLYGVIDTPCWKLHTSPLCTTNTKEGSNICLTRTDRGWYCDNAGSVSFFPQAETCKVQSNRVFCDTMNSLTLPPEVNLCNVDIFNPKYDCKIMTSKTDVSSSVITSLGAIVSCYGKTKCTASNKNRGIIKTFSNGCDYVSNKGVDTVSVGNTLYYVNKQEGKSLYVKGEPIINFYDPLVFPSDEFDASISQVNEKINQSLAFIRKSDELL

SEQ ID NO: 61 - protein, 467 aa, synthetic construct
QNITEEFYQSTCSAVSKGYLSALRTGWYTSVITIELSNIKEPKCNGTDAKVKLIKQELDKYKNAVTELQLLMQSGGPGSGGGGSGGGGSRFPPFLLGVGSAIASGVAVSKVLHLEGEVNKIKSALLSTNKAVVSLSNGVSVLTSKVLDLKNYIDKQLLPIVNKQSCSIPNIETVIEFQQKNNRLLEITREFSVNAGVTTPVSTYMLTNSELLSLINDMPITNDQKKLMSNNVPIVRQQSYSIMSIIKEEVLAYVVQLPLYGVIDTPCWKLHTSPLCTTNTKEGSNICLTRTDRGWYCDNAGSVSFFPQAETCKVQSNRVFCDTMNSLTLPPEVNLCNVDIFNPKYDCKIMTSKTDVSSSVITSLGAIVSCYGKTKCTASNKNRGIIKTFSNGCDYVSNKGVDTVSVGNTLYYVNKQEGKSLYVKGEPIINFYDPLVFPSDEFDASISQVNEKINQSLAFIRKSDELL

SEQ ID NO: 62 - protein, 467 aa, synthetic construct
QNITEEFYQSTCSAVSKGYLSALRTGWYTSVITIELSNIKEPKCNGTDAKVKLIKQELDKYKNAVTELQLLMQSGGPGSGGGGSGGGGSRFPPFPLGVGSAIASGVAVSKVLHLEGEVNKIKSALLSTNKAVVSLSNGVSVLTSKVLDLKNYIDKQLLPIVNKQSCSIPNIETVIEFQQKNNRLLEITREFSVNAGVTTPVSTYMLTNSELLSLINDMPITNDQKKLMSNNVPIVRQQSYSIMSIIKEEVLAYVVQLPLYGVIDTPCWKLHTSPLCTTNTKEGSNICLTRTDRGWYCDNAGSVSFFPQAETCKVQSNRVFCDTMNSLTLPPEVNLCNVDIFNPKYDCKIMTSKTDVSSSVITSLGAIVSCYGKTKCTASNKNRGIIKTFSNGCDYVSNKGVDTVSVGNTLYYVNKQEGKSLYVKGEPIINFYDPLVFPSDEFDASISQVNEKINQSLAFIRKSDELL

SEQ ID NO: 63 - protein, 467 aa, synthetic construct
QNITEEFYQSTCSAVSKGYLSALRTGWYTSVITIELSNIKEPKCNGTDAKVKLIKQELDKYKNAVTELQLLMQSGGPGSGGGGSGGGGSRFLGFPLGVGSAIASGVAVSKVLHLPGEVNKIKSALLSTNKAVVSLSNGVSVLTSKVLDLKNYIDKQLLPIVNKQSCSISNIETVIEFQQKNNRLLEITREFSVNAGVTTPVSTYMLTNSELLSLINDMPITNDQKKLMSNNVPIVRQQSYSIMSIIKEEVLAYVVQLPLYGVIDTPCWKLHTSPLCTTNTKEGSNICLTRTDRGWYCDNAGSVSFFPQAETCKVQSNRVFCDTMNSLTLPPEVNLCNVDIFNPKYDCKIMTSKTDVSSSVITSLGAIVSCYGKTKCTASNKNRGIIKTFSNGCDYVSNKGVDTVSVGNTLYYVNKQEGKSLYVKGEPIINFYDPLVFPSDEFDASISQVNEKINQSLAFIRKSDELL

SEQ ID NO: 64 - protein, 467 aa, synthetic construct
QNITEEFYQSTCSAVSKGYLSALRTGWYTSVITIELSNIKEPKCNGTDAKVKLIKQELDKYKNAVTELQLLMQSGGPGSGGGGSGGGGSRFPPFLLGVGSAIASGVAVSKVLHLPGEVNKIKSALLSTNKAVVSLSNGVSVLTSKVLDLKNYIDKQLLPIVNKQSCSISNIETVIEFQQKNNRLLEITREFSVNAGVTTPVSTYMLTNSELLSLINDMPITNDQKKLMSNNVPIVRQQSYSIMSIIKEEVLAYVVQLPLYGVIDTPCWKLHTSPLCTTNTKEGSNICLTRTDRGWYCDNAGSVSFFPQAETCKVQSNRVFCDTMNSLTLPPEVNLCNVDIFNPKYDCKIMTSKTDVSSSVITSLGAIVSCYGKTKCTASNKNRGIIKTFSNGCDYVSNKGVDTVSVGNTLYYVNKQEGKSLYVKGEPIINFYDPLVFPSDEFDASISQVNEKINQSLAFIRKSDELL

SEQ ID NO: 65 - protein, 467 aa, synthetic construct
QNITEEFYQSTCSAVSKGYLSALRTGWYTSVITIELSNIKEPKCNGTDAKVKLIKQELDKYKNAVTELQLLMQSGGPGSGGGGSGGGGSRFPPFPLGVGSAIASGVAVSKVLHLPGEVNKIKSALLSTNKAVVSLSNGVSVLTSKVLDLKNYIDKQLLPIVNKQSCSISNIETVIEFQQKNNRLLEITREFSVNAGVTTPVSTYMLTNSELLSLINDMPITNDQKKLMSNNVPIVRQQSYSIMSIIKEEVLAYVVQLPLYGVIDTPCWKLHTSPLCTTNTKEGSNICLTRTDRGWYCDNAGSVSFFPQAETCKVQSNRVFCDTMNSLTLPPEVNLCNVDIFNPKYDCKIMTSKTDVSSSVITSLGAIVSCYGKTKCTASNKNRGIIKTFSNGCDYVSNKGVDTVSVGNTLYYVNKQEGKSLYVKGEPIINFYDPLVFPSDEFDASISQVNEKINQSLAFIRKSDELL

SEQ ID NO: 66 - protein, 467 aa, synthetic construct
QNITEEFYQSTCSAVSKGYLSALRTGWYTSVITIELSNIKEPKCNGTDAKVKLIKQELDKYKNAVTELQLLMQSGGPGSGGGGSGGGGSRFLGFPLGVGSAIASGVAVSKVLHLPGEVNKIKSALLSTNKAVVSLSNGVSVLTSKVLDLKNYIDKQLLPIVNKQSCSIPNIETVIEFQQKNNRLLEITREFSVNAGVTTPVSTYMLTNSELLSLINDMPITNDQKKLMSNNVPIVRQQSYSIMSIIKEEVLAYVVQLPLYGVIDTPCWKLHTSPLCTTNTKEGSNICLTRTDRGWYCDNAGSVSFFPQAETCKVQSNRVFCDTMNSLTLPPEVNLCNVDIFNPKYDCKIMTSKTDVSSSVITSLGAIVSCYGKTKCTASNKNRGIIKTFSNGCDYVSNKGVDTVSVGNTLYYVNKQEGKSLYVKGEPIINFYDPLVFPSDEFDASISQVNEKINQSLAFIRKSDELL

SEQ ID NO: 67 - protein, 467 aa, synthetic construct
QNITEEFYQSTCSAVSKGYLSALRTGWYTSVITIELSNIKEPKCNGTDAKVKLIKQELDKYKNAVTELQLLMQSGGPGSGGGGSGGGGSRFPPFLLGVGSAIASGVAVSKVLHLPGEVNKIKSALLSTNKAVVSLSNGVSVLTSKVLDLKNYIDKQLLPIVNKQSCSIPNIETVIEFQQKNNRLLEITREFSVNAGVTTPVSTYMLTNSELLSLINDMPITNDQKKLMSNNVPIVRQQSYSIMSIIKEEVLAYVVQLPLYGVIDTPCWKLHTSPLCTTNTKEGSNICLTRTDRGWYCDNAGSVSFFPQAETCKVQSNRVFCDTMNSLTLPPEVNLCNVDIFNPKYDCKIMTSKTDVSSSVITSLGAIVSCYGKTKCTASNKNRGIIKTFSNGCDYVSNKGVDTVSVGNTLYYVNKQEGKSLYVKGEPIINFYDPLVFPSDEFDASISQVNEKINQSLAFIRKSDELL

SEQ ID NO: 68 - protein, 467 aa, synthetic construct
QNITEEFYQSTCSAVSKGYLSALRTGWYTSVITIELSNIKEPKCNGTDAKVKLIKQELDKYKNAVTELQLLMQSGGPGSGGGGSGGGGSRFPPFPLGVGSAIASGVAVSKVLHLPGEVNKIKSALLSTNKAVVSLSNGVSVLTSKVLDLKNYIDKQLLPIVNKQSCSIPNIETVIEFQQKNNRLLEITREFSVNAGVTTPVSTYMLTNSELLSLINDMPITNDQKKLMSNNVPIVRQQSYSIMSIIKEEVLAYVVQLPLYGVIDTPCWKLHTSPLCTTNTKEGSNICLTRTDRGWYCDNAGSVSFFPQAETCKVQSNRVFCDTMNSLTLPPEVNLCNVDIFNPKYDCKIMTSKTDVSSSVITSLGAIVSCYGKTKCTASNKNRGIIKTFSNGCDYVSNKGVDTVSVGNTLYYVNKQEGKSLYVKGEPIINFYDPLVFPSDEFDASISQVNEKINQSLAFIRKSDELL

SEQ ID NO: 69 - protein, 467 aa, synthetic construct
QNITEEFYQSTCSAVSKGYLSALRTGWYTSVITIELSNIKEPKCNGTDAKVKLIKQELDKYKNAVTELQLLMQSGGPGSGGGGSGGGGSRFLGFPLGVGSAIASGVAVSKVLHLPGEVNKIKSALLSTNKAVVSLSNGVSVLTSKVLDLKNYIDKQLLPIVNKQSCSISNIETVIEFQQKNNRLLEITREFSVNAGVTTPVSTYMLTNSELLSLINDMPITNDQKKLMSNNVPIVRQQSYSIMSIIKEEVLAYVVQLPLYGVIDTPCWKLHTSPLCTTNTKEGSNICLTRTDRGWYCDNAGSVSFFPQAETCKVQSNRVFCDTMNSLTLPSEVNLCNVDIFNPKYDCKIMTSKTDVSSSVITSLGAIVSCYGKTKCTASNKNRGIIKTFSNGCDYVSNKGVDTVSVGNTLYYVNKQEGKSLYVKGEPIINFYDPLVFPSDEFDASISQVNEKINQSLAFIRKSDELL

SEQ ID NO: 70 - protein, 467 aa, synthetic construct
QNITEEFYQSTCSAVSKGYLSALRTGWYTSVITIELSNIKEPKCNGTDAKVKLIKQELDKYKNAVTELQLLMQSGGPGSGGGGSGGGGSRFLGFPLGVGSAIASGVAVSKVLHLPGEVNKIKSALLSTNKAVVSLSNGVSVLTSKVLDLKNYIDKQLLPIVNKQSCSISNIETVIEFQQKNNRLLEITREFSVNAGVTTPVSTYMLTNSELLSLINDMPITNDQKKLMSNNVQIVRQQSYSIMSIIKEEVLAYVVQLPLYGVIDTPCWKLHTSPLCTTNTKEGSNICLTRTDRGWYCDNAGSVSFFPQAETCKVQSNRVFCDTMNSLTLPPEVNLCNVDIFNPKYDCKIMTSKTDVSSSVITSLGAIVSCYGKTKCTASNKNRGIIKTFSNGCDYVSNKGVDTVSVGNTLYYVNKQEGKSLYVKGEPIINFYDPLVFPSDEFDASISQVNEKINQSLAFIRKSDELL

SEQ ID NO: 71 - protein, 467 aa, synthetic construct
QNITEEFYQSTCSAVSKGYLSALRTGWYTSVITIELSNIKEPKCNGTDAKVKLIKQELDKYKNAVTELQLLMQSGGPGSGGGGSGGGGSRFLGFPLGVGSAIASGVAVSKVLHLPGEVNKIKSALLSTNKAVVSLSNGVSVLTSKVLDLKNYIDKQLLPIVNKQSCSIPNIETVIEFQQKNNRLLEITREFSVNAGVTTPVSTYMLTNSELLSLINDMPITNDQKKLMSNNVQIVRQQSYSIMSIIKEEVLAYVVQLPLYGVIDTPCWKLHTSPLCTTNTKEGSNICLTRTDRGWYCDNAGSVSFFPQAETCKVQSNRVFCDTMNSLTLPSEVNLCNVDIFNPKYDCKIMTSKTDVSSSVITSLGAIVSCYGKTKCTASNKNRGIIKTFSNGCDYVSNKGVDTVSVGNTLYYVNKQEGKSLYVKGEPIINFYDPLVFPSDEFDASISQVNEKINQSLAFIRKSDELL

SEQ ID NO: 72 - protein, 467 aa, synthetic construct
QNITEEFYQSTCSAVSKGYLSALRTGWYTSVITIELSNIKEPKCNGTDAKVKLIKQELDKYKNAVTELQLLMQSGGPGSGGGGSGGGGSRFLGFPLGVGSAIASGVAVSKVLHLPGEVNKIKSALLSTNKAVVSLSNGVSVLTSKVLDLKNYIDKQLLPIVNKQSCSIPNIETVIEFQQKNNRLLEITREFSVNAGVTTPVSTYMLTNSELLSLINDMPITNDQKKLMSNNVQIVRQQSYSIMSIIKEEVLAYVVQLPLYGVIDTPCWKLHTSPLCTTNTKEGSNICLTRTDRGWYCDNAGSVSFFPQAETCKVQSNRVFCDTMNSLTLPPEVNLCNVDIFNPKYDCKIMTSKTDVSSSVITSLGAIVSCYGKTKCTASNKNRGIIKTFSNGCDYVSNKGVDTVSVGNTLYYVNKQEGKSLYVKGEPIINFYDPLVFPSDEFDASISQVNEKINQSLAFIRKSDELL

SEQ ID NO: 73 - protein, 467 aa, synthetic construct
QNITEEFYQSTCSAVSKGYLSALRTGWYTSVITIELSNIKEPKCNGTDAKVKLIKQELDKYKNAVTELQLLMQSGGPGSGGGGSGGGGSRFPPFLLGVGSAIASGVAVSKVLHLPGEVNKIKSALLSTNKAVVSLSNGVSVLTSKVLDLKNYIDKQLLPIVNKQSCSIPNIETVIEFQQKNNRLLEITREFSVNAGVTTPVSTYMLTNSELLSLINDMPITNDQKKLMSNNVQIVRQQSYSIMSIIKEEVLAYVVQLPLYGVIDTPCWKLHTSPLCTTNTKEGSNICLTRTDRGWYCDNAGSVSFFPQAETCKVQSNRVFCDTMNSLTLPPEVNLCNVDIFNPKYDCKIMTSKTDVSSSVITSLGAIVSCYGKTKCTASNKNRGIIKTFSNGCDYVSNKGVDTVSVGNTLYYVNKQEGKSLYVKGEPIINFYDPLVFPSDEFDASISQVNEKINQSLAFIRKSDELL

SEQ ID NO: 74 - protein, 467 aa, synthetic construct
QNITEEFYQSTCSAVSKGYLSALRTGWYTSVITIELSNIKEPKCNGTDAKVKLIKQELDKYKNAVTELQLLMQSGGPGSGGGGSGGGGSRFPPFPLGVGSAIASGVAVSKVLHLPGEVNKIKSALLSTNKAVVSLSNGVSVLTSKVLDLKNYIDKQLLPIVNKQSCSIPNIETVIEFQQKNNRLLEITREFSVNAGVTTPVSTYMLTNSELLSLINDMPITNDQKKLMSNNVQIVRQQSYSIMSIIKEEVLAYVVQLPLYGVIDTPCWKLHTSPLCTTNTKEGSNICLTRTDRGWYCDNAGSVSFFPQAETCKVQSNRVFCDTMNSLTLPPEVNLCNVDIFNPKYDCKIMTSKTDVSSSVITSLGAIVSCYGKTKCTASNKNRGIIKTFSNGCDYVSNKGVDTVSVGNTLYYVNKQEGKSLYVKGEPIINFYDPLVFPSDEFDASISQVNEKINQSLAFIRKSDELL

SEQ ID NO: 75 - protein, 467 aa, synthetic construct
QNITEEFYQSTCSAVSKGYLSALRTGWYTSVITIELSNIKEPKCNGTDAKVKLIKQELDKYKNAVTELQLLMQSGGPGSGGGGSGGGGSRFLGFPLGVGSAIASGVAVSKVLHLEGEVNKIKSALLSTNKAVVSLSNGVSVLTSKVLDLKNYIDKQLLPIVNKQSCSPPNIETVIEFQQKNNRLLEITREFSVNAGVTTPVSTYMLTNSELLSLINDMPITNDQKKLMSNNVPIVRQQSYSIMSIIKEEVLAYVVQLPLYGVIDTPCWKLHTSPLCTTNTKEGSNICLTRTDRGWYCDNAGSVSFFPQAETCKVQSNRVFCDTMNSLTLPPEVNLCNVDIFNPKYDCKIMTSKTDVSSSVITSLGAIVSCYGKTKCTASNKNRGIIKTFSNGCDYVSNKGVDTVSVGNTLYYVNKQEGKSLYVKGEPIINFYDPLVFPSDEFDASISQVNEKINQSLAFIRKSDELL

SEQ ID NO: 76 - protein, 467 aa, synthetic construct
QNITEEFYQSTCSAVSKGYLSALRTGWYTSVITIELSNIKEPKCNGTDAKVKLIKQELDKYKNAVTELQLLMQSGGPGSGGGGSGGGGSRFPPFLLGVGSAIASGVAVSKVLHLPGEVNKIKSALLSTNKAVVSLSNGVSVLTSKVLDLKNYIDKQLLPIVNKQSCSIPPIETVIEFQQKNNRLLEITREFSVNAGVTTPVSTYMLTNSELLSLINDMPITNDQKKLMSNNVPIVRQQSYSIMSIIKEEVLAYVVQLPLYGVIDTPCWKLHTSPLCTTNTKEGSNICLTRTDRGWYCDNAGSVSFFPQAETCKVQSNRVFCDTMNSLTLPPEVNLCNVDIFNPKYDCKIMTSKTDVSSSVITSLGAIVSCYGKTKCTASNKNRGIIKTFSNGCDYVSNKGVDTVSVGNTLYYVNKQEGKSLYVKGEPIINFYDPLVFPSDEFDASISQVNEKINQSLAFIRKSDELL

SEQ ID NO: 77 - protein, 467 aa, synthetic construct
QNITEEFYQSTCSAVSKGYLSALRTGWYTSVITIELSNIKEPKCNGTDAKVKLIKQELDKYKNAVTELQLLMQSGGPGSGGGGSGGGGSRFLGFPLGVGSAIASGVAVSKVLHLEGEVNKIKSALLSTNKAVVSLSNGVSVLTSKVLDLKNYIDKQLLPIVNKPSCSISNIETVIEFQQKNNRLLEITREFSVNAGVTTPVSTYMLTNSELLSLINDMPITNDQKKLMSNNVPIVRQQSYSIMSIIKEEVLAYVVQLPLYGVIDTPCWKLHTSPLCTTNTKEGSNICLTRTDRGWYCDNAGSVSFFPQAETCKVQSNRVFCDTMNSLTLPPEVNLCNVDIFNPKYDCKIMTSKTDVSSSVITSLGAIVSCYGKTKCTASNKNRGIIKTFSNGCDYVSNKGVDTVSVGNTLYYVNKQEGKSLYVKGEPIINFYDPLVFPSDEFDASISQVNEKINQSLAFIRKSDELL

SEQ ID NO: 78 - protein, 467 aa, synthetic construct
QNITEEFYQSTCSAVSKGYLSALRTGWYTSVITIELSNIKEPKCNGTDAKVKLIKQELDKYKNAVTELQLLMQSGGPGSGGGGSGGGGSRFPPFLLGVGSAIASGVAVSKVLHLEGEVNKIKSALLSTNKAVVSLSNGVSVLTSKVLDLKNYIDKQLLPIVNKPSCSIPNIETVIEFQQKNNRLLEITREFSVNAGVTTPVSTYMLTNSELLSLINDMPITNDQKKLMSNNVQIVRQQSYSIMSIIKEEVLAYVVQLPLYGVIDTPCWKLHTSPLCTTNTKEGSNICLTRTDRGWYCDNAGSVSFFPQAETCKVQSNRVFCDTMNSLTLPPEVNLCNVDIFNPKYDCKIMTSKTDVSSSVITSLGAIVSCYGKTKCTASNKNRGIIKTFSNGCDYVSNKGVDTVSVGNTLYYVNKQEGKSLYVKGEPIINFYDPLVFPSDEFDASISQVNEKINQSLAFIRKSDELL

SEQ ID NO: 79 - protein, 467 aa, synthetic construct
QNITEEFYQSTCSAVSKGYLSALRTGWYTSVITIELSNIKEPKCNGTDAKVKLIKQELDKYKNAVTELQLLMQSGGPGSGGGGSGGGGSRFPPFPLGVGSAIASGVAVSKVLHLPGEVNKIKSALLSTNKAVVSLSNGVSVLTSKVLDLKNYIDKQLLPIVNKPSCSIPNIETVIEFQQKNNRLLEITREFSVNAGVTTPVSTYMLTNSELLSLINDMPITNDQKKLMSNNVPIVRQQSYSIMSIIKEEVLAYVVQLPLYGVIDTPCWKLHTSPLCTTNTKEGSNICLTRTDRGWYCDNAGSVSFFPQAETCKVQSNRVFCDTMNSLTLPPEVNLCNVDIFNPKYDCKIMTSKTDVSSSVITSLGAIVSCYGKTKCTASNKNRGIIKTFSNGCDYVSNKGVDTVSVGNTLYYVNKQEGKSLYVKGEPIINFYDPLVFPSDEFDASISQVNEKINQSLAFIRKSDELL

SEQ ID NO: 80 - protein, 467 aa, synthetic construct
QNITEEFYQSTCSAVSKGYLSALRTGWYTSVITIELSNIKEPKCNGTDAKVKLIKQELDKYKNAVTELQLLMQSGGGGSGGGGSGGGGSRFPPFPLGVGSAIASGVAVSKVLHLEGEVNKIKSALLSTNKAVVSLSNGVSVLTSKVLDLKNYIDKQLLPIVNKQSCSISNIETVIEFQQKNNRLLEITREFSVNAGVTTPVSTYMLTNSELLSLINDMPITNDQKKLMSNNVPIVRQQSYSIMSIIKEEVLAYVVQLPLYGVIDTPCWKLHTSPLCTTNTKEGSNICLTRTDRGWYCDNAGSVSFFPQAETCKVQSNRVFCDTMNSLTLPPEVNLCNVDIFNPKYDCKIMTSKTDVSSSVITSLGAIVSCYGKTKCTASNKNRGIIKTFSNGCDYVSNKGVDTVSVGNTLYYVNKQEGKSLYVKGEPIINFYDPLVFPSDEFDASISQVNEKINQSLAFIRKSDELL

SEQ ID NO: 81 - protein, 467 aa, synthetic construct
QNITEEFYQSTCSAVSKGYLSALRTGWYTSVITIELSNIKEPKCNGTDAKVKLIKQELDKYKNAVTELQLLMQSGGGGSGGGGSGGGGSRFPPFPLGVGSAIASGVAVSKVLHLEGEVNKIKSALLSTNKAVVSLSNGVSVLTSKVLDLKNYIDKQLLPIVNKQSCSIPNIETVIEFQQKNNRLLEITREFSVNAGVTTPVSTYMLTNSELLSLINDMPITNDQKKLMSNNVPIVRQQSYSIMSIIKEEVLAYVVQLPLYGVIDTPCWKLHTSPLCTTNTKEGSNICLTRTDRGWYCDNAGSVSFFPQAETCKVQSNRVFCDTMNSLTLPPEVNLCNVDIFNPKYDCKIMTSKTDVSSSVITSLGAIVSCYGKTKCTASNKNRGIIKTFSNGCDYVSNKGVDTVSVGNTLYYVNKQEGKSLYVKGEPIINFYDPLVFPSDEFDASISQVNEKINQSLAFIRKSDELL

SEQ ID NO: 82 - protein, 467 aa, synthetic construct
QNITEEFYQSTCSAVSKGYLSALRTGWYTSVITIELSNIKENKCNGTDAKVKLIKQELDKYKNAVTELQLLMQSGGGGSGGGGSGGGGSRFLGFPLGVGSAIASGVAVSKVLHLEGEVNKIKSALLSTNKAVVSLSNGVSVLTSKVLDLKNYIDKQLLPIVNKQSCSIPNIETVIEFQQKNNRLLEITREFSVNAGVTTPVSTYMLTNSELLSLINDMPITNDQKKLMSNNVQIVRQQSYSIMSIIKEEVLAYVVQLPLYGVIDTPCWKLHTSPLCTTNTKEGSNICLTRTDRGWYCDNAGSVSFFPQAETCKVQSNRVFCDTMNSLTLPSEVNLCNVDIFNPKYDCKIMTSKTDVSSSVITSLGAIVSCYGKTKCTASNKNRGIIKTFSNGCDYVSNKGVDTVSVGNTLYYVNKQEGKSLYVKGEPIINFYDPLVFPSDEFDASISQVNEKINQSLAFIRKSDELL

SEQ ID NO: 83 - protein, 467 aa, synthetic construct
QNITEEFYQSTCSAVSKGYLSALRTGWYTSVITIELSNIKEPKCNGTDAKVKLIKQELDKYKNAVTELQLLMQSGGGGSGGGGSGGGGSRFPPFPLGVGSAIASGVAVSKVLHLEGEVNKIKSALLSTNKAVVSLSNGVSVLTSKVLDLKNYIDKQLLPIVNKQSCSIPNIETVIEFQQKNNRLLEITREFSVNAGVTTPVSTYMLTNSELLSLINDMPITNDQKKLMSNNVQIVRQQSYSIMSIIKEEVLAYVVQLPLYGVIDTPCWKLHTSPLCTTNTKEGSNICLTRTDRGWYCDNAGSVSFFPQAETCKVQSNRVFCDTMNSLTLPPEVNLCNVDIFNPKYDCKIMTSKTDVSSSVITSLGAIVSCYGKTKCTASNKNRGIIKTFSNGCDYVSNKGVDTVSVGNTLYYVNKQEGKSLYVKGEPIINFYDPLVFPSDEFDASISQVNEKINQSLAFIRKSDELL

SEQ ID NO: 84 - protein, 467 aa, synthetic construct
QNITEEFYQSTCSAVSKGYLSALRTGWYTSVITIELSNIKEPKCNGTDAKVKLIKQELDKYKNAVTELQLLMQSGGGGSPGGGSGGGGSRFLGFPLGVGSAIASGVAVSKVLHLEGEVNKIKSALLSTNKAVVSLSNGVSVLTSKVLDLKNYIDKQLLPIVNKQSCSISNIETVIEFQQKNNRLLEITREFSVNAGVTTPVSTYMLTNSELLSLINDMPITNDQKKLMSNNVPIVRQQSYSIMSIIKEEVLAYVVQLPLYGVIDTPCWKLHTSPLCTTNTKEGSNICLTRTDRGWYCDNAGSVSFFPQAETCKVQSNRVFCDTMNSLTLPPEVNLCNVDIFNPKYDCKIMTSKTDVSSSVITSLGAIVSCYGKTKCTASNKNRGIIKTFSNGCDYVSNKGVDTVSVGNTLYYVNKQEGKSLYVKGEPIINFYDPLVFPSDEFDASISQVNEKINQSLAFIRKSDELL

SEQ ID NO: 85 - protein, 467 aa, synthetic construct
QNITEEFYQSTCSAVSKGYLSALRTGWYTSVITIELSNIKEPKCNGTDAKVKLIKQELDKYKNAVTELQLLMQSGGGGPGGGGSGGGGSRFPPFLLGVGSAIASGVAVSKVLHLEGEVNKIKSALLSTNKAVVSLSNGVSVLTSKVLDLKNYIDKQLLPIVNKQSCSISNIETVIEFQQKNNRLLEITREFSVNAGVTTPVSTYMLTNSELLSLINDMPITNDQKKLMSNNVPIVRQQSYSIMSIIKEEVLAYVVQLPLYGVIDTPCWKLHTSPLCTTNTKEGSNICLTRTDRGWYCDNAGSVSFFPQAETCKVQSNRVFCDTMNSLTLPPEVNLCNVDIFNPKYDCKIMTSKTDVSSSVITSLGAIVSCYGKTKCTASNKNRGIIKTFSNGCDYVSNKGVDTVSVGNTLYYVNKQEGKSLYVKGEPIINFYDPLVFPSDEFDASISQVNEKINQSLAFIRKSDELL

SEQ ID NO: 86 - protein, 467 aa, synthetic construct
QNITEEFYQSTCSAVSKGYLSALRTGWYTSVITIELSNIKEPKCNGTDAKVKLIKQELDKYKNAVTELQLLMQSGGGGSGGGPSGGGGSRFPPFPLGVGSAIASGVAVSKVLHLEGEVNKIKSALLSTNKAVVSLSNGVSVLTSKVLDLKNYIDKQLLPIVNKQSCSISNIETVIEFQQKNNRLLEITREFSVNAGVTTPVSTYMLTNSELLSLINDMPITNDQKKLMSNNVPIVRQQSYSIMSIIKEEVLAYVVQLPLYGVIDTPCWKLHTSPLCTTNTKEGSNICLTRTDRGWYCDNAGSVSFFPQAETCKVQSNRVFCDTMNSLTLPPEVNLCNVDIFNPKYDCKIMTSKTDVSSSVITSLGAIVSCYGKTKCTASNKNRGIIKTFSNGCDYVSNKGVDTVSVGNTLYYVNKQEGKSLYVKGEPIINFYDPLVFPSDEFDASISQVNEKINQSLAFIRKSDELL

SEQ ID NO: 87 - protein, 488 aa, synthetic construct
QNITEEFYQSTCSAVSKGYLSALRTGWYTSVITIELSNIKEPKCNGTDAKVKLIKQELDKYKNAVTELQLLMQSTPATNNRARRELPRFMNYTLNNAKKTNVTLSKKRKRRFLGFLLGVGSAIASGVAVSKVLHLPGEVNKIKSALLSTNKAVVSLSNGVSVLTSKVLDLKNYIDKQLLPIVNKQSCSISNIETVIEFQQKNNRLLEITREFSVNAGVTTPVSTYMLTNSELLSLINDMPITNDQKKLMSNNVPIVRQQSYSIMSIIKEEVLAYVVQLPLYGVIDTPCWKLHTSPLCTTNTKEGSNICLTRTDRGWYCDNAGSVSFFPQAETCKVQSNRVFCDTMNSLTLPPEVNLCNVDIFNPKYDCKIMTSKTDVSSSVITSLGAIVSCYGKTKCTASNKNRGIIKTFSNGCDYVSNKGVDTVSVGNTLYYVNKQEGKSLYVKGEPIINFYDPLVFPSDEFDASISQVNEKINQSLAFIRKSDELL

SEQ ID NO: 88 - protein, 488 aa, synthetic construct
QNITEEFYQSTCSAVSKGYLSALRTGWYTSVITIELSNIKEPKCNGTDAKVKLIKQELDKYKNAVTELQLLMQSTPATNNRARRELPRFMNYTLNNAKKTNVTLSKKRKRRFLGFLLGVGSAIASGVAVSKVLHLPGEVNKIKSALLSTNKAVVSLSNGVSVLTSKVLDLKNYIDKQLLPIVNKQSCSIPNIETVIEFQQKNNRLLEITREFSVNAGVTTPVSTYMLTNSELLSLINDMPITNDQKKLMSNNVPIVRQQSYSIMSIIKEEVLAYVVQLPLYGVIDTPCWKLHTSPLCTTNTKEGSNICLTRTDRGWYCDNAGSVSFFPQAETCKVQSNRVFCDTMNSLTLPPEVNLCNVDIFNPKYDCKIMTSKTDVSSSVITSLGAIVSCYGKTKCTASNKNRGIIKTFSNGCDYVSNKGVDTVSVGNTLYYVNKQEGKSLYVKGEPIINFYDPLVFPSDEFDASISQVNEKINQSLAFIRKSDELL

SEQ ID NO: 89 - protein, 488 aa, synthetic construct
QNITEEFYQSTCSAVSKGYLSALRTGWYTSVITIELSNIKEPKCNGTDAKVKLIKQELDKYKNAVTELQLLMQSTPATNNRARRELPRFMNYTLNNAKKTNVTLSKKRKRRFLGFPLGVGSAIASGVAVSKVLHLPGEVNKIKSALLSTNKAVVSLSNGVSVLTSKVLDLKNYIDKQLLPIVNKQSCSIPNIETVIEFQQKNNRLLEITREFSVNAGVTTPVSTYMLTNSELLSLINDMPITNDQKKLMSNNVPIVRQQSYSIMSIIKEEVLAYVVQLPLYGVIDTPCWKLHTSPLCTTNTKEGSNICLTRTDRGWYCDNAGSVSFFPQAETCKVQSNRVFCDTMNSLTLPPEVNLCNVDIFNPKYDCKIMTSKTDVSSSVITSLGAIVSCYGKTKCTASNKNRGIIKTFSNGCDYVSNKGVDTVSVGNTLYYVNKQEGKSLYVKGEPIINFYDPLVFPSDEFDASISQVNEKINQSLAFIRKSDELL

SEQ ID NO: 90 - protein, 488 aa, synthetic construct
QNITEEFYQSTCSAVSKGYLSALRTGWYTSVITIELSNIKEPKCNGTDAKVKLIKQELDKYKNAVTELQLLMQSTPATNNGSASELPRFMNYTLNNAKKTNVTLSKKGKGRFLGFLLGVGSAIASGVAVSKVLHLPGEVNKIKSALLSTNKAVVSLSNGVSVLTSKVLDLKNYIDKQLLPIVNKQSCSISNIETVIEFQQKNNRLLEITREFSVNAGVTTPVSTYMLTNSELLSLINDMPITNDQKKLMSNNVPIVRQQSYSIMSIIKEEVLAYVVQLPLYGVIDTPCWKLHTSPLCTTNTKEGSNICLTRTDRGWYCDNAGSVSFFPQAETCKVQSNRVFCDTMNSLTLPPEVNLCNVDIFNPKYDCKIMTSKTDVSSSVITSLGAIVSCYGKTKCTASNKNRGIIKTFSNGCDYVSNKGVDTVSVGNTLYYVNKQEGKSLYVKGEPIINFYDPLVFPSDEFDASISQVNEKINQSLAFIRKSDELL

SEQ ID NO: 91 - protein, 488 aa, synthetic construct
QNITEEFYQSTCSAVSKGYLSALRTGWYTSVITIELSNIKEPKCNGTDAKVKLIKQELDKYKNAVTELQLLMQSTPATNNGSASELPRFMNYTLNNAKKTNVTLSKKGKGRFLGFLLGVGSAIASGVAVSKVLHLPGEVNKIKSALLSTNKAVVSLSNGVSVLTSKVLDLKNYIDKQLLPIVNKQSCSIPNIETVIEFQQKNNRLLEITREFSVNAGVTTPVSTYMLTNSELLSLINDMPITNDQKKLMSNNVPIVRQQSYSIMSIIKEEVLAYVVQLPLYGVIDTPCWKLHTSPLCTTNTKEGSNICLTRTDRGWYCDNAGSVSFFPQAETCKVQSNRVFCDTMNSLTLPPEVNLCNVDIFNPKYDCKIMTSKTDVSSSVITSLGAIVSCYGKTKCTASNKNRGIIKTFSNGCDYVSNKGVDTVSVGNTLYYVNKQEGKSLYVKGEPIINFYDPLVFPSDEFDASISQVNEKINQSLAFIRKSDELL

SEQ ID NO: 92 - protein, 488 aa, synthetic construct
QNITEEFYQSTCSAVSKGYLSALRTGWYTSVITIELSNIKEPKCNGTDAKVKLIKQELDKYKNAVTELQLLMQSTPATNNGSASELPRFMNYTLNNAKKTNVTLSKKGKGRFLGFPLGVGSAIASGVAVSKVLHLPGEVNKIKSALLSTNKAVVSLSNGVSVLTSKVLDLKNYIDKQLLPIVNKQSCSIPNIETVIEFQQKNNRLLEITREFSVNAGVTTPVSTYMLTNSELLSLINDMPITNDQKKLMSNNVPIVRQQSYSIMSIIKEEVLAYVVQLPLYGVIDTPCWKLHTSPLCTTNTKEGSNICLTRTDRGWYCDNAGSVSFFPQAETCKVQSNRVFCDTMNSLTLPPEVNLCNVDIFNPKYDCKIMTSKTDVSSSVITSLGAIVSCYGKTKCTASNKNRGIIKTFSNGCDYVSNKGVDTVSVGNTLYYVNKQEGKSLYVKGEPIINFYDPLVFPSDEFDASISQVNEKINQSLAFIRKSDELL

SEQ ID NO: 93 - protein, 449 aa, synthetic construct
QNITEEFYQSTCSAVSKGYLSALRTGWYTSVITIELSNIKEPKCNGTDAKVKLIKQELDKYKNAVTELQLLMQSTPATGSGSAIASGVAVSKVLHLEGEVNKIKSALLSTNKAVVSLSNGVSVLTSKVLDLKNYIDKQLLPIVNKQSCSISNIETVIEFQQKNNRLLEITREFSVNAGVTTPVSTYMLTNSELLSLINDMPITNDQKKLMSNNVPIVRQQSYSIMSIIKEEVLAYVVQLPLYGVIDTPCWKLHTSPLCTTNTKEGSNICLTRTDRGWYCDNAGSVSFFPQAETCKVQSNRVFCDTMNSLTLPPEVNLCNVDIFNPKYDCKIMTSKTDVSSSVITSLGAIVSCYGKTKCTASNKNRGIIKTFSNGCDYVSNKGVDTVSVGNTLYYVNKQEGKSLYVKGEPIINFYDPLVFPSDEFDASISQVNEKINQSLAFIRKSDELL

SEQ ID NO: 94 - protein, 449 aa, synthetic construct
QNITEEFYQSTCSAVSKGYLSALRTGWYTSVITIELSNIKEPKCNGTDAKVKLIKQELDKYKNAVTELQLLMQSTPATGSGSAIASGVAVSKVLHLPGEVNKIKSALLSTNKAVVSLSNGVSVLTSKVLDLKNYIDKQLLPIVNKQSCSISNIETVIEFQQKNNRLLEITREFSVNAGVTTPVSTYMLTNSELLSLINDMPITNDQKKLMSNNVPIVRQQSYSIMSIIKEEVLAYVVQLPLYGVIDTPCWKLHTSPLCTTNTKEGSNICLTRTDRGWYCDNAGSVSFFPQAETCKVQSNRVFCDTMNSLTLPPEVNLCNVDIFNPKYDCKIMTSKTDVSSSVITSLGAIVSCYGKTKCTASNKNRGIIKTFSNGCDYVSNKGVDTVSVGNTLYYVNKQEGKSLYVKGEPIINFYDPLVFPSDEFDASISQVNEKINQSLAFIRKSDELL

SEQ ID NO: 95 - protein, 449 aa, synthetic construct
QNITEEFYQSTCSAVSKGYLSALRTGWYTSVITIELSNIKEPKCNGTDAKVKLIKQELDKYKNAVTELQLLMQSTPATGSGSAIASGVAVSKVLHLPGEVNKIKSALLSTNKAVVSLSNGVSVLTSKVLDLKNYIDKQLLPIVNKQSCSIPNIETVIEFQQKNNRLLEITREFSVNAGVTTPVSTYMLTNSELLSLINDMPITNDQKKLMSNNVPIVRQQSYSIMSIIKEEVLAYVVQLPLYGVIDTPCWKLHTSPLCTTNTKEGSNICLTRTDRGWYCDNAGSVSFFPQAETCKVQSNRVFCDTMNSLTLPPEVNLCNVDIFNPKYDCKIMTSKTDVSSSVITSLGAIVSCYGKTKCTASNKNRGIIKTFSNGCDYVSNKGVDTVSVGNTLYYVNKQEGKSLYVKGEPIINFYDPLVFPSDEFDASISQVNEKINQSLAFIRKSDELL

SEQ ID NO: 96 - protein, 466 aa, synthetic construct
QNITEEFYQSTCSAVSKGYLSALRTGWYTSVITIELSNIKEPKCNGTDAKVKLIKQELDKYKNAVTELQLLMQSTPATNNRARGSGSGRSLGFLLGVGSAIASGVAVSKVLHLPGEVNKIKSALLSTNKAVVSLSNGVSVLTSKVLDLKNYIDKQLLPIVNKQSCSISNIETVIEFQQKNNRLLEITREFSVNAGVTTPVSTYMLTNSELLSLINDMPITNDQKKLMSNNVPIVRQQSYSIMSIIKEEVLAYVVQLPLYGVIDTPCWKLHTSPLCTTNTKEGSNICLTRTDRGWYCDNAGSVSFFPQAETCKVQSNRVFCDTMNSLTLPPEVNLCNVDIFNPKYDCKIMTSKTDVSSSVITSLGAIVSCYGKTKCTASNKNRGIIKTFSNGCDYVSNKGVDTVSVGNTLYYVNKQEGKSLYVKGEPIINFYDPLVFPSDEFDASISQVNEKINQSLAFIRKSDELL

SEQ ID NO: 97 - protein, 466 aa, synthetic construct
QNITEEFYQSTCSAVSKGYLSALRTGWYTSVITIELSNIKEPKCNGTDAKVKLIKQELDKYKNAVTELQLLMQSTPATNNRARGSGSGRSLGFLLGVGSAIASGVAVSKVLHLPGEVNKIKSALLSTNKAVVSLSNGVSVLTSKVLDLKNYIDKQLLPIVNKQSCSIPNIETVIEFQQKNNRLLEITREFSVNAGVTTPVSTYMLTNSELLSLINDMPITNDQKKLMSNNVPIVRQQSYSIMSIIKEEVLAYVVQLPLYGVIDTPCWKLHTSPLCTTNTKEGSNICLTRTDRGWYCDNAGSVSFFPQAETCKVQSNRVFCDTMNSLTLPPEVNLCNVDIFNPKYDCKIMTSKTDVSSSVITSLGAIVSCYGKTKCTASNKNRGIIKTFSNGCDYVSNKGVDTVSVGNTLYYVNKQEGKSLYVKGEPIINFYDPLVFPSDEFDASISQVNEKINQSLAFIRKSDELL

SEQ ID NO: 98 - protein, 449 aa, synthetic construct
QNITEEFYQSTCSAVSKGYLSALRTGWYTSVITIELSNIKEPKCNGTDAKVKLIKQELDKYKNAVTELQLLMFLGFPLGVGSAIASGVAVSKVLHLEGEVNKIKSALLSTNKAVVSLSNGVSVLTSKVLDLKNYIDKQLLPIVNKQSCSISNIETVIEFQQKNNRLLEITREFSVNAGVTTPVSTYMLTNSELLSLINDMPITNDQKKLMSNNVPIVRQQSYSIMSIIKEEVLAYVVQLPLYGVIDTPCWKLHTSPLCTTNTKEGSNICLTRTDRGWYCDNAGSVSFFPQAETCKVQSNRVFCDTMNSLTLPPEVNLCNVDIFNPKYDCKIMTSKTDVSSSVITSLGAIVSCYGKTKCTASNKNRGIIKTFSNGCDYVSNKGVDTVSVGNTLYYVNKQEGKSLYVKGEPIINFYDPLVFPSDEFDASISQVNEKINQSLAFIRKSDELL

SEQ ID NO: 99 - protein, 449 aa, synthetic construct
QNITEEFYQSTCSAVSKGYLSALRTGWYTSVITIELSNIKEPKCNGTDAKVKLIKQELDKYKNAVTELQLLMFLGFPLGVGSAIASGVAVSKVLHLPGEVNKIKSALLSTNKAVVSLSNGVSVLTSKVLDLKNYIDKQLLPIVNKQSCSISNIETVIEFQQKNNRLLEITREFSVNAGVTTPVSTYMLTNSELLSLINDMPITNDQKKLMSNNVPIVRQQSYSIMSIIKEEVLAYVVQLPLYGVIDTPCWKLHTSPLCTTNTKEGSNICLTRTDRGWYCDNAGSVSFFPQAETCKVQSNRVFCDTMNSLTLPPEVNLCNVDIFNPKYDCKIMTSKTDVSSSVITSLGAIVSCYGKTKCTASNKNRGIIKTFSNGCDYVSNKGVDTVSVGNTLYYVNKQEGKSLYVKGEPIINFYDPLVFPSDEFDASISQVNEKINQSLAFIRKSDELL

SEQ ID NO: 100 - protein, 449 aa, synthetic construct
QNITEEFYQSTCSAVSKGYLSALRTGWYTSVITIELSNIKEPKCNGTDAKVKLIKQELDKYKNAVTELQLLMFLGFPLGVGSAIASGVAVSKVLHLPGEVNKIKSALLSTNKAVVSLSNGVSVLTSKVLDLKNYIDKQLLPIVNKQSCSIPNIETVIEFQQKNNRLLEITREFSVNAGVTTPVSTYMLTNSELLSLINDMPITNDQKKLMSNNVPIVRQQSYSIMSIIKEEVLAYVVQLPLYGVIDTPCWKLHTSPLCTTNTKEGSNICLTRTDRGWYCDNAGSVSFFPQAETCKVQSNRVFCDTMNSLTLPPEVNLCNVDIFNPKYDCKIMTSKTDVSSSVITSLGAIVSCYGKTKCTASNKNRGIIKTFSNGCDYVSNKGVDTVSVGNTLYYVNKQEGKSLYVKGEPIINFYDPLVFPSDEFDASISQVNEKINQSLAFIRKSDELL

SEQ ID NO: 101 - protein, 520 aa, synthetic construct
MKCLLYLAFLFIGVNCQNITEEFYQSTCSAVSKGYLSALRTGWYTSVITIELSNIKEPKCNGTDAKVKLIKQELDKYKNAVTELQLLMQSGGPGSGGGGSGGGGSRFPPFPLGVGSAIASGVAVSKVLHLPGEVNKIKSALLSTNKAVVSLSNGVSVLTSKVLDLKNYIDKQLLPIVNKQSCSISNIETVIEFQQKNNRLLEITREFSVNAGVTTPVSTYMLTNSELLSLINDMPITNDQKKLMSNNVPIVRQQSYSIMSIIKEEVLAYVVQLPLYGVIDTPCWKLHTSPLCTTNTKEGSNICLTRTDRGWYCDNAGSVSFFPQAETCKVQSNRVFCDTMNSLTLPPEVNLCNVDIFNPKYDCKIMTSKTDVSSSVITSLGAIVSCYGKTKCTASNKNRGIIKTFSNGCDYVSNKGVDTVSVGNTLYYVNKQEGKSLYVKGEPIINFYDPLVFPSDEFDASISQVNEKINQSLAFIRKSDELLGSGYIPEAPRDGQAYVRKDGEWVLLSTFLHHHHHHHH

SEQ ID NO: 102 - protein, 531 aa, synthetic construct
MELLILKANAITTILTAVTFCFASGQNITEEFYQSTCSAVSKGYLSALRTGWYTSVITIELSNIKEPKCNGTDAKVKLIKQELDKYKNAVTELQLLMQSGGPGSGGGGSGGGGSRFPPFPLGVGSAIASGVAVSKVLHLEPEVNKIKSALLSTNKAVVSLSNGVSVLTSKVLDLKNYIDKQLLPIVNKQSCSISNIETVIEFQQKNNRLLEITREFSVNAGVTTPVSTYMLTNSELLSLINDMPITNDQKKLMSNNVPIVRQQSYSIMSIIKEEVLAYVVQLPLYGVIDTPCWKLHTSPLCTTNTKEGSNICLTRTDRGWYCDNAGSVSFFPQAETCKVQSNRVFCDTMNSLTLPPEVNLCNVDIFNPKYDCKIMTSKTDVSSSVITSLGAIVSCYGKTKCTASNKNRGIIKTFSNGCDYVSNKGVDTVSVGNTLYYVNKQEGKSLYVKGEPIINFYDPLVFPSDEFDASISQVNEKINQSLAFIRKSDELLSAIGGYIPEAPRDGQAYVRKDGEWVLLSTFLHHHHHHHH

SEQ ID NO: 103 - protein, 537 aa, synthetic construct
MELLILKANAITTILTAVTFCFASGQNITEEFYQSTCSAVSKGYLSALRTGWYTSVITIELSNIKEPKCNGTDAKVKLIKQELDKYKNAVTELQLLMQSGGPGSGGGGSGGGGSRFPPFPLGVGSAIASGVAVSKVLHLEPEVNKIKSALLSTNKAVVSLSNGVSVLTSKVLDLKNYIDKQLLPIVNKQSCSISNIETVIEFQQKNNRLLEITREFSVNAGVTTPVSTYMLTNSELLSLINDMPITNDQKKLMSNNVPIVRQQSYSIMSIIKEEVLAYVVQLPLYGVIDTPCWKLHTSPLCTTNTKEGSNICLTRTDRGWYCDNAGSVSFFPQAETCKVQSNRVFCDTMNSLTLPPEVNLCNVDIFNPKYDCKIMTSKTDVSSSVITSLGAIVSCYGKTKCTASNKNRGIIKTFSNGCDYVSNKGVDTVSVGNTLYYVNKQEGKSLYVKGEPIINFYDPLVFPSDEFDASISQVNEKINQSLAFIRKSDELLSAIGRMKQIERKIEEILSKIYHIENEIARIKKLIGERHHHHHHHH

SEQ ID NO: 104 - protein, 535 aa, synthetic construct
MELLILKANAITTILTAVTFCFASGQNITEEFYQSTCSAVSKGYLSALRTGWYTSVITIELSNIKEPKCNGTDAKVKLIKQELDKYKNAVTELQLLMQSGGPGSGGGGSGGGGSRFPPFPLGVGSAIASGVAVSKVLHLEPEVNKIKSALLSTNKAVVSLSNGVSVLTSKVLDLKNYIDKQLLPIVNKQSCSISNIETVIEFQQKNNRLLEITREFSVNAGVTTPVSTYMLTNSELLSLINDMPITNDQKKLMSNNVPIVRQQSYSIMSIIKEEVLAYVVQLPLYGVIDTPCWKLHTSPLCTTNTKEGSNICLTRTDRGWYCDNAGSVSFFPQAETCKVQSNRVFCDTMNSLTLPPEVNLCNVDIFNPKYDCKIMTSKTDVSSSVITSLGAIVSCYGKTKCTASNKNRGIIKTFSNGCDYVSNKGVDTVSVGNTLYYVNKQEGKSLYVKGEPIINFYDPLVFPSDEFDASISQVNEKINQSLAFIRKSDELLGSRMKQIERKIEEILSKIYHIENEIARIKKLIGERHHHHHHHH

SEQ ID NO: 105 - DNA, 1401 bp, synthetic construct
  source 1..1401: mol_type = other DNA
caaaacatcacagaggaattttaccagtctacatgtagcgccgtgtccaaaggctacctgtctgccctgagaaccggctggtacaccagcgtcatcacaatcgagctgtctaacatcaaggaacctaagtgtaacggaacagatgctaaggtgaagctcatcaaacaggagctggacaagtacaagaatgccgtgactgagctgcagctgctgatgcagagcggcggacctggcagcggcggtggaggcagcggcggcggcggctctagattcctgggcttcctgctgggcgtcggctctgctatcgcctctggcgtggccgtgtctaaagtgctgcacctggaaggcgaagtgaacaagatcaagagcgccctgctttctaccaacaaggccgtggtttccctgagtaacggcgtgagcgtgctgacaagcaaggtgctggatctgaagaactacatcgataagcagctgctgccaatcgttaataagcagagctgcagcattagcaacattgaaaccgtgatcgagttccagcagaagaacaacagactgctggaaatcacccgcgagtttagcgtgaacgctggcgttacaacccctgtgagcacctacatgctgaccaacagcgaactgcttagcctgattaatgacatgcctatcaccaacgaccagaaaaagctgatgtctaacaacgtgcagatcgtgcggcagcaaagctacagcatcatgagcatcatcaaagaggaagtgctggcctacgtggtgcagctgcccctgtacggcgtcatcgacacaccttgctggaagctgcacaccagccctctgtgcaccacaaataccaaggaaggcagcaatatctgcctgaccagaaccgatagaggctggtattgcgacaacgccggcagcgtgtcattcttccctcaggccgagacctgcaaggtgcagtccaatcgggtgttctgcgataccatgaactctctgaccctgccctccgaggtgaacctgtgtaatgtagacatcttcaaccccaagtacgactgcaagatcatgaccagcaaaacagacgtgtctagcagcgtcatcaccagcctcggcgccatcgtgtcttgctacggcaagacaaagtgcaccgccagcaacaaaaaccggggcatcatcaagaccttcagcaatggatgtgactacgtgagcaacaagggcgtggacaccgtgagcgtgggcaacacactgtactacgtgaacaagcaagagggaaaatctctgtatgtgaagggcgagcctatcatcaacttctacgaccccctggtgtttccaagcgatgagttcgacgccagcatctcccaggtgaacgagaagatcaaccagtcgctggctttcatcagaaagagcgatgagctgctg

SEQ ID NO: 106 - DNA, 1401 bp, synthetic construct
  source 1..1401: mol_type = other DNA
caaaacataacagaggaattttaccagtccacctgtagcgctgtttctaaaggctacctgtcagctctgagaacaggctggtacaccagcgtgatcaccatcgaacttagcaacatcaaagaaaacaaatgcaacggtacagatgccaaggtgaaactgatcaagcaggagctggataagtacaagaatgccgtgaccgagctgcagctcctgatgcagtccggcggccctggcagcggcggaggaggcagcggcggcggcggcagcagattcctcggatttcctctgggcgttggaagcgccatcgcctctggagtcgccgtgtctaaggtgctgcacctggaaggcgaggtgaacaagatcaagagcgctctgctgagcaccaacaaggccgtggtgtctctgagcaacggcgtgtccgtgctgactagcaaagtgctggacctgaagaactacatcgataagcagctgctgccaatcgttaacaaacagagctgcagcatcagcaacatcgaaaccgtgatcgagtttcagcagaagaacaacagactgctggaaattacaagagagttcagtgtgaacgccggtgtcaccacccctgtgagcacctacatgctgaccaattctgagctgctgtctctgatcaatgatatgcctatcaccaacgaccagaaaaagctgatgagcaacaacgtgcagatcgtgcggcagcaaagctacagcatcatgagcatcatcaaagaggaagtgctcgcctacgtggtgcagctgcctctgtatggcgtgatcgacacaccttgttggaagctgcacacctctccactgtgcaccacaaacaccaaggaaggctccaatatctgcctgacaaggaccgatagaggctggtactgcgacaacgctggctcagtgagcttcttcccccaggccgagacatgcaaggtgcaatctaatcgggtgttctgcgacaccatgaacagcctgaccctgcctagcgaggtgaacctgtgtaatgtggacatcttcaaccccaagtacgactgcaagatcatgacaagcaagaccgacgtgagctccagcgtcattacaagcctgggcgccatcgtgtcttgctacggcaagaccaagtgtaccgccagcaacaagaaccggggcatcatcaagaccttcagcaatggctgcgactacgtgagcaacaagggagtggacaccgtgtcggtcggcaacacactgtactacgtgaacaagcaggagggcaagagcctgtatgtgaagggcgaacctatcatcaacttctacgaccccctggtgttccccagcgacgagttcgacgccagcatcagccaggtgaacgagaagatcaaccagagcctggccttcatcagaaagtctgatgagctgctg

SEQ ID NO: 107 - DNA, 1401 bp, synthetic construct
  source 1..1401: mol_type = other DNA
caaaacatcaccgaggaattttaccagagcacctgttccgctgtgagcaaaggatatctgagcgccctgagaaccggctggtacaccagcgtgatcacaatcgagcttagcaatatcaaggaaaacaagtgcaacggtacagacgccaaggtgaaactgatcaagcaagagctggataagtacaagaacgccgtgaccgagctgcagctgctgatgcagagcggcggccccggctccggcggcggaggctctggcggaggaggctctagattcctgggcttcctgcttggagtcggctctgccatcgccagcggcgtcgccgtgtcaaaggtcctgcacctggaaggcgaagtgaacaaaatcaagagcgccctgctgagcaccaacaaggccgttgtcagcctgagcaacggcgtgagcgtgctgaccagcaaggtgctggacctgaagaattacatcgacaagcagctgctgcctatcgtgaacaagcagtcttgcagcattagcaacatcgagacagtgatcgagttccagcaaaagaacaacagactgctggaaatcacacgggaatttagcgtcaatgccggcgttacaacccctgtgagcacctacatgctgacaaattctgagctgctgagcctgatcaacgacatgcctatcaccaatgaccagaaaaagctgatgtctaacaacgtgcctatcgtgcggcagcagtcttacagcatcatgtccatcatcaaagaggaagtgctggcttacgtggtgcagctgcctctgtacggagtgatcgataccccttgctggaagctgcacaccagccccctgtgtaccaccaacaccaaggagggctctaacatctgcctgactcggaccgatagaggctggtactgcgacaacgctggctctgtgtccttcttcccccaggccgagacatgcaaggtgcagtccaatagagtgttctgcgacaccatgaactccctgacactgccaagcgaggtgaatctgtgtaacgtggacatcttcaaccctaagtacgactgcaagatcatgaccagcaaaaccgacgtgagcagcagcgtgatcaccagcctgggcgccatcgtgagctgctacggaaagacaaagtgcaccgccagcaacaaaaataggggcatcattaaaaccttcagcaacggctgtgattacgtgagcaacaaaggcgtggacactgtgtctgtgggcaacacactgtactacgtgaacaagcaggagggcaagtccctctatgtgaagggcgagcccattatcaacttctacgatcctctggtgtttccatctgatgagttcgacgccagcatcagccaggtgaacgagaagatcaaccagagcctggctttcatcagaaagagcgacgagctgctg

SEQ ID NO: 108 - DNA, 1401 bp, synthetic construct
  source 1..1401: mol_type = other DNA
cagaacatcacagaggaattttaccagtccacctgtagcgctgtgtctaagggctacctgagcgccctgagaacaggctggtacaccagcgtgatcacaatcgagctgtctaatatcaaggaaaacaagtgtaacggcaccgatgccaaggtgaagctgatcaaacaggagctggataagtacaagaatgccgtcaccgaactgcagctgctgatgcagtctggcggacctggaagcggcggcggcggcagcggcggaggtggcagcagattcctgggcttcctgctgggcgtcggctctgctatcgcctccggcgtggccgtgagcaaggttctgcacctggaaggcgaggtgaataagatcaagtccgccctgctgagcaccaacaaggccgttgtgtccctgtctaatggagtttccgtcctcacctctaaggtgctggacctgaagaactacattgacaagcaactgctgcctatcgtgaacaagcaatcttgcagcatcagcaacatcgagacagtgatcgagttccagcagaagaacaacagactgctggaaatcacacgggagttcagcgtgaatgccggcgtgaccacccctgtgtctacctacatgctgaccaacagcgagctgctctccctcatcaacgacatgcctatcaccaacgaccagaaaaagctgatgagcaacaacgtgcagatcgtgcggcagcaaagctacagcatcatgagcattatcaaggaagaggtgctggcctacgtggtgcagctgcccctgtatggcgtgatcgataccccttgctggaagctgcacaccagtcctctgtgcaccacaaataccaaggagggctccaacatctgcctgaccaggacagacagaggctggtattgtgacaacgccggcagcgtgtcattcttcccacaggccgagacatgtaaagtgcagagcaatagagtgttctgcgataccatgaacagcctgacactgcctcctgaggtgaacctgtgcaacgtggacatcttcaaccccaagtacgactgcaagatcatgaccagcaagacagatgtgagcagcagcgtgatcaccagcctgggggccatcgtgtcctgctacggcaagaccaagtgcacagctagcaacaaaaaccggggcatcatcaagaccttttctaatggctgcgactacgtgtctaacaagggcgtcgacacggtgagcgtgggaaacaccctgtactacgtgaacaaacaggagggcaaaagcctgtacgtgaagggagaaccaatcattaacttctacgaccccctggtgttccccagcgacgagttcgacgccagcatcagccaggtgaacgagaaaatcaaccagagtcttgcttttatcagaaagtctgatgaactgctg

SEQ ID NO: 109 - DNA, 1401 bp, synthetic construct
  source 1..1401: mol_type = other DNA
cagaacatcaccgaagagttctaccagtctacgtgtagcgccgtgtccaaaggctacctgagcgctctgagaaccggctggtacacctccgtgatcacaattgagctgtccaacatcaaggagcctaagtgcaacggcaccgacgccaaggtgaaactgatcaagcaggagctggacaagtacaagaacgccgttacagagctgcagctgctgatgcagagcggcggacctggcagcggcggaggaggcagcggcggcggaggcagcagattcctgggcttcccactgggcgtcggatctgccatcgcctctggtgtggccgtaagcaaagtgctgcacctggaaggcgaggtgaacaagatcaaaagcgccctgctgagcacaaacaaggccgtcgtgtctctgagcaatggcgtgagcgtgctgacctccaaggtgctggacctgaagaactacatcgacaagcagctcctgccaatcgtgaacaagcaaagctgcagcatcagcaatattgagacagtgattgagtttcagcaaaagaacaacaggctgctggaaatcacccgggaatttagcgtcaacgccggcgtgacaacccctgtgagcacctacatgctgacaaacagcgagctgctgagcctcatcaacgacatgcctatcaccaacgaccagaagaagctgatgtccaataacgtgcagatcgtgcggcagcagagctacagcatcatgagcattatcaaggaagaggtgctggcctacgtggtgcaactgcctctgtacggcgtgatcgacaccccctgctggaagctgcacacatcccccctgtgcaccaccaataccaaggaaggctctaatatctgcctgaccagaacagatagaggctggtattgtgacaacgcaggctctgtttcattcttcccccaggccgagacctgcaaggtgcagagcaacagagtgttctgcgacaccatgaacagcctcaccctgcctagcgaggtgaatctgtgtaatgtggacatcttcaaccccaagtacgactgcaagatcatgacatctaagaccgacgtgtctagcagcgtgatcacctctctgggtgctatcgtgtcttgctacggcaaaaccaaatgcaccgccagcaataaaaaccggggcatcatcaagacattcagcaacggatgtgattacgtttctaacaaaggcgttgatacagtgtccgtgggcaacaccctgtactacgtgaataagcaggagggcaagagcctgtatgtgaagggcgaacctatcatcaacttctacgatcctctggtgtttccttctgatgagttcgacgccagcatcagccaggtgaacgagaagatcaaccagagcttggctttcatcagaaagtccgatgaactgctg

SEQ ID NO: 110 - DNA, 1401 bp, synthetic construct
  source 1..1401: mol_type = other DNA
caaaacatcacagaggagttctaccagagcacctgtagcgctgtgagcaagggctacctgagcgccctgagaaccggctggtacaccagcgtgatcaccatcgaactgtctaatatcaaggaacctaagtgtaatggcaccgatgccaaggtgaagctgatcaaacaggagctggataagtacaagaacgctgtgaccgagctgcagctgctgatgcagagcggcggacctggaagcggaggcggaggcagcggcggcggaggatctagattcctgggatttctgctgggcgtgggctctgctatcgcctctggcgtggccgtgagcaaggtgctgcacctggaaggcgaagtcaacaagatcaagtccgctctgctctctacaaacaaggccgtggtctccctgtccaacggcgtgtccgtgctgacaagcaaagtgctggacctgaaaaattacatcgacaaacagctgctgcctattgtgaacaagcaatcatgcagcatcagcaacatcgagacagtgatcgagtttcagcagaaaaacaacagactgctggaaatcactcgggaatttagcgtgaacgccggcgtgaccacccctgtgtccacctacatgctgaccaactctgagctgctgagcctgatcaacgacatgcccattaccaatgatcagaaaaagctgatgagcaacaatgtgcctatcgtcaggcagcagagctacagcatcatgagcatcattaaagaagaggtgctcgcctacgtggtgcaactgcctctgtacggcgttatcgatacaccttgctggaagctgcacacatctccactgtgtaccacaaataccaaggaaggcagcaacatctgcctgacaagaacagatagaggctggtattgcgacaacgccggatctgttagcttcttccctcaggccgagacatgcaaggtgcagtctaaccgggtgttctgcgacaccatgaacagcctgaccctgccaagcgaggtgaatctgtgcaacgtcgacatcttcaaccccaagtacgactgcaagatcatgaccagcaaaaccgacgtgtccagcagcgtgatcaccagcctgggcgccatcgtgagctgctacggcaagactaagtgcacagcctccaacaagaaccggggcatcatcaagaccttcagcaacggttgtgactacgtgtctaacaagggcgtggacaccgtgagcgttggcaacaccctgtactacgtcaacaagcaggagggcaaaagtctgtacgtgaagggcgagcctatcatcaacttctatgaccccctggtgttccccagcgacgagttcgacgccagcatctctcaggtgaacgagaagatcaaccagagcctcgccttcatcagaaagagcgatgagttgctg

SEQ ID NO: 111 - DNA, 1401 bp, synthetic construct
  source 1..1401: mol_type = other DNA
cagaacatcactgaggaattttaccagagcacctgtagcgccgtttctaaaggctacctgagcgccctgagaaccggatggtatacaagcgtcatcaccatcgaactgagtaatattaaggaacctaagtgtaatggcaccgacgccaaggtgaagctgatcaagcaggagctggacaagtacaagaacgccgtgaccgagttgcagctgctgatgcagtctggcggacctggcagcggaggaggcggcagcggcggaggaggctctagattcctgggcttcctgctgggagttggctcggctatcgccagcggcgtggccgtgagcaaagtgctgcacctggaaggcgaggtgaacaagatcaagtcagctctgctgagcacaaacaaggccgtggtgagcctgtccaacggcgtaagcgtgctgaccagcaaggtgctggatctgaagaactacatcgataaacaactgctgcctatcgtgaacaagcaaagctgcagcatcagcaacatcgagacagtgatcgagtttcagcaaaagaacaaccggctgctggagatcaccagggaattttctgtcaatgctggcgtcaccactcctgtgtctacatacatgctgacaaacagcgagctgctgagcctgatcaatgatatgcctatcacaaatgaccagaaaaagctgatgagcaacaacgtgcagatcgtgcggcagcagagctacagcatcatgagcatcatcaaggaagaagtgctggcctacgtcgtgcagctgcctctgtatggcgtgatcgacaccccttgctggaagctgcacaccagcccactgtgtacaaccaacacaaaggaaggctctaacatctgcctgacaagaacagatagaggctggtactgcgacaacgccggcagcgtgtccttcttccctcaggccgagacctgcaaggtgcagagcaacagagtgttctgcgacaccatgaacagcctgaccctgccacctgaggtgaatctgtgcaacgtggacatcttcaaccccaagtacgactgcaagatcatgaccagcaaaaccgatgtgtcctccagcgtgattacatctctgggcgccatcgtgtcctgctacggcaagaccaagtgcaccgctagcaataaaaatcggggcatcatcaaaaccttcagcaacggttgtgactacgtgtccaacaaaggcgtggacaccgtgtccgtgggcaacaccctgtactacgtgaacaagcaggagggtaagtctctgtacgtgaagggcgaacccatcatcaacttctacgaccccctggtgttccccagcgacgagttcgacgcctctatcagccaggtgaacgagaagattaaccagagcctcgccttcatcagaaagtccgatgagctgctg

SEQ ID NO: 112 - DNA, 1401 bp, synthetic construct
  source 1..1401: mol_type = other DNA
caaaacatcaccgaggagttctaccagtctacatgcagcgccgtgagcaagggctacctgagcgccctgagaacaggctggtatacaagcgtgatcaccatcgagctgtccaacatcaaggaaaacaagtgcaacggcaccgacgcaaaggtcaagctgatcaagcaggagctggacaagtataagaacgctgtgaccgagctgcagctcctgatgcagagcggcggacctggaagcggcggcggcggcagtggcggaggcggctcaagattcctgggatttccactgggcgtgggcagcgccatcgcctctggcgtggccgtgtctaaagtgctgcacctggaaggcgaggtgaacaaaatcaagagcgctctgctgagcacaaataaggccgtggtcagcctgtctaacggcgtgtccgtgctgacaagcaaagtgctggacctgaagaactacatcgataagcagctgctccctatcgtgaacaagcaaagctgcagcatctccaatatcgagacagtgatcgaatttcagcaaaagaacaaccggctgctggaaatcaccagagagttcagcgtgaacgccggtgtgacaacccctgtgtctacatacatgctgaccaactccgagctgctgagcctgattaatgatatgcctatcaccaacgaccagaagaagctgatgagcaacaacgtgcccatcgtgcggcagcagagctacagcatcatgagtatcatcaaggaagaagtgctcgcttacgtggtgcagctgccactgtacggcgttatcgacaccccttgttggaagctgcacaccagccctctgtgcaccaccaacacaaaggaaggcagcaatatctgcctgacccgcacagacagaggctggtactgcgacaacgccggctctgtgagcttcttcccccaggccgaaacctgtaaagttcagagcaacagagtgttctgcgatacaatgaacagcctcaccctgcccagcgaggtgaacctgtgtaacgtggacatcttcaaccccaagtacgactgcaagatcatgacctccaagaccgatgtgtctagctctgtcatcacttctctgggcgccatcgtgtcctgctacggcaagaccaaatgtaccgcctcgaacaaaaatcggggcatcatcaagacctttagcaatggctgcgactacgtaagcaacaagggcgtggacaccgtgagcgtcggaaacaccctgtactacgtgaataagcaggagggcaaaagcctgtacgtgaaaggagagcctatcattaacttctacgatcctctggtgttcccttctgatgagttcgacgccagcatcagccaggtgaacgagaagattaaccagagcctggccttcatcagaaagagcgacgagctgctg

SEQ ID NO: 113 - DNA, 1401 bp, synthetic construct
  source 1..1401: mol_type = other DNA
cagaacatcaccgaggaattttaccagagcacttgttctgccgtgtccaagggttatctgagcgccctgagaaccggctggtatacaagcgtgatcaccatcgagctgagcaacatcaaggaaaacaaatgcaacggaacagatgccaaagtgaagctcatcaagcaggagctggataagtacaagaacgctgttacagagctgcagctgctgatgcagtctggcggccctggctccggcggcggaggcagcggaggcggcggctcaagattcctgggcttccccctgggcgtgggatctgctatcgccagcggcgtggccgtgagcaaggtgctgcacctggaaggcgaggtgaacaagatcaaaagcgctctgctgtctaccaacaaggccgtggtgtctctgagcaacggcgtgagcgtgctgaccagcaaggtgctggacctgaagaactacatcgacaagcaactgctgcctattgtgaataaacagtcctgcagcatctctaatattgagacagttatcgagtttcagcaaaagaacaaccggctgctggaaatcaccagagagtttagcgtgaacgctggcgtgaccacccctgtgagcacctacatgctgaccaacagtgaactgctgagtttgatcaatgacatgccaatcacaaatgaccagaaaaagctgatgagcaataatgtccagatcgtgcggcagcagagctacagcatcatgtccatcatcaaggaagaggtgctggcctacgtggtgcaactgcccctgtacggcgttattgacaccccttgctggaagctgcacaccagccccctgtgcacaaccaacaccaaagagggcagcaacatatgcctgacccgcacagatagaggctggtactgcgacaacgccggcagcgtctccttcttcccccaggccgagacatgtaaagtgcagagcaatcgggtgttctgcgataccatgaacagcctgacactgccacctgaagtgaacctgtgtaacgtggacatcttcaaccctaagtacgactgcaagatcatgacctccaagacggacgtgtctagcagcgtgatcacaagcctcggagccatcgtgtcttgttacggcaagaccaagtgcaccgcctctaacaagaatagaggcatcatcaagacattcagcaacggctgcgattacgtgagcaacaagggcgtggacaccgtgtccgtgggcaacaccctgtactacgtgaacaaacaggagggaaagtccctgtacgtcaagggagaacctatcatcaacttctacgaccctctggtgttcccttccgacgagttcgacgccagcatcagccaggtgaacgagaagatcaaccagagcctggccttcatcagaaagtctgatgaactcctg

SEQ ID NO: 114 - DNA, 1401 bp, synthetic construct
  source 1..1401: mol_type = other DNA
caaaacattacagaagagttctaccagagtacatgcagcgccgtgtccaagggctacctgagcgccctgagaaccggctggtacaccagcgtgatcaccatcgagctgagcaacatcaaggaaaacaagtgcaatgggaccgacgccaaggtgaagctgatcaagcaggagcttgataagtataagaatgctgtgaccgagctgcagctgctgatgcagagcggcggccctggcagcggcggcggcggctccggaggcggaggatctagattcctgggcttcctgctgggagtgggatctgccatcgcctccggcgtggccgtgtctaaggttctgcacctggaaggcgaagtgaacaagatcaagagcgccctgctgagcaccaacaaggctgttgtgagcctgtctaacggcgtgtccgtgctgaccagcaaagtgctggacctgaagaactacatcgacaagcaactgctccctatcgttaacaagcagagctgtagcattagcaacattgagacagtgatcgagtttcagcagaagaacaacagactgctggaaatcacccgggaattttctgtgaacgccggcgtcaccacccctgtgtctacatacatgctgaccaatagcgagctgctgtccctgatcaacgacatgcctatcacaaatgaccagaaaaagctgatgagcaacaacgtgccaatcgtgcggcagcagagctacagcatcatgtctatcatcaaagaggaagtcctggcctacgtggtgcaactgcctctgtacggcgtgatcgacactccgtgctggaagctccacaccagccctctgtgtacaaccaacacaaaggaaggcagcaatatctgcctgacccgcaccgacagaggctggtattgcgataacgctggctctgtgtccttcttcccccaggccgagacatgtaaagtgcagagcaatagagtgttctgcgacaccatgaacagcctgacactgccccccgaggtgaatctgtgcaacgtggacatcttcaaccccaagtacgactgcaagatcatgaccagcaaaaccgatgtgtctagcagcgtaatcacaagcctgggcgctatcgtgtcttgctacggcaagaccaagtgcaccgccagcaacaaaaaccggggaatcatcaagacattcagcaacggttgtgactacgtgagcaataaaggcgtggatacagtgtccgtgggcaacaccctgtactacgtgaacaagcaggagggcaaaagcctgtacgtcaagggcgagcctatcataaacttctacgatcctctggtgttccctagcgatgagttcgacgccagcatcagccaggtgaacgagaagatcaaccagtccctggcctttatcagaaagtccgacgagctgctg

SEQ ID NO: 115 - DNA, 1401 bp, synthetic construct
  source 1..1401: mol_type = other DNA
cagaacatcaccgaggagttctaccagagcacctgtagcgccgtgtctaagggctacctgagcgccctgagaaccgggtggtacaccagcgtgatcacaatcgagctgtctaatatcaaggaacctaagtgcaacggcaccgacgcaaaggtcaagctgatcaagcaggagctggataagtacaagaacgccgtcaccgaactgcagctgctgatgcagagcggcggtcctggcagcggaggcggcggctctggaggcggaggctcaagattcctgggcttcccactcggcgtcggctcagctatcgccagcggggtcgccgtgtctaaagtgctgcacctggaaggcgaggtgaacaagatcaagtctgctctgctgtctacaaacaaggccgtggtgagcctgagcaacggcgtttccgtgctgacatctaaggtgctggacctgaagaactacatcgataagcaactgcttccaatcgtgaataaacaaagctgcagcatctccaatatcgagacagtgatcgagtttcagcaaaagaacaaccggctcctggaaatcactcgggaatttagcgtgaacgccggcgtgaccacccctgtgtccacctacatgctgaccaatagcgagctgctgagcctgatcaacgacatgcctattacaaatgaccagaaaaagctgatgagcaacaacgtgcccatagtgcggcagcagagctacagcatcatgagcatcatcaaagaggaagtgctggcctacgtggtgcagctgcccctgtatggcgtgatcgacacaccttgctggaagctgcacacaagccctctgtgcaccacaaacaccaaggaaggcagcaatatctgcctgaccagaacagatagaggatggtattgcgataacgctggctctgtgagctttttccctcaggccgaaacctgcaaggtgcagagcaacagagtgttctgcgacaccatgaacagcctgacactgccttctgaggttaacctgtgtaatgtggacatcttcaaccccaagtacgactgcaagatcatgaccagcaagacagacgtgtccagcagcgttatcaccagcctgggcgccatcgtgagttgctacggcaagaccaagtgtaccgcctctaacaaaaaccgcggcattattaagaccttcagcaatggatgtgactacgtgtccaacaagggcgtggataccgtgtccgtgggcaacaccctgtactacgtgaacaaacaggagggaaaaagcctgtacgtgaaaggcgagcctatcatcaacttctacgaccccctggtgttccccagcgacgagttcgacgccagcatcagccaggtgaatgagaagatcaaccagtctctcgccttcatcagaaagtctgatgagctgctg

SEQ ID NO: 116 - DNA, 1401 bp, synthetic construct
  source 1..1401: mol_type = other DNA
cagaacattacagaggaattttaccagagcacatgtagcgctgtgtccaagggctacctgagcgccctgagaaccggctggtatacatctgtgatcaccatcgagctttccaatatcaaggaacccaagtgcaacggcaccgacgccaaggtcaagctgatcaagcaggagctggataagtacaagaacgccgtcaccgagctgcagctgctgatgcagtctggcggacctggctctggcggaggcggaagcggcggcggtggcagcagattcctgggcttcccactgggcgtgggcagcgctatcgccagcggcgtggccgtgtctaaggtgctgcacctggaaggcgaggtgaacaagatcaagagcgccctgctgagcaccaacaaagccgtggtgtccctgagcaatggagtgtccgtgctgaccagcaaagttctggacctgaagaactacatcgacaagcagctgctgcccatcgtgaacaagcagagctgcagcatcagcaacatcgagaccgtgattgagtttcagcaaaagaacaatcggctgctggaaatcactcgggagttcagcgttaatgccggcgtgaccacccctgtgtctacctacatgctgaccaatagcgagctgctgtctctgatcaatgatatgcctatcaccaacgaccagaaaaagctgatgagcaacaacgtgcagatcgtgcggcagcagtcatatagcatcatgagcatcatcaaagaagaggtgctggcctacgtggtccaactgcctctgtacggcgtgatcgacaccccgtgctggaagctgcacaccagccctctgtgcaccacaaacaccaaggaaggctccaacatctgcctgaccagaacagatagaggctggtactgcgacaacgctggaagcgtgagcttcttccctcaggccgaaacctgcaaggtgcagagcaatagagtgttctgcgacacaatgaacagcctcaccttgccacctgaggtgaacctgtgtaatgtggacatcttcaaccccaagtacgactgcaagatcatgacctctaaaaccgacgtgtccagcagcgtgattacaagcctgggagccatcgtgtcttgctacggcaagacaaagtgtacagccagcaacaaaaaccgcggcatcatcaagaccttcagcaacggctgtgattacgtgagcaacaagggcgtcgacacagtgtccgtcggcaacacactgtactacgtgaacaagcaagagggaaaatctctgtacgtgaagggagaacctatcatcaacttctacgatcctctggtgttccccagcgacgagttcgacgcctctatcagccaggtgaacgagaagatcaaccagagcctggcttttatcagaaagtctgatgagctgctt

SEQ ID NO: 117 - DNA, 1401 bp, synthetic construct
  source 1..1401: mol_type = other DNA
caaaatatcaccgaggagttctaccagtctacatgcagcgctgtgtccaagggctacctgagcgccctgagaacaggctggtacaccagcgtgatcacaatcgagctgagcaacatcaaggaacctaagtgcaacggcaccgatgccaaggtgaagctgatcaagcaggagctggacaagtacaagaatgccgtgaccgagctgcagctgctgatgcagtccggcggtcctggcagcggcggaggcggaagcggaggcggcggatcaagattcctgggcttcctgctgggcgtgggcagcgctatcgcctctggcgtcgccgtgtctaaggtgctgcacctggaaggcgaagtgaataaaatcaaaagcgccctgctgtctaccaacaaggccgtggtgtctctgagcaatggcgtgagcgtgctgacctccaaagtgctggatctgaagaactacatcgataagcaactgctgcctatcgtgaacaagcagtcctgttctatcagcaacatcgaaacagtgatcgagtttcagcagaaaaacaaccggctgctggaaatcactagagagtttagcgtgaacgctggcgtgaccacccctgtgtccacctacatgctgaccaatagcgagctgctcagtctgatcaatgacatgcctatcacaaatgaccagaagaagctgatgagcaacaacgttcctattgtgcggcagcagagctacagcatcatgagcatcatcaaggaagaagtgctcgcctacgtggtccagctgcccctgtacggagtgatcgacacgccctgctggaagctgcacaccagccctctttgtaccacaaacacaaaggagggaagcaacatctgcctgacacggacagacagaggctggtattgcgacaacgccggcagcgtcagcttcttcccacaggccgagacctgcaaggtgcaaagcaacagggtgttctgcgacaccatgaacagcctgaccctgccacctgaggtgaacctgtgtaatgtggacatctttaaccccaagtacgactgcaagatcatgacaagcaagacagatgtgtctagctccgtgatcaccagcctgggagccatcgtgtcctgctacggcaaaaccaagtgcaccgccagcaacaagaacagaggcatcatcaagaccttcagcaacggctgtgactacgtgagcaacaaaggcgtcgacaccgtgagtgttggaaataccctgtactacgtgaacaaacaggagggcaagtccctgtatgtgaagggcgagcccatcatcaacttctacgatcctctggtattccccagcgacgagttcgacgccagcattagccaggtgaacgagaagattaaccagagcctggctttcatcagaaagtctgatgagctcctg

SEQ ID NO: 118 - DNA, 1401 bp, synthetic construct
  source 1..1401: mol_type = other DNA
cagaacatcacagaggaattttaccagagcacatgcagcgctgtgtctaaaggttatctgtctgctctgagaaccggctggtacacctctgtgatcaccatcgagctgagcaacatcaaggagaacaagtgtaatggcaccgacgccaaggtgaagctgatcaagcaggagctggacaagtacaagaatgccgtgaccgagctgcagctgctgatgcagagcggcggccctggcagcggcggaggagggtctggcggcggcggcagtagattcctgggcttccctctgggcgtgggcagtgctatcgccagcggcgtggccgtgagcaaggtgctgcacctggaaggcgaggtgaacaagatcaagtccgccctgctgtctactaacaaagccgtggtctccctaagcaacggcgtgtctgtgctgaccagcaaggtgctggatctgaagaactacatcgacaaacaactgctgcccattgtgaacaagcagagctgctccatcagcaacatcgaaaccgtgatcgagtttcagcaaaaaaacaaccggctgctggaaatcaccagagagttcagcgtgaacgccggcgttacaacccctgtgtctacatacatgctgacaaatagcgagctgctgtccctgatcaacgacatgcctatcaccaatgaccagaagaagctgatgagcaacaacgtgcccatcgtcagacagcagagctacagcatcatgagcattatcaaagaggaagtgctggcctacgtggtgcagctgcctctgtatggcgtgatcgacaccccttgctggaagctgcacaccagccctctgtgtaccaccaacacaaaggaaggcagcaatatctgcctgacacggaccgatagaggctggtactgcgacaacgctggaagcgtctccttcttcccacaggccgagacctgcaaggttcaatccaatagagtgttctgcgataccatgaacagcctgacactgcctccagaagtgaacctgtgcaacgtggatatcttcaaccccaagtacgactgcaaaatcatgaccagcaaaacagatgtgtccagcagcgtgatcaccagcctgggagccatcgtgtcttgttacggcaagaccaagtgcaccgccagcaacaagaacaggggaatcatcaagacatttagcaacggctgtgactacgtgtctaataaaggcgtggacacagtgtccgtcggcaacaccctgtactacgtgaacaagcaggagggaaagagcctgtacgttaagggagagcctatcatcaacttctacgaccccctggtgttccccagcgacgagttcgacgccagcatcagccaggtgaatgaaaagatcaaccagagcctcgccttcatccggaagtctgatgaactcctc

SEQ ID NO: 119 - DNA, 1401 bp, synthetic construct
  source 1..1401: mol_type = other DNA
cagaacatcaccgaggagttctaccagtctacatgtagcgctgtatccaaaggctacctgtctgctctgagaaccggctggtacaccagcgtgattaccatcgagctgagcaacatcaaggagcctaagtgcaacggtacagatgccaaggtgaagctgatcaagcaagagctggataagtacaagaacgccgtcaccgagctgcagctgctgatgcagagcggcggacctggctccggcggcggcggaagcggcggcggcggaagtagattcccacctttcctgctgggagtgggcagcgccatcgcctccggcgtggccgtgagcaaagtgctgcacctggaaggagaagtgaacaagatcaagagcgccctgctcagcaccaacaaagccgtggtgtccctgagcaatggcgtgtctgtcctgaccagcaaggtgctggacctgaagaactacatcgacaagcagctgctgcctattgttaacaagcagtcttgttctatcagcaacatcgagacagtgattgagtttcagcaaaagaacaaccggctgctggaaatcaccagggagttcagcgtgaacgccggcgtgaccacacctgtgtccacctacatgctgacaaatagcgaactgctgagcctgatcaatgatatgcccatcacaaacgaccagaaaaagctgatgagcaacaacgtgcaaatcgtgcggcagcagagctacagcatcatgagcatcatcaaagaggaagtgctggcctacgtggtgcagctccctctgtacggcgttatcgacaccccctgctggaagctgcacacctctccactgtgcacgacaaataccaaggaaggatctaacatctgcctgacaagaaccgacagaggctggtattgtgacaacgctggcagtgtcagcttcttcccccaggccgaaacctgcaaggtgcagagcaatcgggtgttctgcgacacaatgaacagcctgaccctgcctagcgaggtgaatctgtgtaatgtggatatcttcaaccccaaatacgactgcaagatcatgacaagcaaaaccgatgtgagttctagcgtgatcaccagcctgggcgccatcgtgtcttgctacggcaagacaaagtgcaccgccagcaacaagaacagaggcatcatcaagacttttagcaacggctgcgactacgtgtccaataagggcgtggacaccgtgagcgtcggcaacaccctgtactacgtgaacaagcaggaaggcaaatccctgtatgtgaagggcgagcctatcatcaacttctacgaccccctggtgtttccttctgatgagttcgacgccagcatcagccaggtgaacgagaagatcaaccagagcctggctttcatcagaaagtccgacgagctgctg

SEQ ID NO: 120 - DNA, 1401 bp, synthetic construct
  source 1..1401: mol_type = other DNA
cagaacatcaccgaggagttctaccagtctacttgtagcgctgtgtccaagggatatctgagcgccctgagaaccggctggtacaccagcgtcatcacaatcgagctgtcgaacatcaaagaaaacaaatgcaacggtacagatgccaaggtgaaactgatcaaacaggagctggacaagtacaagaatgctgttacagagctgcagctgctgatgcagagcggaggacctggctccggcggaggcggaagcggcggcggcggctcaagattcccccccttcctgctgggcgttggcagcgctatcgcctctggcgtggccgtgtccaaggtgctgcacctggaaggcgaagtgaacaaaatcaagagcgccctactgtccaccaacaaggccgtggtgtctctgagcaacggcgtgagcgtgctgacatctaaggtgctggatctgaagaactacatcgataagcaactgcttccaatcgtcaacaagcaatcttgcagcattagcaatatcgagacagtgatcgaatttcagcaaaaaaacaacagactgctggaaatcacaagagagtttagcgtgaacgccggcgtgaccacacctgtgtctacctacatgctgacaaatagcgagctgctgagcctgatcaacgacatgcctatcaccaacgaccagaaaaagctgatgagcaacaacgtgcctatcgtgcggcagcagtcatatagcatcatgagcatcatcaaggaagaggtgctggcctacgtcgtgcagctgcctttgtacggcgtgatcgacaccccttgctggaagctgcacaccagtcctctgtgcaccaccaacaccaaggaaggctccaatatttgtctgaccagaacagacagaggctggtactgcgacaacgcaggctctgtctcttttttcccacaggccgagacctgcaaggtccagagcaaccgggtgttctgcgataccatgaacagcctgaccctgcctagcgaggtgaatctgtgtaatgtggacatcttcaaccccaagtacgactgcaagatcatgaccagcaaaaccgatgtgagttcttctgtgatcaccagcctgggcgccatcgtcagctgctacggcaagaccaagtgcacagccagcaacaagaaccgcggcatcatcaagaccttcagcaatggatgtgactacgtgagcaataagggcgtggatacagtgtccgtgggaaacaccctgtactacgtgaacaagcaggaaggcaaaagcctctacgtgaagggcgagcctatcatcaacttctacgaccccctggtgttccccagcgacgagttcgacgccagcatcagccaggtgaacgagaagattaaccagagcctggccttcatccggaagagcgacgagctgctg

SEQ ID NO: 121 - DNA, 1401 bp, synthetic construct
  source 1..1401: mol_type = other DNA
cagaacatcactgaagagttttaccagtctacatgcagcgccgtgtctaagggctacctgagcgccctgagaaccggctggtacaccagcgtgatcaccattgagctgtctaacatcaaggaaaacaaatgcaatggcaccgatgccaaggtcaaactgattaaacaggagctggataagtacaagaacgccgtcacagaactgcagctgctgatgcagagcggcggtcctggctctggaggcggaggaagcggcggcggcggcagcagattccctccattcctgcttggcgtcggcagcgctatcgccagcggcgtggccgtgtctaaggtgctgcacctggaaggagaggtgaacaagatcaagtctgctctgctgagcaccaacaaggccgtggtgtccctgagcaacggagtcagcgtgctgaccagcaaggtgctggacctgaagaactacatcgacaagcaactgctgcccatcgtgaataaacaatcttgtagcatcagcaacattgaaaccgtgatcgagtttcagcaaaagaacaacaggctgctggagatcacccgggagttcagcgtgaacgccggcgttacaacacctgtgtccacatacatgctgaccaatagcgaactgctgagcctgatcaatgatatgcccatcaccaacgaccagaaaaagctgatgagcaacaacgtgcagatcgtgcggcagcagagctacagcatcatgtctatcatcaaggaggaagtgctcgcttatgtggtgcagctgcctctgtacggagtgatcgacaccccttgttggaagctgcacacatctcctctgtgtaccaccaataccaaggagggcagcaatatctgcctgaccagaacagatagaggatggtattgcgacaacgctggcagcgtcagcttcttcccccaggccgagacatgcaaggtgcagagcaatagagtgttctgcgatacaatgaacagcctgacactgcctcctgaggtgaacctgtgcaacgtggacatcttcaaccccaagtacgactgcaagatcatgaccagcaagacagacgtgagctccagcgtgattacaagcctgggcgccatcgtgtcctgctacggcaaaaccaagtgcaccgcctctaataaaaaccggggcatcatcaagaccttcagcaacggctgtgactacgtgagcaacaaaggcgttgacaccgtatcggtgggcaacaccctgtactacgtgaacaagcaggaaggcaagagcctgtacgtgaagggcgagcctatcatcaacttctacgaccccctggtgtttccatctgacgagttcgacgccagcatctctcaggtgaacgagaagatcaaccagagcctcgccttcatcagaaagtccgatgagctgctg

SEQ ID NO: 122 - DNA, 1401 bp, synthetic construct
  source 1..1401: mol_type = other DNA
cagaacatcaccgaggaattttaccagagcacatgtagcgctgtttctaagggctacctgtctgctctgagaaccggctggtacacatctgtgatcaccatcgagctgagcaacatcaaagaacctaagtgcaacggcacagatgccaaggtgaagctgatcaagcaggagctggataagtacaagaacgccgtgaccgagctgcagctgctgatgcaaagcggaggtcctggcagcggcggcggcggaagcggaggaggcggatctagattcccacctttcctgctgggcgtgggcagcgccatcgccagcggggtggctgtgagcaaggtgctgcacctggaaggcgaggtcaacaagatcaagagcgccctgctgagcaccaacaaggccgtggtcagcctgtctaacggcgtgagcgtgctgaccagcaaggtgctggacctgaagaactacatcgacaagcagctgctgcctatcgtgaataagcaaagctgttctatcagcaacatcgagacagtgatcgagtttcagcagaaaaacaaccggctgctggaaatcacaagagagtttagcgttaatgctggcgtgacaacacctgtgtctacctacatgctgaccaatagcgagctgctttctctgatcaatgatatgcctattaccaacgaccagaaaaagctgatgtccaacaacgtgcccattgtgcggcagcaaagctacagcatcatgagtatcatcaaggaagaagtgctggcctacgtggtgcagctgcctctgtatggcgttatcgataccccttgttggaagctgcacacaagccctctgtgtaccaccaacacaaaggaaggcagcaatatctgcctgacccgcaccgatagaggctggtattgcgacaacgccggctccgtctccttcttcccccaggccgagacatgcaaggtgcagagcaacagagtgttctgcgacaccatgaacagcctgacactgcccagcgaggtgaacctgtgcaacgtggacatcttcaaccccaagtacgactgcaagatcatgacctctaaaacagacgtgtccagcagcgtgatcaccagcctgggcgccatcgtgtcctgctacggcaaaaccaagtgcaccgcctctaacaaaaatcggggcatcatcaagaccttcagcaatggctgcgactacgtgtccaacaagggcgtcgacaccgtgagcgtgggcaacaccctgtactacgtgaacaaacaggagggcaagagcctgtacgtgaaaggcgaaccaatcatcaacttctacgaccccctggtgttccctagcgacgagttcgacgccagcatttctcaggtgaacgagaagatcaaccagtccctcgccttcatcagaaagtctgatgagctgctc

SEQ ID NO: 123 - DNA, 1401 bp, synthetic construct
  source 1..1401: mol_type = other DNA
cagaacatcaccgaggaattttaccagagcacatgttctgcagttagcaagggctacctgtcagctctgagaaccggctggtacaccagcgtgatcaccatcgagctgtccaatatcaaggaacccaagtgcaacggcaccgatgccaaggtcaagctgatcaagcaggagctggacaagtacaagaacgccgtgacagaactgcagttgctgatgcagtccggcggacctggcagcggaggaggcggcagcggcggcggcggctctagattccctcctttcctgctgggcgtcggctccgctatcgccagtggcgtcgccgtgtccaaagtgctgcacctggaaggagaagtgaataagatcaagagcgccctgctgagcaccaacaaggccgtggtgagcctgtccaacggcgtgtctgtgctgacctctaaggtgctggatctgaagaactacatcgacaagcagctgctgcctatcgtgaacaaacaaagctgcagcattagcaacatcgagacagtgatcgagttccagcagaaaaacaaccggctgctggagatcacccgggagttcagcgtgaatgccggagttacaacccctgtgagcacctacatgctgaccaacagcgaactgctgagcctcatcaacgacatgcctattaccaacgaccagaagaagctgatgagcaacaacgtgcagatcgtgcggcagcaaagctacagcatcatgtctatcatcaaagaggaagtgctggcctacgtggtgcagctgcctctgtatggcgtgatcgacaccccttgctggaagctgcacaccagccctctgtgcaccacaaataccaaggaaggaagtaacatctgcctgacaagaacagatagaggctggtattgcgacaacgccggctctgtcagcttcttcccacaggccgagacatgcaaagtgcagagcaaccgcgtgttctgcgacaccatgaactctctcacactgccccccgaggtgaatctgtgtaacgtggacatcttcaacccaaagtacgattgcaaaattatgaccagcaagaccgacgtgtctagcagcgtgatcacatctctgggcgccatcgtctcctgctacggcaagaccaagtgtaccgccagcaacaagaacagaggaatcatcaagacttttagcaacggttgtgattacgttagcaataaaggcgtggacacagtgagcgtgggcaacaccctgtactacgtgaacaagcaagagggcaaaagcctgtacgtgaagggcgagcctatcatcaatttctacgaccccctggtgttccccagcgacgagttcgacgcctcaatcagccaggtgaatgagaagatcaaccagagcctggcttttatcagaaagtctgatgagctgctg

SEQ ID NO: 124 - DNA, 1401 bp, synthetic construct
  source 1..1401: mol_type = other DNA
caaaatatcaccgaggagttctaccagagcacctgcagcgccgtgtctaagggctacctgagcgccctgagaactggctggtacaccagcgtgatcaccatcgagctctccaacatcaaggaacctaaatgcaacggcaccgacgccaaggtgaaactgatcaagcaggagctcgacaaatacaagaatgctgtgaccgagctgcagctgctgatgcagagcggcggccctggcagcggcggaggcggcagcggcggagggggctcaagattcttgggatttccactgggcgtgggcagcgccatcgcctccggagtggccgtctctaaggtgctgcacctggaaggagaagtgaacaagattaaaagcgccctgctcagcacgaacaaggccgtggtgagcctgagcaatggcgtgtctgtgctgacaagcaaggtgctggacctgaagaactacatcgacaaacaactgctgcctatcgtgaacaagcagtcttgctctatcagcaacatcgagacagtgattgagtttcagcagaagaacaacagactgctggaaatcaccagagagttcagcgtgaacgccggcgtaacaacacctgtgtccacctacatgctgacaaacagcgagctgctgagccttatcaatgacatgcctatcaccaatgaccagaaaaagctgatgagcaacaacgtgcccatcgtgcggcagcagtcatattctatcatgtctatcatcaaggaagaagttctggcttacgtggtccagctgcccctgtacggcgtgattgatacaccatgttggaagctgcacacctctcctctgtgcaccacaaataccaaagaaggcagcaacatctgcctgacccggaccgatagaggctggtactgcgacaacgccggatctgtcagcttcttcccccaggccgagacctgtaaagtgcaatccaacagggtgttctgcgatacaatgaacagcctgacactgcctcctgaggtgaatctgtgtaacgtggacatcttcaaccccaagtacgattgcaagatcatgaccagcaagaccgacgtgtccagctccgtgatcaccagcctgggcgctatcgtgagctgctacggcaagaccaagtgcacagcctctaacaagaaccggggcatcatcaagacattcagcaacggttgtgattacgttagcaacaagggcgtcgacaccgtgtccgttggcaacaccctgtactacgtgaacaagcaggagggcaagagcctgtatgtgaagggcgagcctatcatcaacttctacgaccccctggtgttccctagcgacgagttcgacgccagcatcagccaggtgaacgagaagatcaaccagtctctggcttttatcagaaagtctgatgaactgctg

SEQ ID NO: 125 - DNA, 1401 bp, synthetic construct
  source 1..1401: mol_type = other DNA
cagaacattacagaggagttctaccagagcacatgtagcgctgtgtccaagggctacctgtccgccctgagaaccggctggtacaccagcgtgatcaccatcgagctgagcaacatcaaggagaacaaatgtaacggcaccgacgccaaggtgaagctgatcaagcaagagctggacaagtacaagaacgccgtgaccgaactgcagctgctgatgcagtccggcggacctggcagcggcggtggaggcagtggaggcggaggctctagattcccacctttcctgctgggcgtgggcagtgctatcgccagcggcgtggccgtgagcaaggtgctccacctggaaggcgaagtgaacaagatcaaaagcgccctgctgagcaccaacaaggccgtggtgtccctgtctaatggcgtgtctgtgctgacaagcaaggtgctggacctgaagaactacatcgacaagcaactgctgcctatcgtgaacaagcagagctgcagcatcagcaacatcgaaaccgtgatcgagtttcagcagaaaaacaaccggctgctggagatcacaagagagttcagcgtcaacgccggcgttacaacccctgtgtcgacatacatgctgaccaacagcgagctgctgtctctgatcaatgacatgcccatcaccaacgaccagaagaagctgatgagcaacaacgtgcccatcgtccggcagcagagctacagcatcatgagcatcatcaaggaagaggtgcttgcttatgtggtccagctgcccctgtacggcgttatcgacaccccctgctggaagctgcacacctctcctctgtgcaccaccaataccaaggaaggctccaacatctgcctgacaagaacagatagaggctggtactgcgacaacgccggaagcgtgagctttttccctcaggccgagacctgtaaagtgcagagcaacagggtgttctgcgacactatgaactccctgaccctgcctcctgaggtgaatctgtgtaatgtggacatcttcaaccccaagtacgactgcaagatcatgacatcaaaaaccgatgtgtctagcagcgtgatcacaagcctgggcgccatcgtgtcctgctacggcaagaccaagtgcaccgcctctaataaaaaccggggcatcatcaagaccttctctaatggctgcgattacgttagcaataagggcgtggacaccgtaagcgtgggcaacacactgtactacgtgaacaagcaagaaggcaaaagcctgtatgtgaagggagaacctatcatcaacttctacgatcctctagtctttccatctgatgagttcgacgctagcattagccaggtgaacgagaagatcaaccagtccctggccttcatcagaaagagcgatgagctgctg

SEQ ID NO: 126 - DNA, 1401 bp, synthetic construct
  source 1..1401: mol_type = other DNA
cagaacatcacagaggaattttaccagagcacctgcagcgctgtgtccaagggctacctgagcgccctgagaacaggctggtacacctctgtgatcaccatcgagctgagcaacatcaaggaacccaagtgcaatggcaccgatgccaaggtaaagctgatcaaacaggagttggataagtacaagaatgccgtgaccgagctgcagctgctgatgcagagcggcggtcctggctccggaggcggcggcagcggcggaggcggatctagattccctccattcctgctgggcgtgggcagcgccatcgccagcggagttgctgtgagcaaagtgctgcacctggaaggcgaggtgaacaagatcaagagcgccctgctgtctacaaacaaagctgtggtgtccctgagcaatggcgtgagcgttctgaccagcaaggtcctcgacctgaagaactacatcgacaagcagctgctgcctatcgtgaacaagcaatcttgtagcatcagcaatatcgaaaccgtgatcgagtttcagcaaaagaacaacaggctgctcgaaatcaccagagagttcagcgtgaacgccggagtcaccacacctgtgtccacctacatgctgacaaacagcgagctgctgagcctgatcaacgacatgcccattacaaatgatcagaaaaagctgatgtccaacaacgtgcctattgtgcggcagcaaagctacagcatcatgagcatcatcaaggaagaggtgctggcttacgtggtgcagctgcctctgtacggcgtcatcgacacaccctgttggaagctgcacacaagccctctgtgcaccaccaataccaaggagggctccaacatctgcctgacaagaaccgacagaggctggtactgcgacaacgccggcagcgtgtcattcttcccccaggccgagacctgtaaagtgcagtccaatagagtgttttgcgatacaatgaacagcctgaccctgcctccggaagtgaatctgtgcaacgtggacatcttcaaccccaagtacgactgcaagatcatgaccagcaagacagacgtgtctagttctgttattaccagcctgggagccatcgtgagctgctacggcaaaaccaaatgcaccgccagcaacaagaaccggggcatcatcaagaccttctccaacggatgtgactacgtgtctaacaagggcgtggacaccgtgtctgtcggcaacaccctctactacgtgaacaaacaggaaggcaagagcctgtatgtgaagggagagcctatcatcaacttctatgatcctctggtgttcccatctgatgagttcgacgcctctatcagccaggtgaacgagaagatcaaccagagcctggccttcattcggaagagcgacgagctgctg

SEQ ID NO: 127 - DNA, 1401 bp, synthetic construct
  source 1..1401: mol_type = other DNA
cagaacatcacagaagagttctaccagagcacatgcagtgccgtgagcaagggctacctgagcgctctgcgcaccggctggtacacaagcgtgatcaccatcgagctgagcaatatcaaggagccaaagtgtaatgggacagacgccaaagtcaagctgatcaagcaagagctggacaaatacaagaacgccgtgaccgagctgcagctgctgatgcagagcggcggtcctggctccggcggcggaggcagcggcggcggaggaagcagattccctcccttccctctgggcgtaggcagcgccatcgcctctggcgtggccgtgagcaaggtgctgcacctggaaggcgaagtgaacaagatcaaaagtgccctgttatctacaaacaaagccgtggtgtctctgagcaacggcgttagcgtcctgacctccaaggtgctggacctgaagaattacatcgataagcagctgctgcctatcgtgaataagcaaagctgtagcatcagcaacatcgagacagtgatcgagtttcagcagaagaacaaccggctgctcgaaatcaccagagaatttagcgttaacgccggcgtgaccacccctgtgtccacatacatgctgaccaacagcgagctgctttctctgatcaacgacatgcctatcacaaatgaccagaaaaagctgatgagcaacaacgtgcccatcgtgcggcagcagagctacagcatcatgagcatcatcaaagaagaagtgctcgcttacgtggtgcagctgcccctgtacggcgtgatcgacaccccttgctggaagctgcacaccagcccactgtgtaccaccaataccaaggaaggcagcaacatctgcctgacaagaacagatagaggctggtattgtgataacgctggatctgtgtccttcttcccccaggccgagacttgcaaagtgcaatccaacagagtgttctgcgacaccatgaactccctgaccctgcctcctgaggtgaacctgtgcaacgtggatatcttcaaccccaagtacgactgcaagatcatgacctctaagacagacgtgtctagcagcgtgatcacctcgctgggcgccattgtgagctgctacggcaaaaccaagtgcaccgccagcaacaagaaccggggcatcatcaagaccttcagcaatggctgcgactacgtgtccaacaagggagttgacaccgtgtctgtcggcaacaccctgtactacgtgaataagcaggagggaaagtctctgtatgtgaagggcgagcctatcatcaacttttacgatcctctggtgttccccagcgacgagttcgacgctagcatttctcaggtgaacgagaagatcaaccagtctctggccttcatcagaaaaagcgatgagctgctg

SEQ ID NO: 128 - DNA, 1401 bp, synthetic construct
  source 1..1401: mol_type = other DNA
cagaacatcacggaagagttctaccagagcacatgttctgctgtgagcaagggctacctgtctgccctgagaacaggctggtacaccagcgtgatcacgatcgagctgagcaatatccccgagaacaagtgtaatggcaccgacgccaaggtgaaactgatcaagcaggagctggataagtacaagaacgccgtgaccgagctgcagctgctgatgcagtctggcgggcctggatctggcggcggaggcagcggcggaggaggaagcagattcctgggcttccccctgggcgtgggcagcgccatcgccagcggcgttgctgtctccaaagtgctgcacctggaaggggaagtgaacaaaatcaaaagcgctctgctgtctacaaacaaagccgtggtgtctctgagcaatggcgtgtccgtcctcacatctaaagtgctggacctgaaaaactacatcgacaagcaactgctgcctatcgtgaacaagcagagctgcagcatcagcaacatcgaaaccgtgatcgagtttcagcaaaagaacaacagactgttagaaatcacacgggagttcagcgtgaacgccggcgtgaccactcctgtgagcacatacatgctgaccaatagcgagctcctgagcctgatcaacgacatgcctataaccaacgaccagaaaaagctgatgagcaacaacgtgcctatcgtgcggcagcagagctacagcatcatgagcatcattaaggaagaagtgctggcctacgttgtgcagctgcctctgtatggcgtgatcgataccccttgctggaagctgcacacctctccactttgtaccaccaacaccaaggaaggatctaatatctgcctgaccagaaccgacagaggctggtattgcgacaacgccggaagcgtgagttttttcccacaggccgagacatgcaaggtgcagagcaatagggtgttctgcgacaccatgaacagcctgacactgccccccgaggtgaatctgtgcaacgtggatatcttcaaccctaagtacgactgcaagatcatgacctccaagaccgatgtgtccagctctgtcatcaccagcctgggcgccattgtgagctgctacggcaaaaccaagtgcaccgccagcaacaagaaccggggcatcatcaagacattcagcaacggatgtgactacgtgagcaataagggcgtggacaccgtgtccgtcggaaataccctgtactacgtgaacaagcaggagggcaagtccctgtacgtgaagggcgagcccatcatcaacttctacgatcctctggtgtttcccagcgacgagttcgacgcctctattagccaggtgaacgagaagatcaaccagtcccttgctttcatcagaaagtccgacgagctgctc

SEQ ID NO: 129 - DNA, 1401 bp, synthetic construct
  source 1..1401: mol_type = other DNA
cagaacatcactgaagagttctaccagtctacatgttctgctgtgtcaaagggctacctgagcgccctgagaaccggctggtatacaagcgtgatcaccattgagctgtctaatatcaaggagaacaagtgcaacggaacacctgccaaggtgaaactgatcaaacaggagctggacaagtacaagaatgccgtgaccgagctgcagctgctgatgcagagcggtggacctggctccggcggcggcggatctggcggaggaggaagcagattcctgggcttccctctgggcgtgggcagcgccatcgccagcggcgtagccgtgagcaaggtgctgcacctggaaggcgaggtgaacaagatcaagtccgccctgctgagcacaaacaaagccgtggtctccctgagcaatggcgtgtccgtcctgaccagcaaagtgctggatctgaaaaattacatcgataagcagctgctgcccatcgtgaacaagcagagctgctctatcagcaacatcgaaaccgtgatcgagtttcagcaaaagaacaacagactgctggagatcactcgggaatttagcgtgaacgccggcgtgacaacacctgtgtccacgtacatgctgacaaacagtgaactgctgtctctgatcaacgacatgcctatcaccaatgaccagaagaagctgatgagcaacaacgtgcccatcgtgcggcagcagagctacagcatcatgtccatcatcaaagaggaagtgctggcctacgtggtgcaactgcctctgtacggcgttatcgacaccccttgctggaagctgcacaccagccctctgtgtacaaccaacaccaaggaaggcagcaatatctgcctgaccagaacagacagaggctggtactgcgacaacgctggctctgtgtccttcttcccccaggccgagacctgcaaggtgcagagcaacagggtgttctgcgacaccatgaacagcctgaccctgccacctgaggtgaatctgtgtaatgtggacatcttcaaccccaagtacgactgcaagatcatgacctctaaaacagatgtgtctagctcagtgatcaccagcctgggcgccatcgtgtcttgctacggcaaaaccaagtgtaccgctagcaacaagaaccggggcatcatcaagaccttcagcaacggatgtgactacgtgagcaacaagggcgttgataccgtgtccgtgggcaacaccctgtactacgtgaacaagcaagagggcaagagcctgtacgtgaagggcgagcccattattaacttctatgatcctctcgtgttcccatctgacgagttcgacgccagcatcagccaggtgaacgagaagatcaaccagagcctggcttttatcagaaagagcgatgagcttctg

SEQ ID NO: 130 - DNA, 1401 bp, synthetic construct
  source 1..1401: mol_type = other DNA
cagaacattacagaagagttctaccagagcacctgttctgccgtgagcaagggatatctgagcgccctgcggaccggctggtacaccagcgtgatcacaattgagctgagcaacatcaaggaaaacaagtgcaacggcaccgatgccaaggtgaaactgatcaagcaagagttggataagtacaagaacgccgtgaccgagttgcagctgctcatgcagtctggcggacctggcagcggcggcggcggctcgggcggcggaggcagcagattccttggcttcccactgggcgtcggcagcgccatcgcctctggagttgctgtgtctaaggtgctgcacctggaaggcgaggtgaacaagatcaagagcgctctgctgtctaccaacaaagccgttgtgagcctgagcaacggcgtgagcgtcctgacaagcaaggtgctggacctgaaaaattacatcgacaagcagctgctgccaattgtgaacaaacagagctgcagcatccccaacatcgaaaccgtgatcgagtttcagcagaagaacaacagactgcttgagatcacccgggaatttagcgtgaatgccggagtgacaacccctgtgagcacatacatgctgaccaacagcgagctgctgagcctgatcaatgacatgcctatcacaaacgaccagaaaaagctgatgagcaataacgtgcagatcgtcagacagcagtcctacagcatcatgagtatcatcaaagaagaggtgctggcctacgtggtgcagctgcctctgtatggcgtgatcgacacaccttgttggaagctgcacacctcccccctgtgcaccaccaacaccaaggaaggctccaacatctgcctgaccagaaccgacagaggatggtactgcgacaacgccggcagcgtcagcttcttcccccaggccgagacatgcaaggtgcaaagcaatagagtgttctgcgacaccatgaacagcctcacactgccttctgaggtgaatctgtgtaacgtggacatcttcaaccccaagtacgactgcaagatcatgacctctaagacagatgtgtccagctccgtgatcaccagcctgggcgccatcgtgagctgctacggcaagaccaagtgcaccgcttctaacaagaaccggggcatcattaaaaccttttctaatggctgtgactacgtgagcaacaagggcgtggatacagtgagcgttggaaataccctgtactacgtgaacaagcaagagggcaaatctctgtacgtgaagggcgagcctatcatcaacttctacgaccccctggtgttccctagcgacgagttcgatgcctctatcagccaggtgaacgagaagatcaaccagtctctggccttcatcaggaagtccgatgagctgctg

SEQ ID NO: 131 - DNA, 1401 bp, synthetic construct
  source 1..1401: mol_type = other DNA
cagaacatcacagaggaattttaccagagcacctgcagcgccgtgtccaagggctacctgtctgctctgcggaccggctggtatacaagcgtgatcacaatcgagctgagcaatatcaaggaacctaagtgcaacggcaccgacgccaaggtgaagctgatcaaacaggagctggataagtacaagaacgccgtgacagagctgcagctgctgatgcagagcggaggccctggcagcggcggcggcggcagcggcggcggaggcagtagattcctgggatttcctctgggcgtgggcagcgctatcgcctcaggcgtggccgtctccaaggtgttgcatctggaaggcgaggtcaacaagatcaaaagcgctctgctgtctaccaacaaggccgttgtgtccctgagcaacggcgtcagcgtgctgacctctaaggtgctggacctgaaaaactacatcgacaagcaactgttgccaatcgtgaataaacagagttgcagcatccccaacatcgaaaccgtgatcgagttccaacagaaaaacaacagactgctggaaataacacgggaatttagcgtgaacgccggcgtgaccacccctgtgtctacgtacatgctgacaaacagcgagctgctgagcctgatcaacgacatgcctatcaccaatgaccagaagaagctcatgagcaacaacgtgcagatcgtcagacagcagtcttacagcatcatgagcatcatcaaggaagaggtgctggcctacgtggtgcagctgcctctgtacggcgtgatcgataccccatgttggaagctgcacaccagccctctgtgcaccacaaacaccaaggaaggcagcaatatctgcctgaccagaactgacagaggatggtactgcgacaacgccggaagcgtgtcattcttcccccaggccgagacatgtaaagtccaatctaaccgggtgttctgcgacacaatgaacagcctgaccctgccttctgaggtgaacctgtgcaatgtagatatcttcaaccccaagtacgactgcaagatcatgacctccaaaaccgacgtgtctagcagcgtgatcacctccctgggcgccattgtgtcctgctacggcaagaccaagtgtacagcctctaacaagaatcgcggtatcatcaagacatttagcaacggttgcgattacgttagcaacaaaggcgtggataccgtgtccgtgggaaatacactgtattacgtgaacaaacaggagggcaagagcctgtacgttaagggcgaacccatcattaacttctatgaccccctggtgttccccagcgacgagttcgacgccagcatctcccaggtgaacgagaagatcaaccagtctctcgccttcatcagaaagagcgatgagctcctg

SEQ ID NO: 132 - DNA, 1401 bp, synthetic construct
  source 1..1401: mol_type = other DNA
cagaacatcaccgaggagttctaccagagcacctgttctgccgtgtctaaaggctacctgtctgccctcaggaccggctggtacacctccgtgatcaccatcgagctgagcaatatcaaggagcctaagtgcaacggcaccgacgccaaggtgaagctgattaagcaggagctggataagtacaagaatgccgtgaccgagctgcagttgctgatgcagtccggcggaccaggcagcggcggcggcggctccggcggaggaggctctagattcctgggcttccctctgggcgtgggcagcgctatcgccagcggcgtggccgtgagcaaagtgctgcacctggaaggagaagtgaacaagatcaagagcgccctgctgtctaccaacaaggccgtcgtgtccctgtccaacggcgtttctgtgctgacttccaaggtgctggacctgaagaactacattgacaagcagctgctgcccatcgtgaacaagcagagctgcagcatccccaacatcgaaaccgttatcgagtttcagcagaaaaacaaccggctgctggaaatcacccgggagtttagcgtgaatgccggagtgacaacccctgtgagcacatacatgctgacaaacagcgagcttctgtcgctcatcaacgatatgcctatcacaaacgatcagaaaaagctgatgagcaacaacgtgcaaatcgtgcggcagcagagctacagcatcatgagcatcatcaaggaagaagtgctggcttatgtcgtgcagctgcccctgtatggcgtgattgacaccccttgttggaagctccacacatcacctctgtgtaccaccaataccaaagaaggcagcaacatctgcctgacaagaacagatagaggctggtactgcgacaacgccggcagcgtgtcctttttcccacaggccgagacatgtaaggttcaaagcaatagagtgttctgcgacaccatgaacagcctgaccctgcctccagaggtgaatctgtgcaacgtggacatcttcaaccccaagtatgattgcaagatcatgaccagcaagaccgacgtgagctctagcgtgatcaccagcctgggcgctatcgtcagctgctacggaaaaacaaagtgcacagctagcaacaagaatagaggaatcatcaagaccttcagcaacggctgcgactacgtgtctaataaaggcgtggacacagtgtctgtgggcaacaccctgtactacgtgaacaaacaagagggcaagtctctgtacgtgaaaggcgaacctatcatcaacttctacgaccccctggtgttccccagcgacgagttcgacgccagcatcagccaggtgaacgagaagatcaaccagagcctggccttcatcagaaagagcgatgagttactg

SEQ ID NO: 133 - DNA, 1401 bp, synthetic construct
  source 1..1401: mol_type = other DNA
cagaacatcacagaagagttttaccagtcaacatgcagcgccgtgtctaagggatatctgagcgctctgagaaccggctggtacacctctgtgatcaccatcgagctgagcaacatcaaggaacccaaatgcaacggaacagatgccaaggtgaagctgatcaagcaagagctggacaagtacaaaaacgccgtcaccgagttgcagctgctgatgcagagcggaggcccaggctctggcggcggcggcagcggaggcggtggcagcaggttcctgggcttcccactgggcgtcggcagcgccatcgccagcggcgtggccgtgtccaaagtgctgcacctggaaggcgaggtgaacaagatcaagtccgccctgctgagcaccaacaaggccgtcgtgtctctgtctaatggagtgagcgtgctgaccagcaaggtgctggatctgaagaactacatcgataagcagctgttgcctattgttaataagcagagctgttctatccccaacatcgagacagtgatcgagttccagcagaaaaacaacagactgctggaaatcactagagagttcagcgtgaacgccggcgtgacaacacctgtgagcacctacatgctgaccaatagcgagctgctgtccctgatcaacgacatgcctatcacaaacgaccagaagaagctgatgagcaacaacgtgcccatcgtgcggcagcaaagctacagcatcatgtctatcattaaagaggaagtgctggcttacgttgtgcaactgcccctgtatggagtgatcgataccccttgttggaagctgcacacttcccccctgtgcacaaccaataccaaggaaggctccaacatctgcctgaccagaacagatagaggctggtattgcgacaacgctggcagcgtgtccttcttccctcaggccgagacatgcaaagtgcagtctaatagagtgttttgcgacacaatgaacagcctgaccctgccttctgaggtgaatctatgtaacgtggacatcttcaacccaaagtacgactgcaagatcatgacatctaagaccgacgtgtccagcagcgtgatcaccagcctcggtgccatcgtgtcctgctacggaaagacaaagtgcaccgccagcaacaagaaccggggcatcatcaagaccttttctaacggctgtgactacgtcagcaataaaggcgtggacaccgtgtctgtgggcaacaccctgtactacgtgaacaagcaggagggcaagagcctgtacgtgaaaggcgaacctattatcaacttctacgaccccctggtgttccctagcgacgagttcgacgctagcattagccaggtgaacgagaagatcaaccagagcctggccttcatccggaagtccgatgagctgctc

SEQ ID NO: 134 - DNA, 1401 bp, synthetic construct
  source 1..1401: mol_type = other DNA
cagaacatcaccgaggaattttaccagagcacctgttctgctgtgagcaagggctacctgagcgccctgagaacaggctggtacaccagcgtgatcaccatcgagctgtccaacatcaaggaacctaagtgcaacggtacagacgccaaggtgaaactgatcaagcaagagctcgataagtacaagaacgccgtgacagagctgcagctgctgatgcagagcggcggacctggaagtggcggcggcggcagcggcggaggcggctcaagattccctcctttcctgttgggcgttggatctgctatcgccagcggagttgctgtcagcaaagtgctgcacctggaaggcgaagtgaacaagatcaaaagcgccctgctgagcaccaacaaggcggtggtgagtctgtcgaatggcgtgagcgtgctgaccagcaaggtgctggacctgaaaaactacatcgacaagcagctgctgccaattgtgaacaagcagtcttgtagcattcctaacatagaaaccgtgatcgagttccagcaaaagaacaataggctgcttgaaatcacccgggagttcagcgtgaacgctggcgtgaccacccccgtgtccacatacatgctgacaaacagcgagctgctgtctctgatcaatgatatgcctatcaccaacgaccagaaaaagctgatgagcaacaacgtgcagatcgtcagacagcagagctacagcatcatgagcatcatcaaggaagaggtgctggcctacgtggtgcagctgcccctgtatggagtgatcgacaccccttgttggaagctgcataccagccctctgtgtaccacaaataccaaagagggctctaacatctgcctgaccagaactgatagaggatggtattgcgacaacgccggcagcgtgtctttctttccacaggccgagacgtgcaaggtgcagagcaaccgggtgttctgtgataccatgaacagcctgaccctgcctccagaggtgaatctgtgcaacgtagacatcttcaaccccaagtacgactgcaaaattatgacatctaagacagacgtgtcctctagcgtcatcacatccctgggcgccatcgtgtcctgctacggcaaaacaaagtgcaccgccagcaacaagaaccggggcatcatcaagaccttcagcaatggctgcgactacgtgagcaataagggcgtcgacacagtgtcggtgggcaacaccctgtactacgtgaacaagcaggagggcaagtccctgtacgtgaagggcgagcccatcatcaatttctacgatcctctggtgttccccagcgacgagttcgacgccagcatcagccaggtgaacgagaagatcaaccagagcctggccttcatcagaaagtccgatgaactgctc

SEQ ID NO: 135 - DNA, 1401 bp, synthetic construct
  source 1..1401: mol_type = other DNA
cagaacatcaccgaggaattttaccagagcacatgcagcgctgtgtccaagggctacctgtctgctctgcggacaggctggtacaccagcgtcatcaccatcgagctgagcaacatcaaagaacctaagtgtaacggcaccgatgccaaggtgaagctgatcaagcaggagctggataagtacaagaatgccgtgaccgagctccagctgctgatgcagtctggaggacctggcagcggcggcggaggctctggcggcggcggaagcagattcccaccattccctctgggcgtgggcagcgctatcgccagcggcgtggccgtgtccaaggtgctgcacctggaaggcgaagtgaacaagatcaagagcgccctgctgtccaccaacaaggccgtagtgtctctgagcaatggcgtgagcgttctgacatctaaggtgctggacctgaagaactacatcgataagcaactgctgcccatcgtgaacaagcagagctgttccatccctaacattgagacagtgatcgagttccagcagaagaacaaccggctgctggaaatcaccagagagttcagcgtgaatgccggagtcacgacccctgtgagcacctacatgctgaccaactccgagctgctgagcctgatcaatgacatgcctatcaccaacgaccagaaaaagctgatgagcaacaacgtgcagatcgtgcggcagcagtcctacagcatcatgagtatcatcaaggaagaagtgctggcctatgtggtgcaactgcctctgtatggcgtgatcgacaccccctgctggaagctgcacacctcccctctctgtaccacaaataccaaggaaggctctaatatctgcctgaccagaacagatagaggctggtattgcgacaacgccggcagcgtgtccttcttcccgcaagccgagacatgcaaagtgcagagcaatagagtgttctgcgacacaatgaactcactgacactgcctcctgaggtgaacctgtgcaacgtggacatcttcaaccccaagtacgactgcaagattatgaccagcaagacagacgtgagctctagcgtgatcacaagcctgggcgccatcgtgagctgctacggcaagaccaagtgcaccgccagcaacaagaacaggggcatcatcaagacctttagcaacggttgtgactacgtgagcaacaaaggcgtggatacagtgagcgtcggcaacacactgtactacgtgaacaaacaggagggaaagagcctgtacgtgaaaggagaacccattatcaacttctacgaccccctggtctttcctagcgacgagttcgacgcctctatcagccaggtgaacgagaagatcaaccagtctttggcttttatcagaaaatctgatgagctgctg

SEQ ID NO: 136 - DNA, 1401 bp, synthetic construct
  source 1..1401: mol_type = other DNA
cagaacattaccgaggagttctaccagtctacatgcagcgccgtgagcaagggatacctgagcgctctgagaaccggctggtacacctccgtgatcaccatcgagctgtccaatatcaaggaacctaagtgtaacggcacagacgccaaggtgaaactgatcaagcaggagttggataagtataagaatgccgtgaccgagctgcagctgctgatgcagagcggcggacctggcagcggcggaggaggcagcggcggcggcggcagcagattcctgggcttccctctgggagttggcagcgccatcgccagcggcgtcgccgtgagcaaggtgctgcacctggaaggcgaagtgaacaaaatcaagtcagctctgctgtccaccaacaaggccgtggtgtctctgagcaacggcgtgtccgtgctgacctctaaagtgctggacctgaagaactacatcgacaagcagctgctgcccatcgtgaacaaacaatcttgtagcatcccaaatatcgagacagtgatcgagtttcagcaaaagaacaaccggctgctcgaaatcaccagagagttcagcgtgaatgccggcgttaccacccctgtgagcacatacatgctgaccaatagcgagctgcttagccttatcaacgacatgcctatcacaaatgaccagaaaaagctgatgagcaacaatgtgcccatcgtcagacagcagagctactctatcatgtctattatcaaagaggaagtgctggcttacgtggtgcaactgcctctgtatggagtgatagatacaccgtgctggaagctgcacaccagtccactgtgtaccaccaacaccaaggaaggcagcaatatctgcctgacaagaacagatcgcggctggtactgcgacaacgcaggcagcgtgtcattcttcccccaggccgagacatgcaaggtgcagagcaatcgggtgttctgcgataccatgaacagcctgaccctgcctcctgaggtgaacctgtgcaacgtggacatcttcaaccccaagtacgactgcaagatcatgaccagcaaaaccgatgttagttctagcgtgatcacatctctgggcgccattgtgagctgctacggcaaaaccaagtgcacagcctctaacaagaacagaggcatcatcaagacctttagcaacggctgtgactacgtgtccaacaagggcgtcgacaccgtgagcgtgggcaacaccctgtattacgtgaacaagcaggagggcaagagcctgtacgtgaagggggaacctatcatcaacttctacgaccccctggtgtttccttctgatgagttcgacgcttccatcagccaggtgaacgagaagatcaaccagagcctggccttcatccggaagagcgacgagctcctg

SEQ ID NO: 137 - DNA, 1401 bp, synthetic construct
  source 1..1401: mol_type = other DNA
cagaacatcacagaggagttctaccagagcacctgctccgctgtgtccaagggatacctgagcgccctgagaaccggctggtataccagcgtgattaccatcgagctgagcaacattaaagaacccaagtgcaacggcaccgacgccaaggtgaaactgatcaagcaagagttggataagtataagaatgctgttacagagctccagcttctgatgcagtctggcggtcctggcagcggcggcggcggcagcggcggaggcggcagcagattccctccattcctgctgggcgtcggatctgcaatcgcctctggcgtggccgtgtctaaagtgctgcacctggaaggcgaagtgaacaagatcaagtctgccctgctgtctacaaacaaggccgtcgtgagcctgagcaatggcgtgtctgtgctgaccagcaaggtgctggacctgaagaactacatcgacaagcagctgctcccaatcgtgaacaagcagtcttgttccatccccaacatcgagactgtgatcgagtttcagcagaagaacaacagactgctggaaatcactcgggaatttagcgtgaatgctggcgtgaccacccctgtgtccacctacatgctgacaaacagcgagctcctgagcctgatcaatgatatgcctatcacaaacgaccagaagaagctgatgagcaacaacgtgccaatcgtgcggcagcaaagctacagcatcatgagcatcatcaaggaagaggttctggcttacgtggtgcagctgcctctgtatggcgtgattgataccccttgctggaagctgcacaccagccctctgtgcacaaccaataccaaggaaggcagcaacatctgcctgaccaggaccgatagaggctggtactgcgacaacgccggcagcgtgtcattcttcccccaggccgagacatgcaaggttcaatctaatagagtgttctgcgacaccatgaacagcctgacactgcctcctgaggtgaacctgtgtaatgtggacatcttcaaccccaagtacgactgcaagatcatgaccagcaagaccgacgtgtccagcagcgtcatcacctccctgggagccatcgtgagctgctacggcaaaaccaagtgtacagcctctaacaaaaaccggggcatcatcaaaaccttcagcaatggttgtgactacgtgagcaacaagggagtggatacagtgagcgtgggcaacaccctgtactacgtgaacaagcaggagggcaaatccctgtacgtgaagggcgagcctattatcaacttctacgaccccctggtgttccccagcgacgagttcgacgccagcatcagccaggtgaacgagaagatcaaccagagcctggccttcatcagaaagtccgatgagctgctg

SEQ ID NO: 138 - DNA, 1401 bp, synthetic construct
  source 1..1401: mol_type = other DNA
cagaacatcaccgaggagttctaccaatctacatgttctgctgtgagcaagggctacctgagcgccctgagaaccggctggtacacctctgtcattaccatcgagctttccaacatcaaagaacccaagtgcaatggcaccgatgccaaggtgaagctgatcaaacaggagctggacaagtacaaaaacgccgtgaccgagttgcagctgctgatgcagagcggcgggcctggcagcggcggtggaggcagcggcggcggcggttctaggttccctccattccccctgggcgttggcagcgccatcgccagcggcgtggccgtgtccaaagtgctgcacctggaaggagaagtgaacaagatcaagagcgccctgctgagtaccaacaaggctgtggtgagcctgtccaatggagtttctgtgctgaccagcaaggtgctggatctgaagaactacatcgataagcagctgctgcctatcgtgaacaagcagtcttgtagcatccctaatatcgagacagtgatcgagttccagcagaaaaacaaccggctgctggaaatcacacgggaatttagcgtgaatgctggcgtgaccacccccgtgtccacctacatgctgactaactccgagctcctgtccctgatcaatgacatgcctatcaccaacgaccagaagaagctgatgtccaacaacgtgccaatcgtacggcagcagagctacagcatcatgagcatcatcaaggaagaggtgctggcctacgtcgtgcagctgccgctgtacggcgtcatcgacacaccctgctggaagctgcacaccagccctctgtgcaccaccaataccaaggagggcagcaacatctgcctgaccagaacagacagaggatggtattgtgataacgccggcagcgtgtctttcttccctcaggccgagacatgcaaggtgcagagcaatagagtgttctgcgacacaatgaacagccttaccctgcctcctgaggtgaacctgtgtaacgtggacatcttcaaccctaagtatgactgcaagatcatgacatctaagaccgacgtgtcaagcagcgtgatcaccagcctgggagccatcgtgagctgctacggcaagaccaagtgcaccgccagcaacaaaaacagaggcatcatcaaaacattcagcaacggctgcgactacgtgagcaacaagggcgtggataccgtgtctgtgggcaacaccctgtattacgtgaacaagcaagagggcaagagcctgtacgtcaagggcgaacctatcatcaacttctacgaccccctggtgttccccagcgatgagtttgacgcctctatctcccaggtgaacgagaagatcaaccagtccctggcttttatcagaaagagcgacgagctgctg

SEQ ID NO: 139 - DNA, 1401 bp, synthetic construct
  source 1..1401: mol_type = other DNA
cagaacatcactgaggagttctaccagtccacctgtagcgctgtgtctaagggatacctgagcgctctgagaaccggctggtacacatctgtgatcacaatcgagctgtctaatatcaaggaacctaagtgtaacggcaccgacgccaaggttaagctgatcaagcaagaactggataagtacaagaacgccgtgaccgagctccagctgctgatgcagtctggcggacctggcagcggcggaggcggttcaggcggcggcggcagtagattcctgggatttccactgggcgttggcagcgccatcgccagcggcgtcgccgtgagtaaagtgctgcacctgcccggcgaagtgaacaagatcaagtcagctctgctgagcaccaacaaggccgtggtgagcctcagcaacggagtgtccgtgctgacaagcaaggtcctcgacctgaagaattacatcgacaagcagctgctgcctatcgtgaacaagcagagttgcagcatcagcaacatcgaaaccgtgatcgagttccagcaaaagaacaaccggctgctggagatcacaagagagttcagcgtgaatgccggagtgacaacacctgtgtctacatacatgctgaccaacagcgagctgctgtccctgattaacgacatgcctatcaccaatgaccagaaaaagctgatgagcaataacgtgcccatcgtgcggcagcagagctacagcatcatgagcatcatcaaagaagaagtgctggcctacgtggtacagctgcctctgtatggcgtgattgacaccccttgctggaagctgcacaccagccctctgtgcaccacaaacacaaaggaaggctctaatatctgcctgacccggaccgatagaggctggtactgcgacaacgccggcagcgtgtctttcttcccccaggccgagacatgcaaggtgcaaagcaatcgggtgttctgcgataccatgaacagcctgacactgccaccagaggtgaatctgtgtaacgtggatatcttcaaccccaaatacgactgcaagatcatgaccagcaaaaccgacgtgagctcctccgtgatcaccagcctgggcgctatcgtgtcctgctacggcaagaccaagtgcaccgctagcaacaaaaacagaggaatcatcaagacctttagcaatggctgtgattacgtgtctaacaaaggcgtggacaccgtgagcgtgggcaacaccctgtactacgtgaacaagcaggagggcaaaagcctgtacgttaagggcgagcctatcatcaacttctacgaccccctggtgttccctagcgatgagttcgacgccagcattagccaggtgaacgagaagatcaaccagagccttgccttcatcaggaagtccgacgagctgctg

SEQ ID NO: 140 - DNA, 1401 bp, synthetic construct
  source 1..1401: mol_type = other DNA
cagaacatcacagaagagttctaccagagcacctgttctgctgtgtctaagggctacctgagcgctctgagaaccggatggtatacatcagtgatcacaatcgagctgagcaacatcaaggaacctaagtgcaacggcaccgatgccaaggtgaaactgatcaagcaagagctggataagtataagaatgccgtgaccgagctgcagctgctgatgcagagcgggggccctggcagcggcggcggaggcagcggcggcggcggatctagattccctcctttcctgctgggagtcggcagcgccatcgcctccggcgtggccgtgtccaaggtgctgcacctgcccggcgaggtgaacaagatcaagagtgccctgctcagcaccaacaaggccgtggtgtccttaagcaatggcgtgagcgtgctgaccagcaaggttctggacctgaagaactatatcgacaagcagctcctccccatcgtgaacaagcagagctgcagcatcagcaatattgagacagtgatcgaatttcagcagaagaacaacagactgctggaaatcacaagagagttcagcgtgaatgccggcgtgacaacacctgtgagcacctacatgctgaccaactctgagctgctctctctgatcaatgacatgcctatcacaaacgaccagaaaaagctgatgtctaacaacgtgcccatcgtgcggcagcaatcctacagcatcatgagcatcatcaaggaagaggtgctggcctacgtcgtgcagctgccactgtacggcgtgatcgacaccccgtgctggaagctgcacacaagccctctgtgcaccaccaataccaaggaaggcagcaacatctgcctgacacggacagatagaggctggtactgcgacaacgcaggcagcgtgtcattcttcccccaggccgagacatgcaaggtgcagtctaatagagtgttctgtgataccatgaacagcctgaccctgccacctgaggtgaacctgtgtaatgtggacatcttcaaccccaagtacgactgcaagatcatgaccagcaagaccgatgtgtccagcagcgtgatcacaagcctgggcgccattgtgtcctgctacggcaaaacaaagtgcaccgccagcaacaagaaccggggcatcatcaaaaccttcagcaacggctgtgactacgtgtctaacaaaggcgttgataccgtctccgttggcaacaccctgtactacgtgaacaaacaggagggcaaatccctgtacgtgaaaggcgagcctatcattaacttttacgatcctctggtctttccaagcgacgagttcgacgctagcatctctcaagtgaacgagaagatcaaccagagcctggctttcatccgcaagagcgacgagctgctg

SEQ ID NO: 141 - DNA, 1401 bp, synthetic construct
  source 1..1401: mol_type = other DNA
cagaacattaccgaggaattttaccagagcacctgtagcgccgtgagcaaagggtacctgtctgctctgagaacaggctggtatacaagcgtgatcaccatcgaactgagcaatatcaaagagcctaagtgcaacggcaccgacgccaaggtgaagctgatcaagcaggagctggataagtacaagaacgccgtgacagagctgcagctgctgatgcagtctggaggtcctggaagcggcggaggcggctctggcggaggcggctctagattccctcccttccctctgggcgtgggcagcgccatcgccagcggcgtggccgtgtctaaagtgctgcacctgcctggcgaggtgaacaagattaagagcgctctgctgagcactaacaaggccgtcgtgagcctgtctaacggcgtttccgtgctgacaagcaaggtactggacctgaagaattacatcgacaagcaactgctgcccatcgtgaacaaacaaagctgcagcatctccaatatcgagacagtgatcgagtttcagcaaaagaacaacagactgctggaaatcaccagagagttcagcgtgaatgccggcgtgaccacccctgtgtctacatacatgctgaccaacagcgagctgctgagcctgatcaatgatatgcctatcaccaacgaccagaaaaagctcatgagcaacaacgtgcccatcgtgcggcagcagtcctacagcatcatgagcatcattaaggaagaggtcttggcctatgtggtgcagctgcctctgtacggcgtgatcgatacaccatgttggaagctgcacaccagccccctctgcaccacaaacaccaaggaaggcagcaatatctgcctgacccggaccgatagaggctggtactgcgataacgctggcagcgtgagcttcttccctcaggccgagacctgcaaggtgcagagcaacagagtgttctgcgacaccatgaactctttgaccctgcctccagaagttaacctgtgtaatgtagacatcttcaaccccaagtacgactgcaagatcatgacaagcaagaccgacgtgagcagctccgtgatcaccagcctgggagccatcgtgtcttgttacggcaagacaaagtgtacagcctctaacaagaaccggggcattatcaagaccttttctaacggctgcgactacgtctccaacaaaggcgtcgacacagtgtccgtgggcaacaccctgtactacgtgaacaagcaggagggcaaaagcctgtacgtgaagggcgaacctatcatcaacttctacgaccccctggtgttcccaagcgacgagttcgacgccagcatcagccaggtgaacgagaagatcaaccagagcctggctttcatcaggaagtctgatgagctgctg

SEQ ID NO: 142 - DNA, 1401 bp, synthetic construct
  source 1..1401: mol_type = other DNA
cagaacatcaccgaggagttctaccagagcacttgcagcgccgtgagcaagggctacctgtctgctcttagaaccggatggtacaccagcgtgatcacaatcgagctctccaacatcaaggaacccaagtgtaatggcaccgatgctaaggtgaaactgatcaaacaagagttggataaatataagaacgccgtgaccgagctgcagctgctcatgcagagcggcggtcctggcagcggcggcggaggttctggcggcggaggctcaagattcctgggcttccccctgggcgtgggctctgctatcgcctctggcgtcgccgtgtcaaaggtgctgcacctgcccggcgaggtgaataaaatcaagagcgccctgctgagcaccaacaaagccgtggtgtccctgagcaacggcgtgagcgtgctgacaagcaaggtgctggatctgaagaactacattgataagcagctgctgcctattgtgaacaagcaaagctgctctatcccaaatatcgaaacagtgatcgagtttcagcagaagaacaacaggctgctggaaatcacaagagagttcagcgtgaacgctggcgtcaccacccctgtgagcacatacatgctgaccaacagcgagctgctgtctctgattaacgacatgcctatcacgaatgatcagaaaaagctgatgagcaataatgtgccaatcgtgcggcagcagtcctacagcatcatgagcatcatcaaggaggaagtgctggcctacgtggtgcagctgcctctgtacggcgttatcgacaccccttgctggaagctgcacacgtcccctctgtgtaccaccaacaccaaggaaggctctaacatctgcctgaccagaacagatagaggctggtactgcgacaacgccggcagcgtgagcttcttccctcaggccgaaacctgcaaggtccagagcaaccgggtgttttgcgacactatgaacagcctgacactgccacctgaggtaaacctgtgcaacgtggacatcttcaaccctaaatacgactgtaagatcatgacctctaaaaccgacgtgagcagctctgtgatcacctccctgggcgccatcgtgagctgttacggcaagacaaagtgcacagcctccaacaagaatagaggcatcatcaagaccttcagcaacggatgtgactacgtgagcaataagggagtggacaccgtgtctgttggcaacaccctgtactacgtgaacaagcaggagggaaagagcctgtacgtcaagggcgaacctatcatcaacttctacgaccccctggtgttccccagcgacgagttcgacgccagcatctcacaagtgaacgagaagattaaccagagcctggccttcatcagaaagtccgatgagctgctc

SEQ ID NO: 143 - DNA, 1401 bp, synthetic construct
  source 1..1401: mol_type = other DNA
cagaacatcaccgaggagttctaccagagcacctgtagcgccgtctccaagggctacctgagcgctctgagaacaggctggtacaccagcgtgatcaccattgagctgtctaatatcaaggaacctaagtgtaatggcaccgatgccaaggtgaaactgattaagcaggagctggataagtacaagaacgcggtgacagagctgcagctgctgatgcagagcggaggacctggcagcggaggcggcggcagcggaggaggcggttctagattccctccattcctgctcggcgtcggctctgccatcgccagtggcgtggccgtgagcaaggtgctgcacctgcccggagaggtcaacaagatcaagtctgccctgcttagcaccaacaaagccgtggtgtcactgagcaatggcgtttccgtcctgacatccaaggtgctggacctgaaaaactacatcgacaagcaactgctgcctatcgtgaacaagcagtcctgcagcatccccaacatcgagacagtgatcgagttccagcaaaagaacaatagactgctggaaatcactagagagttcagcgtgaatgctggcgtgaccacccctgtgagcacctacatgctgaccaacagcgagctgctgagcctgatcaacgacatgcctataacaaatgaccagaaaaagctgatgtctaacaacgtgcccatcgtgcggcagcagtcatattctatcatgtccatcatcaaggaggaagtgctggcctacgtggtgcagctccctctgtacggcgtgatcgacaccccgtgctggaagctgcacaccagccctttgtgcaccaccaataccaaggaaggctctaacatctgcctgaccaggacagatagaggctggtattgcgacaacgccggctctgttagcttcttcccacaggccgagacatgtaaagtgcagagcaaccgggtgttctgtgacaccatgaacagcctgaccctgcctcctgaagtgaacctgtgcaatgtggacatcttcaaccccaagtacgattgcaagatcatgaccagcaagaccgacgtgtccagcagcgtgatcaccagcctgggcgccatcgtgtcttgttacggcaagacaaagtgcacagccagcaacaaaaacagaggcatcatcaagacatttagcaacggctgcgactacgtgagcaacaagggagtggatacagtgtctgtgggcaacaccctgtactacgtgaacaaacaggagggaaaaagcctgtacgtgaagggcgagcctatcattaacttctacgaccccctggtgtttcccagcgacgagttcgacgccagcatcagccaggtcaacgagaagatcaaccagagcctggcttttatccggaagtccgatgagctgctg

SEQ ID NO: 144 - DNA, 1401 bp, synthetic construct
  source 1..1401: mol_type = other DNA
cagaacatcacggaagaattttaccagagcacctgtagcgctgtgagcaagggctacctgtctgctctgaggaccggctggtacacctccgtgatcaccatcgagctgtccaacatcaaggagcctaagtgcaatggcaccgatgccaaggtgaagctgatcaagcaggagctggacaagtacaagaacgctgtgaccgaactgcagctgctgatgcagtctggcgggcctggctctggaggcggaggcagcggcggtggcggaagcagattcccacctttccctctgggcgttggaagcgccatcgccagcggcgtggccgtgtccaaggtgctgcacctgcccggcgaggtgaacaagattaagagcgccctgctcagcaccaacaaggccgtcgtgagcctgtccaacggcgtgtctgtgctgacatctaaagtgctggacctgaagaattacatcgataagcagctgctgcctatcgtgaacaagcaaagctgctcaatccccaacatcgaaaccgtgatcgagtttcagcaaaaaaacaacagactgttggagatcactcgggaatttagcgtgaacgccggagtaacaacacctgtgtctacctacatgctgacaaatagcgagctgctgtctctgatcaacgacatgcctatcaccaatgaccagaagaagctaatgagcaacaacgtgcctatcgtgcggcagcagtcctacagcatcatgtctatcatcaaagaagaggtgctggcctatgtggtgcagctgcctctgtatggcgtgatcgacacaccgtgctggaagctgcacacaagccctctgtgtacaaccaataccaaggaaggcagcaatatctgcctgacaagaaccgatagaggctggtactgcgacaacgccggcagcgtgagcttcttcccccaggccgagacatgcaaggtgcagagcaatagagtgttctgcgacaccatgaacagcctgacactgcctccagaggtgaatctgtgcaacgtggacatcttcaaccccaagtatgattgcaagatcatgaccagcaagacagatgtgtccagcagcgtgatcaccagcctgggcgccatcgtttcttgttacggcaaaaccaaatgcaccgcctccaataaaaaccggggcatcattaagaccttcagcaacggctgtgactacgtgtccaacaaaggagtcgacaccgttagcgtcggcaacaccctgtactacgtgaacaagcaggagggcaagagcctgtacgtgaaaggcgaacctatcattaacttctacgaccccctggtgttccccagcgacgagttcgacgccagcatctctcaggtgaacgagaagatcaaccagagcctggctttcatcagaaagtctgatgagcttctg

SEQ ID NO: 145 - DNA, 1401 bp, synthetic construct
  source 1..1401: mol_type = other DNA
cagaacatcacagaggagttctaccagtctacctgttcggctgtgtctaagggctacctgagcgctctgagaactggatggtatacatctgtgatcaccatcgagctgtccaacatcaaggagcctaagtgtaacggcaccgacgccaaggtgaagctgatcaagcaggagctggataagtacaagaacgccgtgaccgagctccagctgctgatgcagagcggcggtcctggcagcggcggcggcggcagcggcggaggaggcagcagattcctgggattcccactgggcgtgggcagcgccatcgcctctggcgtggccgtgagcaaggtgctgcacctgcctggcgaggtgaacaaaattaaaagcgccctgctgagcaccaacaaggctgttgtgtctctgtccaacggagtgtctgtcctgaccagcaaagtgctggatctgaagaactacatcgacaagcagctgctgccaatcgtgaacaaacagagctgttctatcagcaatatcgaaaccgtgatcgagtttcagcagaaaaacaaccggctgctggaaatcactcgggagttcagcgtaaacgctggcgttacaacccctgtgtccacctacatgctgacaaattctgagctgctgagcctgatcaatgacatgcctatcacaaacgaccagaagaagctgatgagcaacaacgtgcctatcgtgagacagcaaagctacagcatcatgagcatcatcaaggaagaagtgctggcctacgtggtgcagctgcctctgtacggcgtgattgataccccttgctggaagctgcacaccagtcctctgtgtaccaccaataccaaagaaggctctaacatctgcctgacaagaaccgatagaggctggtactgcgacaacgccggaagcgtgtcattcttccctcaggccgagacatgcaaggtgcaaagcaacagggtgttctgcgatacaatgaacagcctgaccctgcccagcgaggtgaacctgtgcaacgtggacatcttcaaccccaaatatgattgcaagatcatgaccagcaagacagacgtgtccagcagcgtgattacaagcctgggcgccatcgtgtcctgctacggcaagacaaagtgcaccgcctctaacaagaatcggggcatcatcaaaacctttagcaatggctgcgactacgtcagcaacaagggcgtcgacaccgtgagcgtggggaacaccctgtattacgtgaataagcaggagggcaagagcctgtacgtcaagggagagcccatcatcaacttctacgaccccctggtgtttcctagcgacgagttcgacgcctctatcagccaggtgaacgagaagatcaaccagagcctcgccttcatccggaagtccgacgagctgctc

SEQ ID NO: 146 - DNA, 1401 bp, synthetic construct
  source 1..1401: mol_type = other DNA
cagaacatcacagaggagttctaccagagcacctgttccgctgtgtccaagggctacctgagcgccctgagaacaggctggtacacctccgtgattaccatcgagctgtctaatatcaaggaacccaagtgcaacggcaccgacgccaaggtgaagctgatcaaacaggagctggacaagtacaagaacgcagtgaccgagctgcagctgctgatgcagagcggcggccccggctctggaggtggcggcagcggcggaggcggcagtagattcctgggcttccctctgggcgtgggatcagctatcgcctctggcgtggccgtgtctaaggtgctgcacctgcctggcgaggtgaacaagatcaagagcgctctgctgagcaccaacaaagccgtggtgagcctttctaacggcgtcagcgtgctgaccagcaaggtgctggacctgaagaattacatcgataaacagctgctccccatcgtgaacaagcaaagctgcagcatcagcaatattgaaaccgtcatcgagtttcagcagaagaacaaccggctgctggaaatcacaagggagttcagcgtgaacgccggcgtgaccacccctgtgtccacctacatgctgacaaatagcgaactgctgagcctgatcaatgatatgcctatcacaaacgaccagaaaaagctgatgagcaacaacgtgcagatcgtgcggcaacagagctacagcatcatgtccatcattaaggaagaggtgctggcttacgtggtccagctgccactgtatggcgtgatcgacaccccttgttggaagctgcacaccagccctctctgtacaaccaacaccaaggagggcagcaacatctgcctgaccagaaccgatagaggatggtactgcgacaacgccggcagcgtatcattcttcccccaggccgagacatgcaaggtgcagagtaacagagtgttctgcgataccatgaacagcctgacactgcctcctgaagtgaacctgtgcaatgtggacatcttcaaccccaagtacgattgcaagatcatgacatctaaaacagacgtgtcttcctctgtgatcacctccctgggcgctatcgtgagctgctacggcaagacaaagtgcacagccagcaacaaaaatagaggcatcatcaaaacctttagcaatggatgtgactacgttagcaacaagggtgtggatacagtgtccgtgggaaataccctgtactacgtcaacaagcaggagggcaaaagcctgtacgtgaaaggcgaacctatcatcaacttctacgaccccctggtgtttccatctgatgagttcgacgccagcatctctcaggtgaacgagaagatcaaccagagcctggccttcatccggaagagcgacgagctgctg

SEQ ID NO: 147 - DNA, 1401 bp, synthetic construct
  source 1..1401: mol_type = other DNA
cagaacatcaccgaggagttctaccagagcacctgcagcgccgtgtctaagggctacctgagcgctctgagaaccggctggtacaccagtgtgatcaccatcgagctgagcaacatcaaggaacccaagtgcaacggcaccgatgccaaggtgaagctgatcaagcaggagctggataagtacaagaatgccgtgacagagctacagctgctgatgcagagcggcggacctggcagcggcggcggaggtagcggcggcggcggcagcagattcctgggatttcccctcggcgttggcagcgctatcgccagcggcgtggccgtgtctaaagtgctgcacctgcctggcgaagtcaacaagattaagagcgccctgctgagcaccaacaaagccgtggtgtctctgagcaacggagtgagcgtgctgaccagcaaggtgctggacctgaaaaactacatcgacaagcagctgctgccaatcgtgaacaagcaaagctgcagcatccctaacattgagacagtgatcgagttccagcagaaaaacaaccggctgctcgaaatcaccagagagttcagcgtgaatgccggcgtgacaacacctgtgtctacctacatgctgaccaactccgagctgctgagcctgatcaatgacatgcctatcacaaacgaccagaagaagctgatgagcaacaacgtccagatcgtgcggcagcaaagctacagcatcatgtctatcatcaaggaggaagtgctggcctacgtggtgcagctgcctctgtacggcgtgattgacaccccatgttggaagctgcacacctccccactgtgcacgacaaacaccaaggaaggcagcaatatctgcctcacccggaccgatagaggctggtactgcgacaacgctggctctgtgagcttcttccctcaggccgagacatgcaaggtgcaaagcaacagagtgttttgtgacaccatgaactctctgaccctccctagcgaggtgaacctgtgtaatgtggatatcttcaaccccaaatacgactgcaagatcatgacatccaagactgacgtgagttctagcgtgatcacaagcctgggcgccatcgtgtcctgctacggcaaaaccaagtgtaccgccagcaacaagaataggggcattatcaaaacatttagcaatggctgtgactacgtgtccaacaagggcgtggacaccgtatcagttggaaacacactgtactacgtgaacaagcaggagggcaagtccctgtatgtgaagggagaacctatcatcaacttctacgatcccctggtgttccccagcgacgagttcgacgcttctatcagccaggtcaacgagaagatcaaccagagcctggccttcatcagaaagtccgatgagctgctg

SEQ ID NO: 148 - DNA, 1401 bp, synthetic construct
  source 1..1401: mol_type = other DNA
cagaacatcacagaggaattttaccagagcacctgttctgcagttagcaagggctatctgtctgctctgagaaccggctggtacaccagcgtgatcaccatcgagctgagcaacatcaaagaacccaagtgcaacggcaccgacgccaaggtgaaactgatcaagcaggagctggataagtacaagaacgccgtgaccgagctgcagctgctgatgcagtctggaggtcctggcagcggcggcggaggcagcggcggaggaggctctagattcctgggcttccccctgggagtgggctctgccatcgcctccggcgtggccgtgtccaaggtgttgcacctgccaggcgaagtgaataagatcaagagcgccctgctgagcaccaacaaggccgtggtctctctaagcaatggagtgtccgtgttgaccagcaaagtcctggacctgaagaattacatcgacaagcaactgctgcccattgtgaacaagcagtcttgcagcatccccaacatcgagacagtgatcgagtttcagcagaagaacaatagactgctggagatcacccgggagttcagcgtgaatgctggcgtgaccacccctgtgtctacatacatgctgaccaatagcgagctgctttccctgattaacgatatgcctatcacaaacgaccagaaaaagctgatgtccaacaacgtgcaaatcgtgcggcagcaaagctactctatcatgagcatcatcaaggaagaggtcctggcctacgtggtgcagctgcctctgtacggcgttatcgacaccccttgctggaagctgcacaccagtcctctgtgtaccaccaacacaaaggaaggcagcaatatctgcctgacaaggaccgatagaggctggtactgcgacaacgccggaagcgtgagcttcttccctcaggctgagacatgcaaggtgcagagcaatagagtgttttgcgacaccatgaacagcctcacactgcctcctgaggtgaacctgtgcaacgtggacatcttcaaccccaagtatgactgcaagatcatgaccagcaaaacagatgtgagcagcagcgtgatcacaagcctgggcgccattgtgagctgctacggcaagaccaaatgcaccgccagcaacaagaaccggggcatcatcaagaccttcagcaacggttgtgactacgtgagcaacaagggcgtggatacagtgtctgtgggcaacaccctgtactacgtcaacaagcaggaaggaaaaagcctgtatgtgaagggcgaacctattatcaacttctacgaccccctggtgttcccatctgatgagttcgacgccagcatcagccaggtgaacgagaagatcaaccagagcctggccttcatcagaaagtccgacgagctgctg

SEQ ID NO: 149 - DNA, 1401 bp, synthetic construct
  source 1..1401: mol_type = other DNA
cagaacattacagaggagttctaccagtccacctgtagcgccgtctctaagggatacctgagcgccctgagaaccggctggtacacctctgtgatcacaatcgagctgagcaatatcaaggaacctaagtgcaacggcaccgatgccaaggtgaaactgatcaagcaggagctggacaagtacaagaacgccgtgaccgagttgcagctgctgatgcagagcggcggtcctggctctggaggcggcggctctggcggcggaggcagcagattccctccattcctgctgggcgttggcagcgccatcgccagcggcgtggccgtgagcaaggtgctgcacctgcctggagaagtgaacaaaatcaaaagcgctctgctgagcaccaacaaggctgtggtgagcctgtctaatggagtgtccgtgctgacatctaaggtgctggatctgaagaactacatagacaagcagctgctgccaatcgtgaacaaacagtcttgcagcatccctaacattgaaaccgtgatcgagttccagcagaaaaacaacaggctgctggaaatcacccgggaattttctgtgaatgctggcgtgaccacccctgtgtctacatacatgctgaccaattctgagctgctgagcctgatcaacgacatgcctatcaccaatgaccagaagaagctgatgagcaacaacgtgcaaatcgtgcggcagcagagctacagcatcatgagcatcatcaaagaggaagtgcttgcttacgtggtccagctgcccctgtacggcgtgatcgatacaccttgctggaagctgcacaccagccctctgtgtaccacaaacaccaaggaaggcagcaatatctgcctgacaagaacagatagaggatggtactgcgacaacgccggcagcgttagcttcttcccccaggccgagacatgtaaagtgcaaagcaaccgggtgttctgcgacacaatgaacagcctgaccctgcctcctgaggtgaacctgtgcaatgttgacatcttcaaccccaagtacgactgcaagatcatgaccagcaagaccgacgtgtcaagcagcgtgatcaccagcctgggcgccatcgtgtcatgctacggcaaaaccaagtgcacagcctctaacaagaatagaggcatcatcaagacattcagcaacggctgtgattatgtcagcaacaagggcgtggacaccgtgagcgtgggcaacaccctgtattacgtgaacaagcaagagggcaagagcctctacgtgaagggcgaacccatcatcaacttctacgaccctctggtctttcccagcgacgagttcgacgccagcatcagccaggtgaacgagaagatcaaccagagcctggccttcatcagaaagtccgatgagctgctt

SEQ ID NO: 150 - DNA, 1401 bp, synthetic construct
  source 1..1401: mol_type = other DNA
cagaacatcaccgaggaattttaccagtccacatgcagcgccgtgagcaagggctacctgagcgctctgagaacaggatggtacaccagcgtgatcaccatcgagctgagcaacatcaaggaacctaagtgcaacggtacagatgctaaggtgaagctgatcaagcaggagctggataagtacaagaacgccgtgacagagctgcagctgctgatgcagtctggcggccccggctctggcggcggcggcagcggcggaggcggaagcagattccctccattcccccttggagtgggcagcgccatcgcctctggagtggccgtgtccaaggtgctgcacttgcctggcgaagtgaacaagattaagtctgccctgctgtctacaaacaaagccgtggtcagcctgagcaatggcgttagcgttctgacaagcaaagtgctggacctgaagaactacatcgacaagcaactgctgcctatcgttaacaaacaaagctgttctatccccaacatcgaaaccgtgatcgagttccagcaaaaaaacaaccggctgctggaaatcaccagagagttcagcgtgaacgccggagtgaccacccctgtgagcacctacatgctgaccaatagcgagctgctgagcctgatcaatgatatgcctatcaccaatgaccagaaaaagctgatgagcaacaacgtgcagatcgtgcggcagcagagctacagcatcatgagtatcatcaaggaagaggtgctggcctatgtggtgcagctgcccctgtatggcgtcattgacaccccttgctggaagctgcacacaagccctctctgcaccaccaacaccaaggaaggcagcaacatctgcctgaccagaaccgatagaggctggtactgcgacaacgctggaagcgtgagcttcttcccacaggctgaaacctgcaaggtccagagtaacagagtgttctgtgataccatgaacagcctcacactgccacctgaggtgaatctgtgtaatgtggacatcttcaaccccaagtacgactgcaagatcatgacctccaagacagacgtgtctagcagcgtgatcacatctctgggcgccattgtgtcctgctacggcaagaccaagtgcacagcctctaacaaaaatcggggcatcatcaagacctttagcaatggttgtgactacgtcagcaacaagggcgtggacaccgtgtcggtgggcaacaccctgtactacgtgaacaagcaggagggcaaaagcctgtacgtgaaaggcgagcctatcatcaacttctacgaccccctggtgtttccttctgatgagttcgacgccagcatcagccaggtgaacgagaaaatcaaccagagcctcgccttcatcaggaagtccgacgagctgctg

SEQ ID NO: 151 - DNA, 1401 bp, synthetic construct
  source 1..1401: mol_type = other DNA
cagaacatcacagaggagttctaccagagcacatgttctgccgtgtccaaaggctacctgtctgctctgcggaccggctggtacaccagcgttatcaccatcgagctgagcaacatcaaagaacctaagtgcaacggcaccgacgccaaggtgaaactgatcaagcaagagctggataagtacaagaacgccgtgaccgagctgcagctgctgatgcagagcggcggccctggcagcggaggcggcgggagcggcggcggcggcagcagattcctgggatttcccctgggcgtcggcagcgctattgcctccggtgtcgccgtgtctaaagtgctgcacctggaaggcgaggtgaacaaaatcaagagcgcactgctgtctacaaacaaggccgtggtgtctctcagcaacggcgttagcgtcctgacgagcaaggtgctggacctgaagaactacatcgacaagcagctgctgcctatcgtgaacaagcagtcttgtagccctccaaacatcgaaaccgtgatcgagttccagcaaaaaaacaatcggctgctcgaaatcacccgcgagtttagcgtgaacgccggagtgacaacccctgtgtctacctacatgctgacaaatagcgagctgctgtctctcatcaacgacatgcctatcaccaacgaccagaagaagctgatgagcaacaacgtccctatcgtgagacagcagtcctactccatcatgagcatcatcaaggaagaagtgctggcctacgttgtgcaattaccactgtatggcgtgatcgatacaccttgctggaagctgcacaccagccccctgtgcaccacgaataccaaggaaggcagcaatatctgcctgaccagaacagatagaggctggtactgcgacaacgctggatctgtgagcttcttcccacaggccgagacatgcaaggtgcagagcaatagagtgttctgcgataccatgaacagcctgacgctgccccccgaggtgaatctgtgtaatgtggacatcttcaaccccaagtatgactgcaagatcatgacctctaagaccgatgtgtctagcagcgtgatcacctccctgggcgccatcgtgagttgttacggcaagaccaagtgcacagccagcaacaagaacagaggaatcatcaagacattcagcaacggctgcgactacgtgagcaacaagggcgtggacaccgtgtccgtgggcaacaccctgtactacgtgaacaaacaggagggaaaaagcctgtacgtgaagggcgagcctatcattaacttctacgaccctctggtgttccctagcgatgagttcgacgccagcatcagccaggtgaacgagaagattaatcagagcctggctttcatccggaaaagcgacgagctgctg

SEQ ID NO: 152 - DNA, 1401 bp, synthetic construct
  source 1..1401: mol_type = other DNA
cagaacatcacggaagagttctatcagagcacctgtagcgccgtgagcaaaggatacctgtctgctctgagaacaggatggtatacatctgtgatcacaatcgagctgagcaatattaaagaacctaagtgcaacggcaccgatgccaaggtgaagctgatcaagcaggagctggacaagtataagaatgctgtgaccgagttgcagctgctgatgcagagcggcggtcctggctccggcggcggcggcagcggaggcggaggcagtagattccctcctttcctgctgggcgttggaagcgctatcgccagcggagtagccgtgtctaaggtgctgcacctgccaggcgaggtcaacaagatcaagagcgccctgctgtccacaaacaaggccgttgtgtctctgagcaatggagttagcgtgctgaccagcaaggtgctggatctgaaaaactacatcgacaagcaactgctgcctatcgtgaacaaacagtcctgcagcattcctccaatcgaaaccgtgatcgagtttcagcagaaaaacaaccggctgctggaaatcacaagagagtttagcgtgaacgccggcgtgaccacccctgtgtccacctacatgctgaccaacagcgagctgctgagcctcatcaatgatatgcctattaccaacgaccagaagaagctcatgagcaacaacgtgcctatcgtgcgccagcaaagctacagcatcatgagcatcatcaaggaagaagttcttgcttacgtggtgcagctgcctctgtacggcgtgatcgatacgccttgctggaagctgcacacatcccctctgtgtaccactaataccaaggaaggcagcaatatctgcctgaccagaaccgacagaggttggtactgtgacaacgccggctctgtgagctttttcccccaggccgagacatgcaaggtgcagagcaacagagtgttctgcgataccatgaacagcctgacactgccccccgaagtgaacctgtgtaatgtggacatcttcaaccccaagtacgactgcaaaatcatgaccagcaagaccgacgtctctagcagcgtgatcacctctctgggcgccatcgtgtcatgctacggcaagacaaagtgcaccgcctctaacaagaaccggggcatcatcaagaccttcagcaacggatgtgattacgtgagcaacaagggcgtggacaccgtgtccgtgggcaacaccctgtactacgtgaacaaacaagagggcaaaagcctgtacgtgaagggcgaacctattatcaacttctacgaccccctggtgttcccatctgatgagttcgacgccagcatcagccaggtgaacgagaagatcaaccagagcctggccttcatccggaagtccgacgagctcctg

SEQ ID NO: 153 - DNA, 1401 bp, synthetic construct
  source 1..1401: mol_type = other DNA
cagaacatcacagaagagttctaccagtctacttgcagcgccgtgagcaagggctacctgagtgccctgagaaccggctggtacaccagcgtgatcaccatcgagctgagcaacatcaaggaacccaagtgcaatggaacagacgccaaggtgaagctgatcaagcaggagctggacaagtacaagaacgccgtcacagagctgcagctgctgatgcagagcggcggccccggcagcggcggcggcggctccggcggaggaggctcaagattcctgggatttcctctgggcgttggatctgcaatcgcctctggagtcgccgtgtctaaggtgctccacctggaaggcgaggtgaacaagatcaagagcgccctgctgtccaccaacaaggccgtcgtgagcctgagcaacggcgtgagcgtgctgacaagcaaggtgctggacctgaaaaactacatcgataagcaacttttacccatcgttaacaaaccttcttgtagcataagcaacatcgagacagtgatcgagtttcagcagaaaaacaatagactgctggaaatcactcgggaatttagcgtgaacgctggcgtgaccacccctgtgtccacctacatgctgaccaatagcgagctgcttagcctgatcaacgacatgcctattaccaatgaccagaagaaactgatgagcaacaacgttcctatcgtgcggcagcagagctacagcatcatgtctatcatcaaagaggaagtgctggcctacgtggtgcagctgcctctgtacggcgtaatcgataccccatgctggaagctgcacacctctcctctgtgtaccacaaataccaaggaaggcagcaatatctgcctgacaagaacagatagaggatggtattgtgacaacgccggcagcgtctccttcttcccccaggccgaaacctgcaaggtgcaaagcaatagggtgttctgcgataccatgaacagcctgaccctgcctcctgaggtgaacctgtgcaacgtggacatcttcaacccaaagtacgactgcaagatcatgaccagcaagaccgatgtgagcagctccgtgatcacaagcctgggcgccatcgtgtcctgctacggcaagacaaagtgcaccgccagcaacaaaaacagaggaatcatcaagaccttcagcaatggttgtgattacgtgtccaacaaaggcgtggacaccgtgtctgtgggcaacaccctgtattacgtgaacaaacaggagggaaagtccctgtacgtcaagggcgagccaatcatcaacttctacgaccccctggtgttccctagcgacgagttcgacgccagcatcagccaggtgaacgagaagattaaccagagcctggcttttatcagaaagtctgatgagctgctg

SEQ ID NO: 154 - DNA, 1401 bp, synthetic construct
  source 1..1401: mol_type = other DNA
caaaacatcacagaggaattttaccagtccacctgttctgctgtcagcaaaggctacctgagcgccctacggaccggatggtatacaagcgtgatcactattgagctgtctaacatcaaggaacccaagtgcaacggcaccgacgccaaggtgaagctgatcaaacaggagctggataagtacaagaacgccgtgacagagctgcagctgctgatgcagtcgggcgggcctggctctggaggaggcggcagcggtggcggcggatctagattccctcctttcctgctgggcgttggcagcgccatcgcctccggcgtggccgtgagcaaggtgctgcacctggaaggcgaggtgaacaagatcaagagcgccctgctgtctaccaacaaggccgtggtctccctgagcaatggcgtgtccgtgctgaccagcaaagtcctggacctgaaaaattacatcgacaagcagctgcttcccattgtgaacaaacctagctgcagcattcccaacattgagacagtgatcgagttccagcaaaaaaacaacagactgctggaaatcacccgggagttcagcgtgaacgctggcgtgaccacacctgtcagcacatacatgctgaccaacagcgagctgcttagcctgatcaacgacatgcccatcaccaatgatcagaagaagctgatgagcaacaacgtgcagatcgtgcggcagcagagctacagcatcatgagcatcatcaaagaagaggtgctggcttacgtggtccagctgcctctgtacggcgtgatcgacaccccttgttggaagctgcacacctccccactttgtaccaccaacaccaaggaaggcagcaatatctgcctgacaagaaccgatagaggctggtactgcgacaacgccggcagcgtgtcttttttcccccaggccgagacatgcaaagttcagagcaatagagtgttctgcgatacaatgaacagcctgacactgcctccagaagtgaacctgtgtaatgtggacatcttcaaccccaagtacgactgcaagatcatgacaagcaagaccgatgtgtctagcagcgtgatcaccagtctcggcgccatcgtgtcctgctacggaaagaccaagtgcaccgccagcaacaagaacagaggcatcatcaagacattcagcaatggctgcgactacgtgtccaacaagggcgtcgacaccgtgtcagtgggcaataccctgtactacgtgaacaagcaggagggcaagagcctgtacgtgaagggcgagcctatcatcaacttctacgatcctctggtgtttccaagcgacgagttcgacgccagcatcagccaggtgaacgagaagatcaaccagtctctggccttcatcaggaagtccgacgagctgctg

SEQ ID NO: 155 - DNA, 1401 bp, synthetic construct
  source 1..1401: mol_type = other DNA
cagaacatcacagaggaattttaccagagcacatgcagcgctgtgagcaagggctacctgtctgctctgagaaccggctggtatacaagcgttatcacaatcgagttgtctaatatcaaggaacctaagtgtaatggcaccgatgccaaggtcaagctgatcaagcaggagctggacaagtacaagaacgccgtcaccgagctgcagctgctgatgcagagcggcggacctggaagcggaggcggcggcagcggcggaggcggaagcagattcccaccttttccactcggcgtgggctctgccatcgccagcggcgtggccgtgtccaaggtgctgcacctgccaggcgaggtgaacaagatcaaatccgccctgctgagcaccaacaaggccgtggttagcctgtctaacggcgtgagcgtgctgacatctaaggtgctggatctgaagaattacatcgacaagcagctgctccctatcgtgaacaagccctcttgtagcatccccaacatcgaaaccgtgatcgagttccagcaaaagaacaaccggctgctggagatcactcgggagttcagcgtcaacgccggcgtgaccacacctgtgagcacttacatgctgaccaacagcgagctgctgtctctgatcaacgacatgcctatcacaaatgaccagaaaaagctgatgagcaacaacgtgcctatcgtgcggcagcagagctacagcatcatgagcatcatcaaggaggaagtgctggcttacgtggtgcagctgcctctgtatggagtgatcgacaccccttgctggaagctgcacactagccctctgtgtacaaccaacaccaaggaaggcagcaacatctgcctgacccggaccgatagaggctggtactgcgacaacgcaggcagcgtgtccttcttcccccaggccgagacctgcaaggtgcaatccaatagagtgttctgcgacaccatgaacagcctgaccctgccccccgaggtgaacctgtgcaacgtggacattttcaaccccaagtacgactgcaagatcatgacctccaaaaccgacgtgtcctctagcgtgataacatctctgggagccatcgtgagctgctacgggaagaccaagtgcaccgcctctaacaagaacagaggcatcatcaaaacatttagcaatggctgtgactacgtttccaataaaggcgtggataccgtgagcgttggaaacacactgtactacgtgaataagcaagagggcaaatccctgtacgtgaagggcgagcctatcatcaacttctacgatcctctggtgttcccctctgatgagttcgacgccagcatcagccaggtgaacgagaaaatcaaccagtctctggccttcatcagaaagagcgacgagctgctg

SEQ ID NO: 156 - DNA, 1401 bp, synthetic construct
  source 1..1401: mol_type = other DNA
cagaacatcacggaagagttctaccagtcgacctgcagcgctgtgtccaagggatacctgagcgccctgagaaccggctggtacaccagcgtgatcactatcgagctgtccaacatcaaagagcctaagtgcaacggcacggacgccaaggtgaagctgatcaaacaggagctggacaagtataagaacgccgtcacagagctgcagctgctgatgcagtctggaggcggcggctcaggcggcggcggcagcggaggcggcggaagcagattccctccattccccctgggcgtgggaagcgccatcgccagcggcgtggccgtgtccaaggtgctgcacctggaaggcgaggtgaacaagatcaaaagcgcactgttgtctaccaataaggccgtggtgtctctgagcaacggggtttccgtgctgaccagcaaagtgctggatctgaagaactacattgataagcaactgctgcctatcgtgaacaagcagtcttgtagcattagcaatatcgagacagtgatcgagtttcagcagaaaaacaaccggctgctggaaatcacacgggagttcagcgtgaatgccggagtcaccacaccagtgagcacatacatgctgaccaatagcgaactgctgagcctgatcaatgacatgcctatcaccaacgaccagaagaagctgatgagcaacaacgtgcccatcgtcagacagcagagctacagcatcatgagtatcatcaaggaagaagtgctggcttatgtggtgcagctgcccctgtacggcgtcatcgacaccccttgttggaagctgcacacaagccctctgtgcaccaccaacaccaaggaaggctctaatatttgcctgaccagaacagatagaggctggtattgcgacaacgccggctctgtgagcttcttccctcaggccgagacatgcaaggtccagtccaatagggtgttctgcgataccatgaacagcctgacactgcctcctgaggtgaacctgtgtaacgtggatatcttcaaccccaaatacgactgcaagatcatgacctctaagaccgacgtgtctagcagcgtgatcaccagcctgggagccatcgtgagctgctacggcaaaaccaagtgtaccgccagcaacaagaaccggggcatcatcaagaccttcagcaacggctgcgactacgtgtccaacaagggcgtggacaccgtgtccgtgggcaacaccctgtactacgtgaacaaacaagagggcaagagcctgtacgtgaagggcgaacctatcatcaacttctacgaccccctggtgtttccatctgatgagttcgacgcctccatcagccaggtgaacgagaagattaaccagagcctcgccttcatcagaaagagcgacgagctgctt

SEQ ID NO: 157 - DNA, 1401 bp, synthetic construct
  source 1..1401: mol_type = other DNA
cagaacatcaccgaggagttctaccagagcacctgttctgccgtgagcaagggctacctgagcgctctgagaaccggctggtatacatctgtgatcacaatcgaactgagcaacatcaaggaacccaagtgcaacggcaccgacgccaaggtgaagctgatcaagcaggagctggacaagtacaaaaacgctgtgacagagctgcagctgctgatgcagtctggaggaggcggcagcggcggcggcggctccggcggcggaggcagcagattcccacctttccccctgggcgtgggctccgctatcgcctcaggcgtggccgtgtctaaagtgctgcacctggaaggagaagtgaacaagatcaagagcgccctgctgagcacaaacaaggccgtggtgtccctgagcaacggcgtgagcgtgctgacaagcaaagtgctggatctgaagaactacatcgacaagcaactgctgcccatcgtgaataaacagagctgcagcatacctaatatcgaaacagtgatcgaatttcagcagaaaaacaaccggctgcttgagatcaccagagagttttctgttaacgctggcgttaccaccccagtgagcacctacatgctgaccaacagcgaactgctcagcctgatcaatgacatgcctatcaccaacgaccagaagaagctgatgtctaacaatgtacctatcgtcagacagcaatcttacagcatcatgagcatcatcaaagaggaagtgctggcttatgttgtgcagctgcccctgtatggcgtgatcgacacaccctgctggaagctgcacaccagccctctgtgtacaaccaataccaaggagggaagcaacatctgcctgacccgcaccgatagaggctggtactgcgacaacgccggcagcgtgtcattcttccctcaggccgagacatgcaaggtgcaaagcaacagagtgttctgcgacaccatgaacagcctgacactgcctccagaggtgaatctgtgcaacgtggatatcttcaatcctaaatacgattgcaagatcatgacctccaagaccgacgtgagcagctccgtcatcaccagcctgggcgccattgtgtcttgttacggcaaaaccaagtgtaccgccagcaacaaaaaccggggaatcatcaagacattcagcaatgggtgtgactacgtgagcaacaagggcgtggatacagtcagcgtgggcaataccctgtactacgtcaacaagcaggagggcaagtccctgtacgttaagggagagcctatcattaacttctacgaccctctggtgttccccagcgacgagttcgacgcctctatcagccaggtgaacgagaagattaaccagtctctggcctttatccggaagtctgatgagctcctg

SEQ ID NO: 158 - DNA, 1401 bp, synthetic construct
  source 1..1401: mol_type = other DNA
cagaacatcaccgaggaattttaccagtctacctgcagcgccgtgtctaagggatacctgtctgccctgagaaccggctggtatacctccgtgatcaccatcgaactgtccaatatcaaggaaaacaagtgtaatggaacagacgccaaggtgaagctgatcaaacaggagctggacaagtacaagaacgccgtgaccgagctgcagctgctgatgcagagcggtggcggcggaagcggtggaggcggatctggcggcggcggctcaaggttcctgggcttccccctgggagttggaagcgccatcgccagcggcgtggccgtgtccaaggtgctgcacctggaaggcgaggtgaataaaatcaagtccgccctgctgagcacaaacaaggccgtggtgtctctctctaacggcgtctctgtgctgacttctaaggtgctggatctgaaaaactacatcgacaagcagctgctccctatcgtgaacaagcaatcttgtagcatccctaacatcgagaccgtcatcgagttccagcagaagaacaatagactgctggaaatcaccagagagtttagcgtgaacgctggcgtgacaacacctgtgagcacatacatgctgacaaatagcgagctgctgagcctgatcaacgacatgcctatcaccaacgaccagaaaaagctgatgagcaacaacgtgcagatcgtgcggcagcagagctacagcattatgagcatcatcaaggaagaggtgctggcttacgtggtgcaactgcctctgtacggcgtgattgacaccccttgttggaagctgcacaccagccccctttgtaccacaaataccaaagagggctccaatatctgcctgacaagaacagatagaggctggtactgcgacaacgccggctccgtgagcttcttcccacaggctgaaacctgtaaagtgcagagcaaccgggtgttctgcgatacaatgaacagcctgaccctgccatctgaagtgaacctgtgcaacgtggacatcttcaatcccaagtacgactgcaagatcatgaccagcaagaccgatgtgtccagcagcgtgattacaagcctgggcgccatcgtctcctgctacggcaagaccaagtgcacagccagcaacaaaaaccggggcatcatcaagaccttcagcaatggctgcgactacgtgagcaacaagggcgttgacaccgtgtctgtgggcaacaccctgtactacgtgaacaagcaggagggaaaaagcctgtatgtcaagggcgaacctatcatcaacttctacgaccccctggtgttcccttctgatgagttcgacgcctctataagccaggtgaacgagaagatcaaccagagcctggccttcatccggaagagcgacgagctgctg

SEQ ID NO: 159 - DNA, 1401 bp, synthetic construct
  source 1..1401: mol_type = other DNA
cagaacatcaccgaggaattttaccagtccacctgcagcgccgtgtctaagggatacctgagcgctctgagaacaggctggtacaccagcgtaattaccatcgagctgagcaacatcaaagagcctaagtgcaacggcaccgatgccaaggtcaagctgatcaagcaggagctggacaagtacaagaacgccgtgacagagctgcagctgctgatgcagagcggcggaggaggcagcggcggcggcggctcaggcggcggcgggagtagattcccccccttccctctgggcgtcggctctgctatcgccagcggcgtggccgttagcaaggtgctgcacctggaaggcgaggtgaacaaaatcaagtccgccctgctgtctacaaataaagccgtggtgagtctgtccaatggcgtctccgtgctgacaagcaaggtgctggatctgaagaactacatcgacaagcagctgctgcccatcgtgaacaagcaaagctgttctatccctaacatcgagaccgtgatcgagttccagcaaaagaacaaccggctgctggaaatcactcgggagttcagcgtgaacgccggcgtgaccacccctgtgagcacatacatgctgaccaacagcgagctgctcagcttgatcaacgacatgcctatcaccaatgaccagaaaaagctgatgagcaacaacgtgcagatcgtgcggcagcagagctacagcatcatgagcatcatcaaggaagaggtgctggcttatgttgtgcaactgcccctctacggcgtgatcgacaccccatgctggaagctgcacaccagccctctgtgcacaacaaacacgaaagaaggatctaacatctgcctgacaagaacagatagaggatggtactgcgacaacgctggcagcgtgtccttcttcccacaggctgaaacctgtaaagtgcagtctaatagagtcttctgcgacaccatgaacagcctgaccctgccacctgaggtgaatctgtgtaatgtggacatcttcaaccctaagtatgactgcaagatcatgacctctaagaccgacgtgtccagcagcgtgatcacctccctcggcgccattgtgtcttgctacggcaaaacaaagtgtacagccagcaacaaaaacaggggaatcatcaagacatttagcaacggatgtgactacgtgtctaataaaggcgtggatacagtgagcgtgggcaacaccctgtactacgtgaacaagcaggagggcaagagcctgtacgtgaagggcgaacctattatcaacttctatgatcctctggtgttccccagcgacgagttcgacgccagcatcagccaggtgaatgagaagatcaaccagtccctggcctttatcagaaagtctgatgagctgctg

SEQ ID NO: 160 - DNA, 1401 bp, synthetic construct
  source 1..1401: mol_type = other DNA
cagaacatcacggaagagttctaccagtctacatgctccgctgtgtctaagggctacctgagcgccctgagaaccggctggtacaccagcgtgatcacaatcgagctgtctaatattaaagaacccaagtgcaacggcaccgacgctaaggtgaagctgatcaagcaggagctcgataagtataagaacgctgtcacagagctgcaactgctgatgcagagcggcggcggcggttctcctggcggcggaagcggcggcggcggctcaagattcctgggcttccctctgggagttggaagcgccatcgcctctggcgtcgccgtctctaaagtgctgcacctggaaggcgaggtcaacaagatcaagtccgctctgcttagcacaaacaaggccgtggtgtctctgtccaatggcgtttccgtgcttacctctaaggtgctggacctgaaaaactacatcgacaagcaactgctccctatcgtgaacaagcagagctgcagcatcagcaacattgagacagtgatcgagtttcagcagaaaaacaatcggctgctggaaatcaccagggaatttagcgtgaatgccggcgtgaccacccctgtgtcaacctacatgctgacaaacagtgaactgctgagcctgatcaatgatatgcctatcaccaacgaccagaagaagctgatgtccaacaacgtcccaatcgtgagacagcagagctacagcatcatgagcatcatcaaggaagaggtgctggcttatgtagtgcagctgcctctgtacggcgtgattgatacaccatgttggaagctgcacacctctcccctctgcaccaccaataccaaggagggcagcaacatctgcctgacccggacagatagaggatggtactgcgacaatgccggatctgtctccttcttccctcaggccgagacttgtaaagtgcagagcaacagagtgttctgcgacaccatgaacagcctgaccctgccacctgaggtgaacctgtgtaacgtggacatcttcaaccccaagtacgactgcaagatcatgaccagcaagacagacgtgtccagcagcgtgatcacatctctgggcgccatcgtgagctgctacggcaagaccaagtgcaccgctagcaacaaaaatcggggcatcatcaagacattcagcaacggctgcgattacgtgagcaacaagggcgtggacaccgtgagcgtgggcaacacactgtactacgtgaacaaacaggagggaaaaagcctgtacgtgaaaggcgaacctatcatcaacttctacgaccctctggtgttccccagcgacgagttcgacgccagcatcagccaagtgaacgagaagatcaaccagagcctggccttcatcagaaagtctgatgagctgctg

SEQ ID NO: 161 - DNA, 1401 bp, synthetic construct
  source 1..1401: mol_type = other DNA
cagaacatcaccgaggaattttaccagtccacctgttctgccgtgagcaagggctacctgtctgctctgaggaccggctggtacaccagcgtcatcaccatcgagctgtccaacatcaaggaacctaagtgcaacggcacagatgccaaggtgaaactgatcaagcaagagctggataagtacaagaatgccgtgaccgagctgcagctgctgatgcagagcggcggcggcggccctggcggtggcggcagcggcggcggcggcagcagattcccccccttcctgctgggcgtcggctcagctatcgccagcggcgtggccgtcagcaaggtgctgcacctggaaggcgaggtgaacaagatcaagagcgccctgctgagcacaaacaaggccgtggtctcactgagtaatggcgtgtccgttctgacctccaaggtgctggatctgaagaactacatcgacaagcagctgctccccatcgtgaacaagcagagctgcagcatcagcaacatcgaaaccgtgatcgagtttcagcaaaagaacaaccggctgctggaaatcacccgggagttcagcgtgaacgccggagtgacaacacctgtgtctacatacatgctgaccaacagcgagctgctgagcctgatcaacgacatgcctatcacaaatgaccagaagaagctgatgtctaacaacgtgcctattgtgcggcagcagagctacagcatcatgagcatcatcaaagaggaagtgctggcttatgtggtgcagctgcctctgtacggcgtgatcgatacaccctgctggaagctgcacaccagccctctgtgtaccacgaacacaaaagagggcagcaacatctgcctgaccagaaccgatagaggatggtactgcgacaatgctggcagtgtgagcttcttcccacaggccgagacatgtaaagtgcagagcaacagagttttctgcgacaccatgaacagcctgaccctgcctccagaggtgaacctgtgcaatgtggacatcttcaaccccaagtacgactgcaagatcatgaccagcaagaccgacgtgagcagctctgtcattaccagccttggagccatcgtgtcttgctacggcaagaccaaatgcaccgccagcaacaaaaacagaggcatcatcaagacctttagcaatggatgtgactacgtgagcaacaagggagttgacacagtgtctgtgggcaacaccctgtactacgtgaataagcaggagggcaagagcctgtacgtgaagggcgagcctatcattaatttctacgaccccctggtgttcccttccgacgagttcgacgctagcatctcccaggtgaacgagaagatcaaccagagcctggccttcatcagaaagtctgatgaactgctg

SEQ ID NO: 162 - DNA, 1401 bp, synthetic construct
  source 1..1401: mol_type = other DNA
cagaacataacagaggagttctaccagagcacttgttctgccgtgtccaaaggctacctgtctgctctgagaacaggctggtacacctctgttatcaccatcgagctgagcaatatcaaagaacccaagtgcaacggtacagatgccaaggtgaaactgatcaagcaggagctggacaagtataagaacgccgtgaccgagctgcagctgctgatgcagagcggcggcggcggcagcggcggaggccctagcggaggcggcggcagcagattcccccccttccctctgggcgttggatctgccatcgccagcggggtggccgtgagcaaggtgctgcacctggaaggcgaggtgaacaagatcaagagcgccctgctgagcaccaacaaggccgtcgtgagcctgagcaacggcgtgtccgtgctgacaagcaaggtgctggatctgaaaaactacatcgacaagcagctgctgcctatcgtgaacaagcagagctgcagcatcagcaacatcgagacagtgatcgaatttcagcagaaaaacaaccggctgctggaaatcacaagagagttcagcgtgaatgctggcgtgaccacccctgtgtcaacatacatgctgaccaatagcgagctgctgagtttgatcaacgacatgcctattacaaatgaccagaagaagctgatgagcaacaacgtgcctatcgtcagacagcagtcctacagcatcatgagcatcatcaaggaggaagtgctagcttacgtggtgcagctgcccctgtatggagtcatcgatacaccttgctggaagctgcacaccagcccactgtgcaccaccaataccaaggaaggcagcaacatctgcctgacccggacagatagaggctggtattgcgacaacgccggctctgtgagttttttcccacaagctgaaacctgtaaagtacaatctaatagagtgttctgcgacaccatgaacagcctgaccctgcctccagaggtgaacctgtgtaacgtggacatcttcaaccctaagtacgattgcaagatcatgaccagcaagacagacgtgtccagcagcgtgatcacctccctcggcgccatcgtgtcctgctacggaaaaaccaagtgtaccgcctctaacaagaatcggggcattatcaaaacatttagcaacggctgcgactacgtgtctaataagggcgtcgacaccgtgtctgtgggcaacacactgtactacgtgaacaaacaagagggcaagtcactgtacgtgaagggcgagcctatcatcaacttctacgaccctctggtgttccccagcgacgagttcgacgcttctatcagccaggtgaacgagaagatcaaccagagcctggccttcatcaggaagtctgatgagctgctg

SEQ ID NO: 163 - DNA, 1464 bp, synthetic construct
  source 1..1464: mol_type = other DNA
cagaacatcaccgaggaattttaccagagcacatgctctgccgtgtctaagggctacctgagcgccctgagaaccggctggtatacaagcgtgatcacaatcgagctctccaacatcaaggagcctaagtgcaatggcaccgacgctaaagtgaagctgatcaagcaagagctggataagtacaaaaatgcagtgaccgagctgcagctgctgatgcagagcacacctgccaccaacaatagagccagaagggaactgcctagattcatgaactacaccctgaacaacgccaagaagaccaacgtgaccctgtccaagaagagaaagcggagatttctgggcttcctgctgggcgtgggctctgccatcgcctctggagtggccgtgagcaaagtgctgcatctgcccggcgaggtgaacaagatcaagagcgctctgctgagcacaaataaagccgtggtgtccctgtccaacggcgtgagcgtgctgaccagcaaggtgctggacctgaaaaactacatcgataagcaactgctgcctatcgtgaacaagcagtcttgtagcatttctaatatcgagaccgtgattgagttccagcagaagaacaacagactgctggaaatcactcgggagttcagcgtcaatgccggcgtgaccacaccagtgtctacctacatgttgacaaatagcgagctgctgagcctgatcaatgacatgcctatcaccaacgaccagaagaagctgatgagcaacaacgtgcccatcgtgcggcagcaatcatatagcatcatgagcattatcaaggaagaagtgctggcttacgtcgtccaactccccctgtacggagttatcgacaccccttgctggaagctgcacacctcacctctctgcaccaccaacacgaaggaaggcagcaacatctgcctgaccagaaccgatagaggctggtactgcgacaacgctggcagcgtgagcttcttcccccaggctgaaacctgtaaagtgcagagcaaccgggtgttctgcgacacaatgaacagcctgacactgccacctgaggtgaacctgtgtaacgtggacatcttcaacccaaagtacgactgcaagatcatgaccagcaagaccgacgtgtctagcagcgtgatcacatctctgggcgccatcgtgagctgctacggcaagacaaagtgcaccgcctctaacaagaatcgcggaatcatcaaaacatttagcaacggatgtgattacgtgagcaataaaggtgttgacaccgtgtccgtgggcaacaccctgtactacgtgaacaagcaggagggaaaatctctgtacgtgaagggcgaacccatcatcaacttctacgatcctctggtgttccctagcgacgagttcgacgccagcattagccaggtgaacgagaagatcaaccagagcctggccttcatcagaaagtccgatgagctgctg

SEQ ID NO: 164 - DNA, 1464 bp, synthetic construct
  source 1..1464: mol_type = other DNA
cagaacattaccgaggagttctaccagtctacctgcagcgccgtgtccaagggctacctgagcgccctgagaaccggctggtacaccagcgtgatcacaatcgagctgagcaacatcaaggaacccaagtgtaacggcaccgatgccaaggtgaagctgatcaagcaggagcttgataagtacaagaacgccgtgacagaactgcagctgctcatgcagagcacacccgccacaaacaaccgggccagaagggaactgccaagattcatgaactacaccctgaacaacgctaaaaagacaaacgtgacactgagcaagaagcggaagagacggttcctgggcttcctgctgggagtgggcagcgccatagctagcggcgtggccgtgtctaaggtgctgcacctgcctggcgaagtgaacaaaatcaagagtgccctgctgagcaccaacaaggccgtggtgtccctgtctaacggcgtgtctgttctgaccagcaaggtcctggacctgaagaattacatcgacaaacaactgctgcccatcgtgaacaagcagtcttgtagcatccctaacatcgaaaccgtgatcgagtttcagcagaaaaataatagactgctggaaatcaccagagaatttagcgtgaatgctggcgtgaccacccctgtgtccacctacatgctgacaaacagcgagctgctgagcctcatcaacgacatgcctatcaccaatgaccagaagaaactgatgagcaacaatgtgcccatcgtgcggcagcaaagctacagcatcatgagcatcatcaaggaagaggtgctggcctacgtcgtgcaactgccactgtacggagtcattgatacaccatgttggaagctgcacaccagtcctctgtgtaccacaaacacaaaggagggctctaacatctgcctgacaagaacagatagaggctggtactgcgacaacgccggcagcgtgtccttcttcccccaggccgagacatgcaaggtgcagtctaacagagttttctgcgataccatgaactctctgaccctgcctcctgaggtgaatctgtgcaatgtggatatcttcaaccctaagtatgactgcaagatcatgaccagcaagaccgacgtgtccagctctgtgatcacaagcctgggcgccatcgtgtcctgctacggcaaaaccaagtgcaccgccagcaacaagaacagaggcatcatcaaaacattcagcaatggatgtgactacgttagcaacaagggggtggacacagtgtctgtcggcaacaccctgtactacgtgaacaagcaggagggcaagtccctgtatgtgaaaggcgagcctatcatcaacttctacgatcctctggtgtttcctagcgacgagttcgacgccagcatcagccaggtgaacgagaagatcaaccagagccttgcttttatcagaaagagcgacgagctgctg

SEQ ID NO: 165 - DNA, 1464 bp, synthetic construct
  source 1..1464: mol_type = other DNA
cagaacatcaccgaggagttctaccagagcacatgcagcgccgtgagcaagggctacctgtctgcccttagaacaggctggtatacaagcgtgatcaccatcgagctgtccaatatcaaggagcctaagtgcaacggcaccgacgccaaggtgaaactgatcaagcaggagctggataagtacaagaacgccgtgaccgagctgcagctgctgatgcagagcacaccagccaccaacaaccgggccagaagagaactgcccagattcatgaactacaccctgaacaacgctaagaagacaaatgtgacactgagcaagaaaagaaagcggagattcctgggcttccctctgggagtcggaagcgctatcgccagcggcgtggccgtgtccaaagtgctgcacctgcctggagaagtgaacaagatcaagtctgctctgctgagcaccaacaaggcagtggtgagtctcagcaatggcgtctccgtgctgacctccaaggtgctggacctgaagaactacatcgacaaacaactgctgccaatcgtgaacaaacaatcttgcagcattcctaacatcgagactgtgatcgagtttcagcagaagaataacagactgctggaaatcaccagagagtttagcgttaacgctggcgtgacaacccctgtgtccacctacatgctgaccaacagtgaactgctgagcctgattaacgacatgcctatcaccaatgatcagaaaaaactgatgagcaacaatgtgccaatcgtgcggcagcaaagctacagcataatgagcatcatcaaagaggaagtgctggcctacgtcgtgcagctgcctctgtacggtgtgatcgacaccccttgttggaagctgcacaccagccctctgtgcaccacaaatactaaggaaggctccaacatctgcctgacacggaccgatagaggctggtactgcgacaacgccggctctgtgtccttcttcccccaggccgaaacctgcaaggtgcagagcaacagagtgttctgcgacacgatgaacagcctgacactgccccccgaggtgaacctgtgtaatgtggacatcttcaaccccaagtacgattgcaagatcatgaccagcaagaccgatgtgtcttcttctgtcatcacaagcctgggcgccatcgttagctgctacggcaagaccaagtgtaccgccagcaacaagaacaggggcatcattaagaccttttctaatggatgtgactacgtgtctaacaagggcgtggatacagtgtcagtgggcaacaccctgtactacgtgaacaaacaggagggcaagagcctgtacgtgaagggcgagcccatcatcaatttctacgaccccctcgtgtttcctagcgacgagttcgacgccagcatcagccaggtgaacgagaagatcaaccagagcctggccttcatcagaaagagcgatgagctgctg

SEQ ID NO: 166 - DNA, 1464 bp, synthetic construct
  source 1..1464: mol_type = other DNA
cagaacatcacagaagagttctaccagagcacctgttctgccgtgtctaagggctacctgtctgccctgagaaccggctggtatacatctgtgatcacaatcgagctgtccaacataaaagagcctaagtgcaacggcaccgatgccaaggtgaagctgatcaagcaggagctggacaagtacaagaacgccgtgaccgagctacagctgctgatgcagagcacccctgccaccaacaacggcagcgctagcgaactgccaaggttcatgaactacaccctgaacaacgctaaaaagacaaatgtgacactgtctaagaagggcaaaggcagatttctaggcttcctgctgggcgttggaagcgccatcgcctctggcgtggccgtgagcaaagtgctgcacctgcctggcgaggtgaacaagatcaagagcgctctgctgtctaccaacaaggcagtggtgagcctgtctaacggcgtgtctgtcctgacctccaaggtgctggacctaaaaaactatatcgacaagcagctgctgcctatcgtgaacaagcaaagctgcagcatcagcaacatcgaaaccgtgatcgagtttcagcaaaagaacaatagactgctggaaatcacccgcgagttcagcgtcaacgccggagtgaccacccctgtgtcgacctacatgctgacaaacagcgagctgctgagcctgatcaacgatatgcccattacaaacgaccagaaaaagctgatgagcaacaacgttcctattgtgcggcagcagagctacagcatcatgagcattatcaaggaagaagtgctggcctacgtggtgcagctgcccctgtacggcgtgatcgataccccctgctggaagctgcacactagccctctctgtaccaccaataccaaggaaggcagcaacatctgcctgaccagaacagatagaggctggtactgcgataacgccggctctgtgtcctttttccctcaggccgagacatgcaaggtgcaatctaatcgggtgttctgtgacacaatgaacagcctgacactgccacctgaggtaaatctgtgtaatgtggacatcttcaaccccaagtacgactgcaagatcatgacctccaagacagacgtgtcctctagcgtgatcaccagcctgggagctatcgtgagctgctacgggaagaccaagtgcaccgccagcaataaaaaccggggcatcatcaagaccttcagcaacggctgcgactacgtcagcaacaaaggcgtggatacagtgtctgtgggaaacaccctgtactacgttaataagcaggagggcaagtccctctacgtcaagggcgaacctatcatcaacttctacgaccccctggtgtttccaagcgacgagttcgacgccagcatctcccaggtgaacgagaagatcaaccagagcctggccttcatccggaaaagcgacgagctcctg

SEQ ID NO: 167 - DNA, 1464 bp, synthetic construct
  source 1..1464: mol_type = other DNA
cagaacatcaccgaggaattttaccagtctacctgtagcgccgtgagcaagggatacctctctgctctgcggaccggctggtatacctccgttatcacaatcgagctgagcaacatcaaggaacctaagtgtaacgggaccgacgctaaggtgaaactgatcaagcaagagctggacaagtacaagaacgccgtgaccgagctgcagctgctgatgcagagcacccctgctacaaacaatggaagcgcctccgagctgcctagattcatgaactacaccctgaacaacgcaaagaagaccaacgtgaccctgagcaaaaagggcaagggcagatttctgggcttcctgctgggagtcggcagcgccatcgccagcggagtggccgtgtctaaggtgctgcacctgcctggcgaggtgaacaagatcaaatccgccctgctgagcaccaacaaggccgtggtctccctttctaacggcgtgtctgtgctgaccagcaaggtcctcgacctgaaaaattacatcgacaagcagctgctgcctatcgtgaacaagcagagctgcagcatccccaacatcgaaaccgtgatcgagtttcagcagaaaaacaatcggctgctggaaatcacccgggagttcagcgtgaacgccggcgttaccacacctgtgtccacatacatgctgacaaacagcgagctgctgtccctgatcaacgacatgcctattaccaacgaccagaagaagctgatgagcaacaacgtgcccatcgtgcgccagcaatcctacagcatcatgagcatcatcaaggaagaggtgctggcttatgtggtgcagctgcccctgtacggcgtgattgacaccccttgctggaagctgcacaccagccctctgtgtacaaccaataccaaggaaggctctaatatctgcctgaccagaaccgatagaggctggtactgcgacaacgccggcagcgtgagcttcttcccacaggccgagacatgtaaagtccagtctaatagagtgttctgcgatacaatgaacagcctgacactgccacctgaagtgaatctgtgcaatgttgatatcttcaaccccaaatacgactgcaagatcatgaccagcaagaccgacgtgagcagcagcgttatcaccagcctgggcgccattgtgtcctgctacggcaagaccaagtgcaccgccagcaacaaaaacagaggcatcattaagaccttcagcaacggctgtgattatgtgtcaaacaagggcgtggatacagtgagcgtgggaaataccctgtactacgtgaacaagcaagagggcaagtccctgtacgtgaagggcgaacccatcatcaacttctacgatcctctggtgttccccagcgacgagttcgacgcttctatttcacaggtgaatgagaagatcaaccagagcctggccttcatcagaaagtctgatgagctgctg

SEQ ID NO: 168 - DNA, 1464 bp, synthetic construct
  source 1..1464: mol_type = other DNA
cagaacatcaccgaggagttctaccagagcacctgttctgccgtgtccaaaggctacctgagcgccctcagaaccggctggtatacatccgtgatcactatcgagctgagcaatatcaaggaacctaagtgcaacggcaccgacgccaaggtgaagctgatcaagcaggagcttgataaatacaagaacgccgtgaccgagctgcagctgctgatgcagtctacccctgctacaaacaacggcagcgcctctgaactgcctagattcatgaattacaccctgaacaacgctaagaaaaccaatgtgaccctgtcaaaaaagggaaaaggaagattcctgggctttcctctgggggttggcagcgctatcgcctccggtgtcgccgtgagcaaagtgctgcacctgcctggcgaggtcaacaagatcaaaagcgctctgctgagcaccaataaggccgtggtctctctcagcaatggagtcagcgtgctgaccagcaaggtgctggacctgaagaactacattgacaagcaactgctgcctattgtgaacaagcagtcatgcagcatccctaacatcgagacagtgatcgagtttcagcaaaagaacaatcggctgttggagatcacccgcgagttcagcgttaatgccggcgtgacaaccccagtgtccacatacatgctgacgaacagcgagctgctgagcctgatcaatgatatgcctatcaccaacgaccagaagaaactgatgagtaacaacgtgcccatcgtgagacagcagagctacagtatcatgtctatcattaaagaagaggtgctggcttacgtggtgcagctgcccctgtatggcgttatcgacaccccatgctggaagctccatacaagccctctttgtaccaccaacaccaaggaaggcagcaacatctgcctgacccggacagatagaggctggtactgcgacaacgcaggctccgtgtccttcttccctcaggccgagacatgcaaggtgcagagcaatcgggtgttttgtgataccatgaacagcctgaccctgccacctgaggtgaatctgtgtaacgtggacatcttcaaccccaagtacgactgcaagatcatgacctctaagaccgatgtgtccagcagcgtgatcaccagcctgggagccattgtgagctgttacggcaagaccaagtgcacagccagcaacaagaaccggggcatcatcaagaccttcagcaacggctgcgactatgtgagcaacaagggcgtggacaccgtgagcgtgggcaacacactgtactacgtgaacaaacaggagggcaagtccctgtacgtgaagggcgaacccatcatcaacttctacgaccccctggtgttccccagcgatgagttcgacgcctctatttctcaagtgaacgagaagatcaaccagagcctggccttcatcagaaagagcgacgagctcctg

SEQ ID NO: 169 - DNA, 1347 bp, synthetic construct
  source 1..1347: mol_type = other DNA
cagaacatcaccgaggagttctaccagtctacctgtagcgccgtgtctaagggatacctgagcgccctgagaaccggctggtacaccagcgtgatcaccatcgagctgagcaacatcaaagagcctaagtgcaacggtacagacgccaaggttaagctgatcaaacaagagctggataagtacaagaacgccgtaaccgagctgcagctgctgatgcagagtacccctgcaactggcagcggctctgccatcgccagcggcgtggccgttagcaaagtactgcacctggaaggcgaggtgaacaaaatcaagtctgctctgctctccacaaacaaggccgtggtgagcctgtctaatggcgtgagcgtgctgaccagcaaggtgctggacctgaaaaactacatcgacaagcaactcctgccaatcgtcaacaagcagagctgcagcattagcaatattgaaaccgttatcgagtttcagcagaagaacaaccggctgctggaaatcacaagagagttcagcgtcaacgctggcgtgacaacccctgtgtctacctacatgctgaccaacagtgaactgctgagcctgatcaacgacatgcccatcaccaatgaccagaaaaagctgatgagcaacaacgtgcctatcgtgcggcagcaaagctacagcatcatgagcatcatcaaggaggaagtgctggcttatgtggtccagctgcctctgtatggcgtgattgatacaccttgttggaagctgcacacctcccctctgtgcaccacaaacacaaaggaaggctccaacatctgcctgacaagaacagatagaggctggtattgcgacaacgccggctctgttagcttcttcccccaggccgagacttgtaaagtgcagagcaatagagtgttctgcgacaccatgaacagcctgaccctgccccccgaagtgaacctgtgtaatgtcgacatcttcaaccccaagtacgactgcaagatcatgaccagcaagaccgacgtgtctagcagcgtgatcacctctctgggcgccatcgtgtcctgctacggcaagaccaagtgcaccgccagcaacaagaaccggggcatcatcaagacatttagcaatggatgtgattacgtgtccaacaaaggagtggacaccgtgtccgttggaaataccctgtactacgtgaacaagcaggagggcaaaagtctgtacgtgaagggcgaacctatcatcaacttctacgatcctctggtgtttccatctgatgagttcgacgccagcatcagccaggtgaatgagaagatcaaccagagcctggctttcatcagaaagagcgacgagctgctg

SEQ ID NO: 170 - DNA, 1347 bp, synthetic construct
  source 1..1347: mol_type = other DNA
cagaacatcaccgaggagttctaccagagcacgtgtagcgccgtgagcaaaggctacctgtctgccctgagaactggctggtacacctctgtcatcaccatcgagctgagcaacatcaaggaacctaaatgtaacggcacagacgccaaggtgaagctgatcaagcaggagctggataagtacaagaacgcagtgacagagctgcagctgctgatgcagagcacccccgccacaggctccggctccgccatcgcctctggagtcgctgttagcaaggtgctgcacctgcctggcgaggtgaacaaaatcaagtctgctctgctgagcaccaacaaggccgtggtctctctgagcaacggcgtgtcggtgctgacaagcaaggtcctggacctgaaaaactacatcgataagcaactgctgcctattgtgaacaagcaatcttgcagcatcagcaatatcgagaccgtgattgagttccagcagaaaaataaccggctgctggaaatcacccgggaatttagcgtgaacgccggagtgaccacccctgtgtctacctacatgctgaccaactcagagctgctgagcctgatcaatgacatgcctatcaccaacgaccagaagaagctgatgagcaacaatgtgccaatcgtgcggcaacagtcctacagcatcatgtctatcattaaggaagaggttctggcctacgtggtgcagctgccactgtacggcgtgatcgatacaccttgttggaagctgcacaccagtcctctgtgtacaaccaataccaaggaaggctctaacatctgcctgacaagaacagatagaggatggtattgtgacaacgctggcagcgtgagcttcttcccccaggccgagacatgcaaggtgcagagcaacagagtgttctgcgacaccatgaacagcctgacactgcctccagaggtgaatctgtgcaacgtggacatcttcaaccccaagtacgactgcaagatcatgaccagcaaaaccgatgtgtctagcagcgtgatcacaagcctgggagccatcgtgtcctgctacggcaaaaccaagtgcaccgccagcaacaagaacagaggcattatcaagacctttagcaacggctgcgattacgtgtctaacaaaggagtggacaccgtgagcgttggaaataccctgtactacgtgaacaagcaggagggcaagagcctgtatgtgaaaggcgagcccatcatcaacttctatgaccctctcgtgttccccagcgatgagttcgacgcctctatcagccaggtgaacgagaagatcaaccagagcctcgctttcatcagaaagagcgacgagctgctc

SEQ ID NO: 171 - DNA, 1347 bp, synthetic construct
  source 1..1347: mol_type = other DNA
cagaacatcaccgaggaattttaccagtctacctgtagcgctgtctctaaaggatatctgtccgctctgagaacaggctggtacaccagcgtgatcacaatcgaactgagcaacatcaaagagcctaagtgcaatggtacagatgccaaggtgaagctgattaagcaggagctggataagtacaagaacgctgtgaccgaactgcagctgctgatgcagagcacccctgctacaggcagcggcagcgcaatcgccagcggcgtcgccgtgtcaaaggtgctccatctgcctggcgaggtgaacaagatcaagagtgccctgcttagcaccaacaaagccgtggtgtctctgtctaatggcgtgtctgtgctgacaagcaaggtgctggacctgaagaactacatcgataagcagctgctgcccatcgtgaataaacagagctgcagcatccccaacatcgagacagtcatcgagttccagcagaaaaacaacaggctgctggaaatcacaagagagttcagcgtgaatgccggagtgacaacccctgtgagcacatacatgctgacaaatagcgagctgctgtctctgatcaacgacatgcctatcaccaatgaccagaagaagctgatgagcaacaacgtgcctatcgtgcggcagcagagctatagcatcatgagcattatcaaggaagaggtgctggcctacgtcgtgcaactgcccctgtacggcgtgatcgacacaccttgttggaagctgcacaccagccctctgtgcaccaccaacaccaaggaaggcagcaacatctgcctgaccagaaccgatagaggctggtactgcgataacgccggaagcgtgagcttcttcccccaagctgaaacctgcaaggtccagagcaacagagtgttttgtgacaccatgaactccctgaccctgccacctgaggtgaacctgtgcaacgtggacatcttcaaccccaaatacgactgcaagatcatgaccagcaagaccgacgtgtcttccagcgtgattacatctctgggcgccatcgtgagctgctacggcaagacaaagtgtacagccagcaataaaaaccggggcatcatcaagacctttagcaacggctgcgactacgtgtccaacaagggcgtggacaccgtgagtgtgggcaacaccctgtactacgtgaacaagcaggagggcaaaagcctgtatgttaagggagaacccatcatcaacttctacgatcctctggtgttcccatctgatgagttcgacgcctctatcagccaggtgaacgagaagatcaaccagtcactggccttcatcagaaagtccgacgagctgctc

SEQ ID NO: 172 - DNA, 1398 bp, synthetic construct
  source 1..1398: mol_type = other DNA
caaaacatcaccgaagaattttaccagagcacatgcagcgccgtgtctaaaggatacctgagcgccctgcggacaggatggtacacatctgtgatcacaatcgagctgagcaacatcaaagagcctaagtgcaacggcaccgatgccaaggtcaagctgattaagcaggagctggataagtacaagaacgccgtgaccgagctgcagctgctgatgcaaagcacacctgccaccaacaaccgcgccaggggctccggcagtggcagaagcctgggcttcctgctgggagtgggcagcgccatcgccagcggagtggccgtctctaaggtgctgcacctgcctggcgaagttaacaaaatcaagagcgcactgctgtctacaaacaaagccgtggtcagcctcagtaacggcgtgtccgtgctgacaagtaaggtgctggacctgaaaaactacatcgacaagcagctgttgccaatcgtgaacaagcaatcttgtagcatctccaacatcgagacagtgatcgagtttcagcagaagaacaaccggctgctggaaatcacccgggagttcagcgtgaacgccggtgtgaccaccccagtgagtacatacatgctgaccaacagcgagctgctgagcctcatcaacgacatgcctatcaccaatgatcagaaaaagctgatgtccaacaacgtgcctatcgttagacagcagagctactccatcatgagcattatcaaggaagaagtgctcgcttatgtggtgcagctgcctctgtatggcgtgatcgacaccccgtgctggaagctgcacacctcccctctgtgcaccacaaatactaaggaaggcagcaatatctgtctgaccagaacagatagaggatggtactgcgacaacgctggcagcgtgtccttcttcccccaggccgagacctgtaaagtccagtctaatagagtgttctgtgacaccatgaatagcctgacactgccccccgaggtgaacctgtgcaatgttgacatcttcaaccccaagtacgattgcaagatcatgacaagcaagaccgacgtgagctctagcgtgatcacaagcctgggcgccatcgtgagctgctacggcaagaccaagtgcaccgccagcaacaagaatagagggatcatcaaaacctttagcaatggctgcgactacgtgtctaacaagggcgtggataccgtgtccgtgggaaataccctgtactacgtgaacaagcaggagggcaaaagcctgtacgtgaagggcgagcccatcattaacttctacgaccctctggtgttccctagcgacgagtttgacgcctcgatcagccaggtgaacgagaagatcaaccagagccttgctttcatcagaaagagcgacgagctgctg

SEQ ID NO: 173 - DNA, 1398 bp, synthetic construct
  source 1..1398: mol_type = other DNA
cagaacatcacagaggagttctaccagagcacatgcagcgctgtttccaagggctacctgtcagctcttagaaccggatggtacaccagcgtgatcacaatcgagctgagcaacatcaaagagcccaagtgcaacggtacagacgccaaggtgaagctgatcaaacaagagctggataagtacaagaacgccgtgaccgagctgcagctgctgatgcagagcacccctgccaccaacaatcgggccagaggcagcggaagcggaagaagcctgggcttcctgctgggcgtgggcagcgctatcgccagtggcgtcgccgtgtctaaagtgctgcacctccctggcgaggtgaacaagatcaagtccgccctgctgagcaccaacaaggccgttgtgtccctgagcaatggcgtgtctgtcctgaccagcaaggtgctggacctgaagaactacatcgacaagcaactgctgcccatcgtgaacaagcagagctgttctattcctaacatcgagacagtgatcgagtttcagcagaaaaacaaccggctgctggaaatcactcgggagttcagcgtgaatgccggcgttaccacccctgtgtccacctacatgctgaccaattctgagctgctcagcctgatcaacgacatgcctatcacaaatgaccagaaaaagctgatgtccaacaacgtgcctatcgtgcggcagcaaagctacagcatcatgagcatcatcaaggaagaggtgctggcttatgtggtgcagctgccactgtacggcgtgatagataccccctgttggaagctgcacaccagccctctgtgcaccaccaatacaaaggaaggcagcaacatctgcctgaccaggacagatagaggatggtactgcgataatgctggcagcgtgtcttttttccctcaggccgaaacctgtaaagtccagtctaacagagtgttctgcgacaccatgaactccctgaccctgccaccagaagtgaacctgtgtaatgtggacatcttcaaccccaagtacgactgcaagatcatgaccagcaagacagatgtgtcaagcagcgtgatcaccagcctgggcgccatcgtgtcctgttacggcaagaccaagtgcacagccagcaacaagaaccgcggcatcattaagaccttctccaacggctgcgactacgtgagcaacaaaggcgtggacacagtgtctgtgggaaataccctgtactacgtgaacaagcaggagggcaaaagcctgtacgtgaagggcgagcctatcatcaacttctacgaccctctggttttccccagcgacgagttcgacgcctctatcagccaggtgaacgagaagatcaaccagagcctggccttcatcagaaagtctgatgagctactc

SEQ ID NO: 174 - DNA, 1347 bp, synthetic construct
  source 1..1347: mol_type = other DNA
cagaacatcacagaagagttctaccagagcacatgcagcgccgtgtcaaagggatacctgtctgccctgagaaccggctggtataccagcgtgatcaccatcgagctgagcaatatcaaggaacccaagtgtaatggcacagacgccaaggtgaagctgatcaaacaagagctggacaagtacaagaatgctgtgaccgagctgcagctgctgatgttcctgggcttcccactgggcgtgggctctgctatcgcctctggagtcgccgtgtctaaagtgctgcacctggaaggcgaggtgaacaagatcaagagcgctctgctgagcaccaacaaggccgtggtcagcctgagcaacggcgtgagcgtcctgaccagcaaggtgctggatctgaagaactacatcgacaagcaactgctgcccatcgtgaataaacagtcttgttccatctccaacatcgaaaccgtgatcgagttccagcagaaaaacaacagactgctggaaataacccgggagttcagcgttaacgccggagtgaccacccctgtgagtacatacatgctgaccaacagcgagctgctctctctgatcaatgatatgcctattaccaacgatcagaaaaagctgatgagcaacaacgtgcccatcgtgcgccagcaaagctacagcatcatgagcatcatcaaggaggaagtgcttgcttatgtggtgcagctgcctctgtatggcgtgattgacaccccttgctggaagctgcacaccagccctctctgtaccacaaataccaaggaaggaagcaacatctgcctgaccagaacagatagaggctggtactgcgacaacgccggcagcgtctccttcttcccacaggccgagacatgtaaagttcagagcaatagagtgttctgcgacacaatgaacagcctgacactgccacctgaggtgaacctgtgcaacgtggacatcttcaaccctaagtacgactgcaagatcatgacctccaagaccgatgtgtctagcagcgtcatcacaagcctcggcgccatcgtgtcttgctacggcaagaccaagtgcaccgccagcaacaaaaaccggggcatcatcaagacatttagcaatggatgtgactacgtgtctaacaagggcgttgatacagtgtccgtgggcaacaccctgtactacgtaaacaagcaggagggcaagagcctgtacgtgaagggcgagcctatcatcaatttctacgaccctctggtgttccccagcgacgagttcgacgcctctatttctcaggtgaacgagaagatcaaccagagcctggccttcatcagaaagagcgacgagctgctg

SEQ ID NO: 175 - DNA, 1347 bp, synthetic construct
  source 1..1347: mol_type = other DNA
cagaacatcacagaagagttctaccagtctacctgtagcgctgtgtccaaaggctacctgagcgctctgagaaccggctggtacacctccgtgatcacgattgagctgagcaatatcaaggaacccaagtgcaacggcaccgacgccaaggtgaagctgatcaaacaggagctggacaagtacaagaatgccgtgaccgagctgcaactgctcatgttcctgggcttccccctgggcgtgggcagtgctatcgcctctggcgtggccgtgtctaaggtcctgcacctgcctggcgaggtgaacaagatcaagagcgccctgctgtctacaaacaaggccgttgtgtccctttctaacggcgtcagcgtgctgaccagcaaggtgctggatctgaagaactacatcgacaaacagctgctcccaatcgtgaacaagcagagctgcagcatctctaatatcgagacagtgatcgagtttcagcagaagaacaacagactgctggaaatcaccagggaatttagcgtcaacgccggagttacaacacctgtgtccacctacatgctgaccaatagcgagctgctgagcctgatcaatgatatgcctattaccaacgaccagaaaaagctgatgagcaacaacgtgcctatcgtgcgccagcaaagctacagcatcatgagcatcattaaggaagaagtgctcgcctacgtcgtgcagctgcctctgtacggcgtcatcgacaccccttgctggaagctgcacacctctccactgtgtaccaccaacacaaaggaaggcagcaacatctgcctgaccagaaccgatagaggctggtattgcgacaacgctggaagcgtgagttttttccctcaggccgagacatgtaaagtgcagagcaaccgggtgttctgcgacacaatgaacagcctgaccctgcctcccgaggtgaatctgtgcaacgtggacatcttcaaccccaaatacgactgcaagatcatgaccagcaagacagatgtgtctagcagcgtgatcactagcctgggagccatcgtgtcctgctacggcaagaccaagtgcaccgccagcaacaagaaccggggtatcatcaagaccttcagcaatggctgtgactacgtttctaacaagggcgtggacaccgtgtctgttggaaataccctgtactatgtgaacaagcaagagggcaagagcctgtacgtgaaaggcgaacctatcatcaacttctacgatcctctggtgttcccgagcgatgagttcgacgccagcatcagccaggtgaacgagaagatcaaccagagcctggccttcatcagaaagtccgacgagctgctg

SEQ ID NO: 176 - DNA, 1347 bp, synthetic construct
  source 1..1347: mol_type = other DNA
caaaacattacagaggaattttaccagagcacctgcagcgctgtgtctaaaggctacctgagcgccctgagaacaggatggtacaccagcgtgatcaccatcgagctgtctaacattaaggagcctaagtgcaatggcaccgatgccaaggtgaagctcatcaagcaagagctggacaagtataagaatgctgtgaccgagttgcagctgctgatgttcctgggcttcccactgggcgtgggatctgctatcgccagcggcgtggccgtgtccaaggtactgcacctgcctggcgaagtgaacaaaatcaagagcgccctgctgagcaccaacaaagccgtcgtgtccctgagcaacggcgtaagcgtgctgaccagcaaggtgctggacctgaagaactacatcgataagcagctgctcccaatcgtgaacaagcagtcttgtagcatccccaacatcgagacagtgatcgagtttcagcagaagaacaacagactgctggaaatcacccgggagttcagcgtgaacgccggcgtgacaacacctgtgtccacatacatgctgaccaatagcgagctgctgagcctgatcaatgacatgcctatcaccaacgatcagaaaaagctgatgagcaacaacgtgcccatcgtgcggcagcaaagctacagcatcatgagcatcatcaaggaggaagttcttgcttatgtggtgcagctgcctctgtacggcgtgatcgacaccccttgctggaagctgcacaccagccctctgtgcaccaccaacaccaaggaaggctccaatatctgcctgacaagaaccgacagaggctggtactgcgacaacgccggatctgtgtcattcttccctcaggccgagacatgtaaagtccagagcaacagagtgttttgtgataccatgaacagcctgacactgccccccgaggtgaacctgtgtaacgtggacatcttcaaccccaagtacgattgcaagatcatgacaagcaaaaccgacgtgtccagctccgtgatcaccagcctgggcgccatcgtgtcttgctacggcaagacaaagtgtaccgcctctaacaagaacaggggcattatcaagaccttcagcaacggctgcgactatgtgtctaataagggcgtcgacaccgtgtctgttggaaataccctgtactacgttaataaacaggagggcaaatctctgtacgtgaagggagaacctatcatcaacttctacgaccctctggtgttccccagcgatgagttcgacgccagcatcagccaggtgaacgagaagatcaaccagagcctggccttcatcagaaagagcgacgagctgctc

SEQ ID NO: 177 - DNA, 1560 bp, synthetic construct
  source 1..1560: mol_type = other DNA
atgaaatgtctgctgtacctggccttcctgttcatcggcgtgaactgccagaacatcaccgaggagttctaccagtctacatgttcagccgtgtctaagggatatctgagcgccctgcggaccggctggtacacctctgtgatcaccatcgagctgagcaacattaaggagcctaaatgtaatggcacagatgccaaagtgaagctgatcaaacaagagctggataagtacaagaacgctgtgaccgagctgcagctgctgatgcagagcggcggtcctggcagcggaggcggcggctctggcggcggcggcagccgatttccccccttccctctgggagtgggaagcgctatcgccagcggcgtcgccgtgtccaaggtgctgcacctgccaggcgaggtgaacaaaatcaagagcgccctgctcagcacaaacaaggccgtcgtgtctctgagcaacggcgtctccgtgctgaccagcaaggtgctggacctgaaaaactacatcgacaagcaactgctgcctatcgtgaacaagcagagctgcagcatcagcaatattgagaccgtgatcgagtttcagcagaagaacaatagactgctggaaatcacaagagagttcagcgtgaatgccggcgtgacaacccctgtgagcacctacatgctgacaaatagcgagctgctgagcctgatcaacgacatgcctatcaccaatgaccagaaaaagctgatgagcaacaacgtgcctatcgtgcggcagcaaagctacagcatcatgagcatcatcaaggaagaagttctggcctacgtggtccagctgccactgtatggcgtcatcgatacaccttgctggaagctgcacaccagccctctgtgtaccaccaacacgaaggaaggcagcaacatctgcctgaccagaaccgatagaggctggtactgcgacaacgccggatctgtgtccttcttcccccaggccgagacctgcaaggtgcagtcaaatagagtgttctgcgacaccatgaacagcttgaccctgcctccagaagtgaacctgtgcaacgtggacatcttcaaccccaagtacgattgcaagatcatgacttctaagaccgacgtgtcctcctctgtgattacatcccttggagccatcgtgtcgtgctacggcaaaaccaagtgcaccgccagcaacaagaaccggggcatcatcaagacattcagtaatggctgtgactacgtgagcaacaagggcgtcgacaccgtgtctgttggcaacaccctctattacgtgaacaagcaggaaggcaaaagcctgtacgtgaagggagaacccatcatcaacttctacgaccccctggtgtttcctagcgatgagttcgacgcttctatcagccaggtgaacgagaagatcaaccagtctctggctttcatcagaaagagcgacgagctgctcggcagcggatacatccccgaggcccctagagatggccaggcatacgtgcggaaggacggcgaatgggtgctgctgtctacatttctgcaccaccaccatcaccaccaccac

SEQ ID NO: 178 - DNA, 1593 bp, synthetic construct
  source 1..1593: mol_type = other DNA
atggaactgctcattctgaaggcaaatgccatcaccaccatcctgaccgccgtgaccttctgcttcgccagcggccagaacatcacagaggaattttaccagagcacctgcagtgccgtgagcaagggctacctgtctgccctgagaacaggctggtacaccagcgtgatcaccatcgagctgtccaacatcaaggaacctaagtgcaacggcaccgacgccaaggtgaagctgatcaagcaggagctggataagtacaagaacgccgtgaccgagctgcagctgctgatgcagagcggcggtcctggcagtggcggaggcggcagcggcggaggaggctctagattcccaccattccctcttggcgttggaagcgccatcgcctccggcgtggccgtgtctaaagtgctgcacctggaacccgaggtgaataaaatcaagagcgccctgctctccaccaacaaggccgtcgtgagcctgagcaatggcgtctctgtgctgactagcaaagtgctggacctgaaaaactacatcgacaagcagctgctgcctattgtgaacaagcaaagctgtagcatcagcaacatcgagacagttatcgagttccagcagaaaaacaaccggctgctggaaatcactcgggagttcagcgtgaacgctggcgttaccacacctgtgtccacctacatgctgacaaacagcgagctgctgtctctgatcaatgacatgcctatcacaaacgaccaaaagaagctgatgagcaacaacgtgcctatcgtgagacagcaaagctacagcatcatgagcatcatcaaagaggaagtgctggcttatgtggtgcagctacctctgtacggcgtgatcgacaccccctgctggaagctgcacaccagccctctgtgcaccacaaacaccaaggaaggcagcaatatatgcctgacccggacagatagaggatggtactgcgacaacgctggcagcgtgagcttcttcccccaggctgagacctgtaaagtgcagagcaacagagtgttctgcgacaccatgaacagcctgaccctgcctcctgaagtgaatctgtgtaatgtggacatcttcaaccccaagtacgactgcaagatcatgaccagcaagaccgacgtgtccagcagcgtgatcaccagcctgggcgccattgtgtcttgttacggaaagaccaagtgcaccgccagtaacaaaaatcgcggaatcatcaagacattcagcaacggctgcgattacgtgtccaacaagggcgtggatacagtgagcgtgggcaacacactgtactacgtgaacaagcaggagggcaagagcctgtatgtgaagggagagcccatcatcaacttctatgaccccctggtgttcccatctgatgagtttgatgccagcatctctcaggtgaacgagaagatcaaccagtctctggccttcatccggaaaagcgacgagctgctgagcgctatcggcggctacatccctgaggcccctagagatggccaggcctacgtcagaaaggacggcgaatgggtcctgctgagcacatttctgcaccaccaccaccatcaccaccac

SEQ ID NO: 179 - DNA, 1611 bp, synthetic construct
  source 1..1611: mol_type = other DNA
atggaacttctgatactgaaagccaacgccatcaccacaatcctgacagccgtgacattctgcttcgccagcggacagaacatcacagaggaattttaccagagcacctgcagcgctgtgtccaagggctacctgagcgccctgcggaccggctggtacaccagcgtcatcaccatcgagctgtctaacattaaagagcctaagtgcaacggcaccgacgctaaggtcaaactgatcaagcaagagctggacaagtacaagaacgccgtgaccgagctccagctgctgatgcagagcggtggacctggcagcggcggcggaggctctggaggcggcggcagccgatttcctccattccctctgggcgtgggcagtgccatcgctagtggagtcgccgtgtccaaggtgctgcacctggaacccgaggtgaacaaaatcaagagcgccctcctgagcacaaacaaggccgttgtttctctgtccaacggcgtgtccgtgctgacctcgaaggtgctggatctgaagaattacatcgacaagcaactgctgcctatcgtgaacaagcaatcttgttctatcagcaatatcgaaaccgtgatcgagtttcagcagaagaacaacagactgctggaaatcacccgggagttcagcgtgaacgccggcgtcaccacccctgtgtccacatacatgctgaccaacagcgagctgctgtctctgatcaatgacatgcctattacgaacgaccagaaaaagctgatgagcaacaacgtgcctatcgtgcgccagcagtcttacagcatcatgtctattatcaaagaagaagtgctggcctacgtggtgcagctccctctgtatggcgtgatcgacaccccttgttggaagctgcacaccagccccctgtgcaccaccaataccaaggaaggcagcaatatctgtctgaccagaaccgacagaggctggtactgcgataatgctggctctgtgtcattcttcccccaggccgagacatgcaaagtgcagtccaatagagtgttctgcgacacaatgaacagcctgacactgcctcctgaggtgaacctgtgtaatgtggacatcttcaaccccaagtatgattgcaagatcatgaccagcaagacagatgtgagcagcagcgtgatcaccagcctgggagccatcgtgtcctgctacggcaagaccaagtgtacagcctctaacaagaaccggggcatcatcaagacctttagcaacggctgcgactacgtgtctaacaagggcgtggatacagtgagcgtcggcaacaccctgtactacgtgaacaaacaggagggaaaaagcctgtacgtgaagggcgagccaatcatcaacttctacgaccccctggtgttccccagcgacgagttcgacgccagcatcagccaggtgaacgagaagatcaaccagagcctggccttcatcagaaagtccgatgagctgctatctgctatcggcagaatgaagcagatcgaacggaagattgaagagatcctgagcaagatctaccacatcgagaacgagatcgccagaatcaagaagctgatcggcgagagacaccaccaccatcaccaccaccac

SEQ ID NO: 180 - DNA, 1605 bp, synthetic construct
  source 1..1605: mol_type = other DNA
atggaactgctgatcctgaaggccaacgctatcacaaccatcctgacagccgtgaccttctgcttcgcctctggccagaacatcacagaggagttctaccagtctacatgtagcgctgtgtctaagggatatctgtctgccctgaggaccggctggtataccagcgtgatcacaatcgagctgagcaatatcaaggagcccaagtgtaacggcaccgatgccaaggtcaagctgatcaaacaggagctggacaagtacaagaacgccgtgacagagctgcaactgcttatgcagagcggcggccctggcagcggcggcggcggaagcggaggtggaggctccagattcccccccttccccctgggagtgggcagcgccatcgccagcggcgtggccgtgtccaaagtgctgcacctggaacctgaggtcaacaagatcaagtccgctctgctgagcacaaacaaggccgtggtgtccctgtccaatggagtgtctgtgctgaccagcaaagtgctggatctgaaaaactacatcgacaagcaactgctgcctatcgtgaacaagcaaagctgcagcattagcaacatcgagaccgtgatcgagtttcagcagaaaaacaacagactgctggaaatcacccgggaatttagcgtgaacgctggcgtgaccacgcctgtgagcacctacatgctgaccaacagcgagctgctgagcctgattaacgacatgcctatcaccaacgaccagaagaaactgatgagtaacaacgtgcctatcgtgcggcagcagagctactccatcatgagcatcatcaaggaagaagttctggcctacgtggtgcagctgccactctacggcgtgatcgacacaccctgttggaagctccacacatctcctctgtgtaccaccaataccaaggaaggcagcaatatctgcctgaccagaaccgatagaggatggtactgcgacaacgccggcagcgtgtccttcttcccacaggccgagacatgcaaggtgcagtctaatcgggtgttctgcgataccatgaacagcctgacactgcctcctgaggttaacctgtgcaacgtggacatcttcaaccctaagtacgactgcaagatcatgaccagcaagacagacgtgagcagctctgttatcacatctctgggcgccatcgtgtcttgttacggcaagaccaagtgcaccgcctctaacaaaaatagaggcatcatcaagaccttcagcaatggctgcgactacgtgagcaacaagggcgtggacaccgtgtccgtcggcaacaccctgtactacgtcaacaagcaggagggcaagagcctctacgtgaagggcgaacccatcattaacttctacgatcctctcgtgtttcctagcgacgagttcgacgctagcattagccaggtgaatgagaagatcaaccagagcctggccttcatcagaaagtctgatgagctgctgggcagccggatgaaacagatcgagagaaagattgaagagatcctgagcaagatctaccatatcgaaaacgagatcgccagaatcaaaaagctgatcggcgagcggcaccaccatcaccaccaccaccac